European Patent Application EP 4 578 870 A1, published July 2, 2025. Title: 一种融合前构象的呼吸道合胞病毒重组融合蛋白、其制备方法及用途. Applicant: 北京百邑无忧科技发展有限公司. The sequence listing filed with the application follows.

SEQUENCE LISTING (180 sequences)

SEQ ID NO: 1 - protein, 574 aa, synthetic construct
MELLIHRSSAIFLTLAINALYLTSSQNITEEFYQSTCSAVSRGYFSALRTGWYTSVITIELSNIKETKCNGTDTKVKLIKQELDKYKNAVTELQLLMQNTPAANNRARREAPQYMNYTINTTKNLNVSISKKRKRRFLGFLLGVGSAIASGIAVSKVLHLEGEVNKIKNALLSTNKAVVSLSNGVSVLTSKVLDLKNYINNQLLPIVNQQSCRISNIETVIEFQQKNSRLLEITREFSVNAGVTTPLSTYMLTNSELLSLINDMPITNDQKKLMSSNVQIVRQQSYSIMSIIKEEVLAYVVQLPIYGVIDTPCWKLHTSPLCTTNIKEGSNICLTRTDRGWYCDNAGSVSFFPQADTCKVQSNRVFCDTMNSLTLPSEVSLCNTDIFNSKYDCKIMTSKTDISSSVITSLGAIVSCYGKTKCTASNKNRGIIKTFSNGCDYVSNKGVDTVSVGNTLYYVNKLEGKNLYVKGEPIINYYDPLVFPSDEFDASISQVNEKINQSLAFIRRSDELLHNVNTGKSTTNIMITTIIIVIIVVLLSLIAIGLLLYCKAKNTPVTLSKDQLSGINNIAFSK

SEQ ID NO: 2 - protein, 16 aa, synthetic construct
SGGPGSGGGGSGGGGS

SEQ ID NO: 3 - protein, 16 aa, synthetic construct
SGGGGSGGGGSGGGGS

SEQ ID NO: 4 - protein, 16 aa, synthetic construct
SGGGGSPGGGSGGGGS

SEQ ID NO: 5 - protein, 16 aa, synthetic construct
SGGGGPGGGGSGGGGS

SEQ ID NO: 6 - protein, 16 aa, synthetic construct
SGGGGSGGGPSGGGGS

SEQ ID NO: 7 - protein, 37 aa, synthetic construct
NTPAANNRARREAPQYMNYTINTTKNLNVSISKKRKR

SEQ ID NO: 8 - protein, 37 aa, synthetic construct
NTPAANNGSASEAPQYMNYTINTTKNLNVSISKKGKG

SEQ ID NO: 9 - protein, 7 aa, synthetic construct
STPATGS

SEQ ID NO: 10 - protein, 7 aa, synthetic construct
GSGSGRS

SEQ ID NO: 11 - protein, 25 aa, synthetic construct
MELLILKANAITTILTAVTFCFASG

SEQ ID NO: 12 - protein, 25 aa, synthetic construct
MELPILKTNAITAILAAVTLCFASS

SEQ ID NO: 13 - protein, 25 aa, synthetic construct
MELLIHRSSAIFLTLAVNALYLTSS

SEQ ID NO: 14 - protein, 16 aa, synthetic construct
MKCLLYLAFLFIGVNC

SEQ ID NO: 15 - protein, 19 aa, synthetic construct
MGWSCIILFLVATATGVHS

SEQ ID NO: 16 - protein, 17 aa, synthetic construct
MRAWIFFLLCLAGRALA

SEQ ID NO: 17 - protein, 18 aa, synthetic construct
MAFLWLLSCWALLGTTFG

SEQ ID NO: 18 - protein, 20 aa, synthetic construct
MYRMQLLSCIALSLALVTNS

SEQ ID NO: 19 - protein, 16 aa, synthetic construct
MKPIFLVLLVVTSAYA

SEQ ID NO: 20 - protein, 21 aa, synthetic construct
MAPGRIFLVLFLISNTKPIHP

SEQ ID NO: 21 - protein, 25 aa, synthetic construct
MATTAMRMIISIIFISTYVTHITLC

SEQ ID NO: 22 - protein, 21 aa, synthetic construct
MIPGRIFLVLLLIFNTKPIHP

SEQ ID NO: 23 - protein, 15 aa, synthetic construct
MNLLLILTFVAAAVA

SEQ ID NO: 24 - protein, 29 aa, synthetic construct
GSGYIPEAPRDGQAYVRKDGEWVLLSTFL

SEQ ID NO: 25 - protein, 35 aa, synthetic construct
GSRMKQIERKIEEILSKIYHIENEIARIKKLIGER

SEQ ID NO: 26 - protein, 31 aa, synthetic construct
SAIGGYIPEAPRDGQAYVRKDGEWVLLSTFL

SEQ ID NO: 27 - protein, 37 aa, synthetic construct
SAIGRMKQIERKIEEILSKIYHIENEIARIKKLIGER

SEQ ID NO: 28 - protein, 8 aa, synthetic construct
HHHHHHHH

SEQ ID NO: 29 - protein, 467 aa, synthetic construct
QNITEEFYQSTCSAVSRGYFSALRTGWYTSVITIELSNIKEPKCNGTDTKVKLIKQELDKYKNAVTELQLLMQSGGPGSGGGGSGGGGSRFLGFLLGVGSAIASGIAVSKVLHLEGEVNKIKNALLSTNKAVVSLSNGVSVLTSKVLDLKNYINNQLLPIVNQQSCRISNIETVIEFQQKNSRLLEITREFSVNAGVTTPLSTYMLTNSELLSLINDMPITNDQKKLMSSNVQIVRQQSYSIMSIIKEEVLAYVVQLPIYGVIDTPCWKLHTSPLCTTNIKEGSNICLTRTDRGWYCDNAGSVSFFPQADTCKVQSNRVFCDTMNSLTLPSEVSLCNTDIFNSKYDCKIMTSKTDISSSVITSLGAIVSCYGKTKCTASNKNRGIIKTFSNGCDYVSNKGVDTVSVGNTLYYVNKLEGKNLYVKGEPIINYYDPLVFPSDEFDASISQVNEKINQSLAFIRRSDELL

SEQ ID NO: 30 - protein, 467 aa, synthetic construct
QNITEEFYQSTCSAVSRGYFSALRTGWYTSVITIELSNIKETKCNGTDTKVKLIKQELDKYKNAVTELQLLMQSGGPGSGGGGSGGGGSRFLGFPLGVGSAIASGIAVSKVLHLEGEVNKIKNALLSTNKAVVSLSNGVSVLTSKVLDLKNYINNQLLPIVNQQSCRISNIETVIEFQQKNSRLLEITREFSVNAGVTTPLSTYMLTNSELLSLINDMPITNDQKKLMSSNVQIVRQQSYSIMSIIKEEVLAYVVQLPIYGVIDTPCWKLHTSPLCTTNIKEGSNICLTRTDRGWYCDNAGSVSFFPQADTCKVQSNRVFCDTMNSLTLPSEVSLCNTDIFNSKYDCKIMTSKTDISSSVITSLGAIVSCYGKTKCTASNKNRGIIKTFSNGCDYVSNKGVDTVSVGNTLYYVNKLEGKNLYVKGEPIINYYDPLVFPSDEFDASISQVNEKINQSLAFIRRSDELL

SEQ ID NO: 31 - protein, 467 aa, synthetic construct
QNITEEFYQSTCSAVSRGYFSALRTGWYTSVITIELSNIKETKCNGTDTKVKLIKQELDKYKNAVTELQLLMQSGGPGSGGGGSGGGGSRFLGFLLGVGSAIASGIAVSKVLHLEGEVNKIKNALLSTNKAVVSLSNGVSVLTSKVLDLKNYINNQLLPIVNQQSCRISNIETVIEFQQKNSRLLEITREFSVNAGVTTPLSTYMLTNSELLSLINDMPITNDQKKLMSSNVPIVRQQSYSIMSIIKEEVLAYVVQLPIYGVIDTPCWKLHTSPLCTTNIKEGSNICLTRTDRGWYCDNAGSVSFFPQADTCKVQSNRVFCDTMNSLTLPSEVSLCNTDIFNSKYDCKIMTSKTDISSSVITSLGAIVSCYGKTKCTASNKNRGIIKTFSNGCDYVSNKGVDTVSVGNTLYYVNKLEGKNLYVKGEPIINYYDPLVFPSDEFDASISQVNEKINQSLAFIRRSDELL

SEQ ID NO: 32 - protein, 467 aa, synthetic construct
QNITEEFYQSTCSAVSRGYFSALRTGWYTSVITIELSNIKETKCNGTDTKVKLIKQELDKYKNAVTELQLLMQSGGPGSGGGGSGGGGSRFLGFLLGVGSAIASGIAVSKVLHLEGEVNKIKNALLSTNKAVVSLSNGVSVLTSKVLDLKNYINNQLLPIVNQQSCRISNIETVIEFQQKNSRLLEITREFSVNAGVTTPLSTYMLTNSELLSLINDMPITNDQKKLMSSNVQIVRQQSYSIMSIIKEEVLAYVVQLPIYGVIDTPCWKLHTSPLCTTNIKEGSNICLTRTDRGWYCDNAGSVSFFPQADTCKVQSNRVFCDTMNSLTLPPEVSLCNTDIFNSKYDCKIMTSKTDISSSVITSLGAIVSCYGKTKCTASNKNRGIIKTFSNGCDYVSNKGVDTVSVGNTLYYVNKLEGKNLYVKGEPIINYYDPLVFPSDEFDASISQVNEKINQSLAFIRRSDELL

SEQ ID NO: 33 - protein, 467 aa, synthetic construct
QNITEEFYQSTCSAVSRGYFSALRTGWYTSVITIELSNIKEPKCNGTDTKVKLIKQELDKYKNAVTELQLLMQSGGPGSGGGGSGGGGSRFLGFPLGVGSAIASGIAVSKVLHLEGEVNKIKNALLSTNKAVVSLSNGVSVLTSKVLDLKNYINNQLLPIVNQQSCRISNIETVIEFQQKNSRLLEITREFSVNAGVTTPLSTYMLTNSELLSLINDMPITNDQKKLMSSNVQIVRQQSYSIMSIIKEEVLAYVVQLPIYGVIDTPCWKLHTSPLCTTNIKEGSNICLTRTDRGWYCDNAGSVSFFPQADTCKVQSNRVFCDTMNSLTLPSEVSLCNTDIFNSKYDCKIMTSKTDISSSVITSLGAIVSCYGKTKCTASNKNRGIIKTFSNGCDYVSNKGVDTVSVGNTLYYVNKLEGKNLYVKGEPIINYYDPLVFPSDEFDASISQVNEKINQSLAFIRRSDELL

SEQ ID NO: 34 - protein, 467 aa, synthetic construct
QNITEEFYQSTCSAVSRGYFSALRTGWYTSVITIELSNIKETKCNGTDTKVKLIKQELDKYKNAVTELQLLMQSGGPGSGGGGSGGGGSRFLGFPLGVGSAIASGIAVSKVLHLEGEVNKIKNALLSTNKAVVSLSNGVSVLTSKVLDLKNYINNQLLPIVNQQSCRISNIETVIEFQQKNSRLLEITREFSVNAGVTTPLSTYMLTNSELLSLINDMPITNDQKKLMSSNVPIVRQQSYSIMSIIKEEVLAYVVQLPIYGVIDTPCWKLHTSPLCTTNIKEGSNICLTRTDRGWYCDNAGSVSFFPQADTCKVQSNRVFCDTMNSLTLPSEVSLCNTDIFNSKYDCKIMTSKTDISSSVITSLGAIVSCYGKTKCTASNKNRGIIKTFSNGCDYVSNKGVDTVSVGNTLYYVNKLEGKNLYVKGEPIINYYDPLVFPSDEFDASISQVNEKINQSLAFIRRSDELL

SEQ ID NO: 35 - protein, 467 aa, synthetic construct
QNITEEFYQSTCSAVSRGYFSALRTGWYTSVITIELSNIKETKCNGTDTKVKLIKQELDKYKNAVTELQLLMQSGGPGSGGGGSGGGGSRFLGFPLGVGSAIASGIAVSKVLHLEGEVNKIKNALLSTNKAVVSLSNGVSVLTSKVLDLKNYINNQLLPIVNQQSCRISNIETVIEFQQKNSRLLEITREFSVNAGVTTPLSTYMLTNSELLSLINDMPITNDQKKLMSSNVQIVRQQSYSIMSIIKEEVLAYVVQLPIYGVIDTPCWKLHTSPLCTTNIKEGSNICLTRTDRGWYCDNAGSVSFFPQADTCKVQSNRVFCDTMNSLTLPPEVSLCNTDIFNSKYDCKIMTSKTDISSSVITSLGAIVSCYGKTKCTASNKNRGIIKTFSNGCDYVSNKGVDTVSVGNTLYYVNKLEGKNLYVKGEPIINYYDPLVFPSDEFDASISQVNEKINQSLAFIRRSDELL

SEQ ID NO: 36 - protein, 467 aa, synthetic construct
QNITEEFYQSTCSAVSRGYFSALRTGWYTSVITIELSNIKEPKCNGTDTKVKLIKQELDKYKNAVTELQLLMQSGGPGSGGGGSGGGGSRFLGFLLGVGSAIASGIAVSKVLHLEGEVNKIKNALLSTNKAVVSLSNGVSVLTSKVLDLKNYINNQLLPIVNQQSCRISNIETVIEFQQKNSRLLEITREFSVNAGVTTPLSTYMLTNSELLSLINDMPITNDQKKLMSSNVPIVRQQSYSIMSIIKEEVLAYVVQLPIYGVIDTPCWKLHTSPLCTTNIKEGSNICLTRTDRGWYCDNAGSVSFFPQADTCKVQSNRVFCDTMNSLTLPSEVSLCNTDIFNSKYDCKIMTSKTDISSSVITSLGAIVSCYGKTKCTASNKNRGIIKTFSNGCDYVSNKGVDTVSVGNTLYYVNKLEGKNLYVKGEPIINYYDPLVFPSDEFDASISQVNEKINQSLAFIRRSDELL

SEQ ID NO: 37 - protein, 467 aa, synthetic construct
QNITEEFYQSTCSAVSRGYFSALRTGWYTSVITIELSNIKEPKCNGTDTKVKLIKQELDKYKNAVTELQLLMQSGGPGSGGGGSGGGGSRFLGFLLGVGSAIASGIAVSKVLHLEGEVNKIKNALLSTNKAVVSLSNGVSVLTSKVLDLKNYINNQLLPIVNQQSCRISNIETVIEFQQKNSRLLEITREFSVNAGVTTPLSTYMLTNSELLSLINDMPITNDQKKLMSSNVQIVRQQSYSIMSIIKEEVLAYVVQLPIYGVIDTPCWKLHTSPLCTTNIKEGSNICLTRTDRGWYCDNAGSVSFFPQADTCKVQSNRVFCDTMNSLTLPPEVSLCNTDIFNSKYDCKIMTSKTDISSSVITSLGAIVSCYGKTKCTASNKNRGIIKTFSNGCDYVSNKGVDTVSVGNTLYYVNKLEGKNLYVKGEPIINYYDPLVFPSDEFDASISQVNEKINQSLAFIRRSDELL

SEQ ID NO: 38 - protein, 467 aa, synthetic construct
QNITEEFYQSTCSAVSRGYFSALRTGWYTSVITIELSNIKETKCNGTDTKVKLIKQELDKYKNAVTELQLLMQSGGPGSGGGGSGGGGSRFLGFLLGVGSAIASGIAVSKVLHLEGEVNKIKNALLSTNKAVVSLSNGVSVLTSKVLDLKNYINNQLLPIVNQQSCRISNIETVIEFQQKNSRLLEITREFSVNAGVTTPLSTYMLTNSELLSLINDMPITNDQKKLMSSNVPIVRQQSYSIMSIIKEEVLAYVVQLPIYGVIDTPCWKLHTSPLCTTNIKEGSNICLTRTDRGWYCDNAGSVSFFPQADTCKVQSNRVFCDTMNSLTLPPEVSLCNTDIFNSKYDCKIMTSKTDISSSVITSLGAIVSCYGKTKCTASNKNRGIIKTFSNGCDYVSNKGVDTVSVGNTLYYVNKLEGKNLYVKGEPIINYYDPLVFPSDEFDASISQVNEKINQSLAFIRRSDELL

SEQ ID NO: 39 - protein, 467 aa, synthetic construct
QNITEEFYQSTCSAVSRGYFSALRTGWYTSVITIELSNIKEPKCNGTDTKVKLIKQELDKYKNAVTELQLLMQSGGPGSGGGGSGGGGSRFLGFPLGVGSAIASGIAVSKVLHLEGEVNKIKNALLSTNKAVVSLSNGVSVLTSKVLDLKNYINNQLLPIVNQQSCRISNIETVIEFQQKNSRLLEITREFSVNAGVTTPLSTYMLTNSELLSLINDMPITNDQKKLMSSNVPIVRQQSYSIMSIIKEEVLAYVVQLPIYGVIDTPCWKLHTSPLCTTNIKEGSNICLTRTDRGWYCDNAGSVSFFPQADTCKVQSNRVFCDTMNSLTLPSEVSLCNTDIFNSKYDCKIMTSKTDISSSVITSLGAIVSCYGKTKCTASNKNRGIIKTFSNGCDYVSNKGVDTVSVGNTLYYVNKLEGKNLYVKGEPIINYYDPLVFPSDEFDASISQVNEKINQSLAFIRRSDELL

SEQ ID NO: 40 - protein, 467 aa, synthetic construct
QNITEEFYQSTCSAVSRGYFSALRTGWYTSVITIELSNIKEPKCNGTDTKVKLIKQELDKYKNAVTELQLLMQSGGPGSGGGGSGGGGSRFLGFPLGVGSAIASGIAVSKVLHLEGEVNKIKNALLSTNKAVVSLSNGVSVLTSKVLDLKNYINNQLLPIVNQQSCRISNIETVIEFQQKNSRLLEITREFSVNAGVTTPLSTYMLTNSELLSLINDMPITNDQKKLMSSNVQIVRQQSYSIMSIIKEEVLAYVVQLPIYGVIDTPCWKLHTSPLCTTNIKEGSNICLTRTDRGWYCDNAGSVSFFPQADTCKVQSNRVFCDTMNSLTLPPEVSLCNTDIFNSKYDCKIMTSKTDISSSVITSLGAIVSCYGKTKCTASNKNRGIIKTFSNGCDYVSNKGVDTVSVGNTLYYVNKLEGKNLYVKGEPIINYYDPLVFPSDEFDASISQVNEKINQSLAFIRRSDELL

SEQ ID NO: 41 - protein, 467 aa, synthetic construct
QNITEEFYQSTCSAVSRGYFSALRTGWYTSVITIELSNIKETKCNGTDTKVKLIKQELDKYKNAVTELQLLMQSGGPGSGGGGSGGGGSRFLGFPLGVGSAIASGIAVSKVLHLEGEVNKIKNALLSTNKAVVSLSNGVSVLTSKVLDLKNYINNQLLPIVNQQSCRISNIETVIEFQQKNSRLLEITREFSVNAGVTTPLSTYMLTNSELLSLINDMPITNDQKKLMSSNVPIVRQQSYSIMSIIKEEVLAYVVQLPIYGVIDTPCWKLHTSPLCTTNIKEGSNICLTRTDRGWYCDNAGSVSFFPQADTCKVQSNRVFCDTMNSLTLPPEVSLCNTDIFNSKYDCKIMTSKTDISSSVITSLGAIVSCYGKTKCTASNKNRGIIKTFSNGCDYVSNKGVDTVSVGNTLYYVNKLEGKNLYVKGEPIINYYDPLVFPSDEFDASISQVNEKINQSLAFIRRSDELL

SEQ ID NO: 42 - protein, 467 aa, synthetic construct
QNITEEFYQSTCSAVSRGYFSALRTGWYTSVITIELSNIKEPKCNGTDTKVKLIKQELDKYKNAVTELQLLMQSGGPGSGGGGSGGGGSRFLGFLLGVGSAIASGIAVSKVLHLEGEVNKIKNALLSTNKAVVSLSNGVSVLTSKVLDLKNYINNQLLPIVNQQSCRISNIETVIEFQQKNSRLLEITREFSVNAGVTTPLSTYMLTNSELLSLINDMPITNDQKKLMSSNVPIVRQQSYSIMSIIKEEVLAYVVQLPIYGVIDTPCWKLHTSPLCTTNIKEGSNICLTRTDRGWYCDNAGSVSFFPQADTCKVQSNRVFCDTMNSLTLPPEVSLCNTDIFNSKYDCKIMTSKTDISSSVITSLGAIVSCYGKTKCTASNKNRGIIKTFSNGCDYVSNKGVDTVSVGNTLYYVNKLEGKNLYVKGEPIINYYDPLVFPSDEFDASISQVNEKINQSLAFIRRSDELL

SEQ ID NO: 43 - protein, 467 aa, synthetic construct
QNITEEFYQSTCSAVSRGYFSALRTGWYTSVITIELSNIKEPKCNGTDTKVKLIKQELDKYKNAVTELQLLMQSGGPGSGGGGSGGGGSRFPPFLLGVGSAIASGIAVSKVLHLEGEVNKIKNALLSTNKAVVSLSNGVSVLTSKVLDLKNYINNQLLPIVNQQSCRISNIETVIEFQQKNSRLLEITREFSVNAGVTTPLSTYMLTNSELLSLINDMPITNDQKKLMSSNVQIVRQQSYSIMSIIKEEVLAYVVQLPIYGVIDTPCWKLHTSPLCTTNIKEGSNICLTRTDRGWYCDNAGSVSFFPQADTCKVQSNRVFCDTMNSLTLPSEVSLCNTDIFNSKYDCKIMTSKTDISSSVITSLGAIVSCYGKTKCTASNKNRGIIKTFSNGCDYVSNKGVDTVSVGNTLYYVNKLEGKNLYVKGEPIINYYDPLVFPSDEFDASISQVNEKINQSLAFIRRSDELL

SEQ ID NO: 44 - protein, 467 aa, synthetic construct
QNITEEFYQSTCSAVSRGYFSALRTGWYTSVITIELSNIKETKCNGTDTKVKLIKQELDKYKNAVTELQLLMQSGGPGSGGGGSGGGGSRFPPFLLGVGSAIASGIAVSKVLHLEGEVNKIKNALLSTNKAVVSLSNGVSVLTSKVLDLKNYINNQLLPIVNQQSCRISNIETVIEFQQKNSRLLEITREFSVNAGVTTPLSTYMLTNSELLSLINDMPITNDQKKLMSSNVPIVRQQSYSIMSIIKEEVLAYVVQLPIYGVIDTPCWKLHTSPLCTTNIKEGSNICLTRTDRGWYCDNAGSVSFFPQADTCKVQSNRVFCDTMNSLTLPSEVSLCNTDIFNSKYDCKIMTSKTDISSSVITSLGAIVSCYGKTKCTASNKNRGIIKTFSNGCDYVSNKGVDTVSVGNTLYYVNKLEGKNLYVKGEPIINYYDPLVFPSDEFDASISQVNEKINQSLAFIRRSDELL

SEQ ID NO: 45 - protein, 467 aa, synthetic construct
QNITEEFYQSTCSAVSRGYFSALRTGWYTSVITIELSNIKETKCNGTDTKVKLIKQELDKYKNAVTELQLLMQSGGPGSGGGGSGGGGSRFPPFLLGVGSAIASGIAVSKVLHLEGEVNKIKNALLSTNKAVVSLSNGVSVLTSKVLDLKNYINNQLLPIVNQQSCRISNIETVIEFQQKNSRLLEITREFSVNAGVTTPLSTYMLTNSELLSLINDMPITNDQKKLMSSNVQIVRQQSYSIMSIIKEEVLAYVVQLPIYGVIDTPCWKLHTSPLCTTNIKEGSNICLTRTDRGWYCDNAGSVSFFPQADTCKVQSNRVFCDTMNSLTLPPEVSLCNTDIFNSKYDCKIMTSKTDISSSVITSLGAIVSCYGKTKCTASNKNRGIIKTFSNGCDYVSNKGVDTVSVGNTLYYVNKLEGKNLYVKGEPIINYYDPLVFPSDEFDASISQVNEKINQSLAFIRRSDELL

SEQ ID NO: 46 - protein, 467 aa, synthetic construct
QNITEEFYQSTCSAVSRGYFSALRTGWYTSVITIELSNIKEPKCNGTDTKVKLIKQELDKYKNAVTELQLLMQSGGPGSGGGGSGGGGSRFPPFLLGVGSAIASGIAVSKVLHLEGEVNKIKNALLSTNKAVVSLSNGVSVLTSKVLDLKNYINNQLLPIVNQQSCRISNIETVIEFQQKNSRLLEITREFSVNAGVTTPLSTYMLTNSELLSLINDMPITNDQKKLMSSNVPIVRQQSYSIMSIIKEEVLAYVVQLPIYGVIDTPCWKLHTSPLCTTNIKEGSNICLTRTDRGWYCDNAGSVSFFPQADTCKVQSNRVFCDTMNSLTLPSEVSLCNTDIFNSKYDCKIMTSKTDISSSVITSLGAIVSCYGKTKCTASNKNRGIIKTFSNGCDYVSNKGVDTVSVGNTLYYVNKLEGKNLYVKGEPIINYYDPLVFPSDEFDASISQVNEKINQSLAFIRRSDELL

SEQ ID NO: 47 - protein, 467 aa, synthetic construct
QNITEEFYQSTCSAVSRGYFSALRTGWYTSVITIELSNIKEPKCNGTDTKVKLIKQELDKYKNAVTELQLLMQSGGPGSGGGGSGGGGSRFPPFLLGVGSAIASGIAVSKVLHLEGEVNKIKNALLSTNKAVVSLSNGVSVLTSKVLDLKNYINNQLLPIVNQQSCRISNIETVIEFQQKNSRLLEITREFSVNAGVTTPLSTYMLTNSELLSLINDMPITNDQKKLMSSNVQIVRQQSYSIMSIIKEEVLAYVVQLPIYGVIDTPCWKLHTSPLCTTNIKEGSNICLTRTDRGWYCDNAGSVSFFPQADTCKVQSNRVFCDTMNSLTLPPEVSLCNTDIFNSKYDCKIMTSKTDISSSVITSLGAIVSCYGKTKCTASNKNRGIIKTFSNGCDYVSNKGVDTVSVGNTLYYVNKLEGKNLYVKGEPIINYYDPLVFPSDEFDASISQVNEKINQSLAFIRRSDELL

SEQ ID NO: 48 - protein, 467 aa, synthetic construct
QNITEEFYQSTCSAVSRGYFSALRTGWYTSVITIELSNIKEQKCNGTDTKVKLIKQELDKYKNAVTELQLLMQSGGPGSGGGGSGGGGSRFPPFLLGVGSAIASGIAVSKVLHLEGEVNKIKNALLSTNKAVVSLSNGVSVLTSKVLDLKNYINNQLLPIVNQQSCRISNIETVIEFQQKNSRLLEITREFSVNAGVTTPLSTYMLTNSELLSLINDMPITNDQKKLMSSNVPIVRQQSYSIMSIIKEEVLAYVVQLPIYGVIDTPCWKLHTSPLCTTNIKEGSNICLTRTDRGWYCDNAGSVSFFPQADTCKVQSNRVFCDTMNSLTLPPEVSLCNTDIFNSKYDCKIMTSKTDISSSVITSLGAIVSCYGKTKCTASNKNRGIIKTFSNGCDYVSNKGVDTVSVGNTLYYVNKLEGKNLYVKGEPIINYYDPLVFPSDEFDASISQVNEKINQSLAFIRRSDELL

SEQ ID NO: 49 - protein, 467 aa, synthetic construct
QNITEEFYQSTCSAVSRGYFSALRTGWYTSVITIELSNIKEPKCNGTDTKVKLIKQELDKYKNAVTELQLLMQSGGPGSGGGGSGGGGSRFLGFPLGVGSAIASGIAVSKVLHLEGEVNKIKNALLSTNKAVVSLSNGVSVLTSKVLDLKNYINNQLLPIVNQQSCRISNIETVIEFQQKNSRLLEITREFSVNAGVTTPLSTYMLTNSELLSLINDMPITNDQKKLMSSNVPIVRQQSYSIMSIIKEEVLAYVVQLPIYGVIDTPCWKLHTSPLCTTNIKEGSNICLTRTDRGWYCDNAGSVSFFPQADTCKVQSNRVFCDTMNSLTLPPEVSLCNTDIFNSKYDCKIMTSKTDISSSVITSLGAIVSCYGKTKCTASNKNRGIIKTFSNGCDYVSNKGVDTVSVGNTLYYVNKLEGKNLYVKGEPIINYYDPLVFPSDEFDASISQVNEKINQSLAFIRRSDELL

SEQ ID NO: 50 - protein, 467 aa, synthetic construct
QNITEEFYQSTCSAVSRGYFSALRTGWYTSVITIELSNIKEPKCNGTDTKVKLIKQELDKYKNAVTELQLLMQSGGPGSGGGGSGGGGSRFPPFLLGVGSAIASGIAVSKVLHLEGEVNKIKNALLSTNKAVVSLSNGVSVLTSKVLDLKNYINNQLLPIVNQQSCRISNIETVIEFQQKNSRLLEITREFSVNAGVTTPLSTYMLTNSELLSLINDMPITNDQKKLMSSNVPIVRQQSYSIMSIIKEEVLAYVVQLPIYGVIDTPCWKLHTSPLCTTNIKEGSNICLTRTDRGWYCDNAGSVSFFPQADTCKVQSNRVFCDTMNSLTLPPEVSLCNTDIFNSKYDCKIMTSKTDISSSVITSLGAIVSCYGKTKCTASNKNRGIIKTFSNGCDYVSNKGVDTVSVGNTLYYVNKLEGKNLYVKGEPIINYYDPLVFPSDEFDASISQVNEKINQSLAFIRRSDELL

SEQ ID NO: 51 - protein, 467 aa, synthetic construct
QNITEEFYQSTCSAVSRGYFSALRTGWYTSVITIELSNIKEPKCNGTDTKVKLIKQELDKYKNAVTELQLLMQSGGPGSGGGGSGGGGSRFPPFPLGVGSAIASGIAVSKVLHLEGEVNKIKNALLSTNKAVVSLSNGVSVLTSKVLDLKNYINNQLLPIVNQQSCRISNIETVIEFQQKNSRLLEITREFSVNAGVTTPLSTYMLTNSELLSLINDMPITNDQKKLMSSNVPIVRQQSYSIMSIIKEEVLAYVVQLPIYGVIDTPCWKLHTSPLCTTNIKEGSNICLTRTDRGWYCDNAGSVSFFPQADTCKVQSNRVFCDTMNSLTLPPEVSLCNTDIFNSKYDCKIMTSKTDISSSVITSLGAIVSCYGKTKCTASNKNRGIIKTFSNGCDYVSNKGVDTVSVGNTLYYVNKLEGKNLYVKGEPIINYYDPLVFPSDEFDASISQVNEKINQSLAFIRRSDELL

SEQ ID NO: 52 - protein, 467 aa, synthetic construct
QNITEEFYQSTCSAVSRGYFSALRTGWYTSVITIELSNIPETKCNGTDTKVKLIKQELDKYKNAVTELQLLMQSGGPGSGGGGSGGGGSRFPPFPLGVGSAIASGIAVSKVLHLEGEVNKIKNALLSTNKAVVSLSNGVSVLTSKVLDLKNYINNQLLPIVNQQSCRISNIETVIEFQQKNSRLLEITREFSVNAGVTTPLSTYMLTNSELLSLINDMPITNDQKKLMSSNVPIVRQQSYSIMSIIKEEVLAYVVQLPIYGVIDTPCWKLHTSPLCTTNIKEGSNICLTRTDRGWYCDNAGSVSFFPQADTCKVQSNRVFCDTMNSLTLPPEVSLCNTDIFNSKYDCKIMTSKTDISSSVITSLGAIVSCYGKTKCTASNKNRGIIKTFSNGCDYVSNKGVDTVSVGNTLYYVNKLEGKNLYVKGEPIINYYDPLVFPSDEFDASISQVNEKINQSLAFIRRSDELL

SEQ ID NO: 53 - protein, 467 aa, synthetic construct
QNITEEFYQSTCSAVSRGYFSALRTGWYTSVITIELSNIKETKCNGTPTKVKLIKQELDKYKNAVTELQLLMQSGGPGSGGGGSGGGGSRFPPFPLGVGSAIASGIAVSKVLHLEGEVNKIKNALLSTNKAVVSLSNGVSVLTSKVLDLKNYINNQLLPIVNQQSCRISNIETVIEFQQKNSRLLEITREFSVNAGVTTPLSTYMLTNSELLSLINDMPITNDQKKLMSSNVPIVRQQSYSIMSIIKEEVLAYVVQLPIYGVIDTPCWKLHTSPLCTTNIKEGSNICLTRTDRGWYCDNAGSVSFFPQADTCKVQSNRVFCDTMNSLTLPPEVSLCNTDIFNSKYDCKIMTSKTDISSSVITSLGAIVSCYGKTKCTASNKNRGIIKTFSNGCDYVSNKGVDTVSVGNTLYYVNKLEGKNLYVKGEPIINYYDPLVFPSDEFDASISQVNEKINQSLAFIRRSDELL

SEQ ID NO: 54 - protein, 467 aa, synthetic construct
QNITEEFYQSTCSAVSRGYFSALRTGWYTSVITIELSNIKETKCNGTDTKVKLIKQELDKYKNAVTELQLLMQSGGPGSGGGGSGGGGSRFLGFPLGVGSAIASGIAVSKVLHLEGEVNKIKNALLSTNKAVVSLSNGVSVLTSKVLDLKNYINNQLLPIVNQQSCRISPIETVIEFQQKNSRLLEITREFSVNAGVTTPLSTYMLTNSELLSLINDMPITNDQKKLMSSNVQIVRQQSYSIMSIIKEEVLAYVVQLPIYGVIDTPCWKLHTSPLCTTNIKEGSNICLTRTDRGWYCDNAGSVSFFPQADTCKVQSNRVFCDTMNSLTLPSEVSLCNTDIFNSKYDCKIMTSKTDISSSVITSLGAIVSCYGKTKCTASNKNRGIIKTFSNGCDYVSNKGVDTVSVGNTLYYVNKLEGKNLYVKGEPIINYYDPLVFPSDEFDASISQVNEKINQSLAFIRRSDELL

SEQ ID NO: 55 - protein, 467 aa, synthetic construct
QNITEEFYQSTCSAVSRGYFSALRTGWYTSVITIELSNIKEPKCNGTDTKVKLIKQELDKYKNAVTELQLLMQSGGPGSGGGGSGGGGSRFLGFPLGVGSAIASGIAVSKVLHLEGEVNKIKNALLSTNKAVVSLSNGVSVLTSKVLDLKNYINNQLLPIVNQQSCRISPIETVIEFQQKNSRLLEITREFSVNAGVTTPLSTYMLTNSELLSLINDMPITNDQKKLMSSNVQIVRQQSYSIMSIIKEEVLAYVVQLPIYGVIDTPCWKLHTSPLCTTNIKEGSNICLTRTDRGWYCDNAGSVSFFPQADTCKVQSNRVFCDTMNSLTLPSEVSLCNTDIFNSKYDCKIMTSKTDISSSVITSLGAIVSCYGKTKCTASNKNRGIIKTFSNGCDYVSNKGVDTVSVGNTLYYVNKLEGKNLYVKGEPIINYYDPLVFPSDEFDASISQVNEKINQSLAFIRRSDELL

SEQ ID NO: 56 - protein, 467 aa, synthetic construct
QNITEEFYQSTCSAVSRGYFSALRTGWYTSVITIELSNIKEPKCNGTDTKVKLIKQELDKYKNAVTELQLLMQSGGPGSGGGGSGGGGSRFLGFPLGVGSAIASGIAVSKVLHLEGEVNKIKNALLSTNKAVVSLSNGVSVLTSKVLDLKNYINNQLLPIVNQQSCRISPIETVIEFQQKNSRLLEITREFSVNAGVTTPLSTYMLTNSELLSLINDMPITNDQKKLMSSNVQIVRQQSYSIMSIIKEEVLAYVVQLPIYGVIDTPCWKLHTSPLCTTNIKEGSNICLTRTDRGWYCDNAGSVSFFPQADTCKVQSNRVFCDTMNSLTLPPEVSLCNTDIFNSKYDCKIMTSKTDISSSVITSLGAIVSCYGKTKCTASNKNRGIIKTFSNGCDYVSNKGVDTVSVGNTLYYVNKLEGKNLYVKGEPIINYYDPLVFPSDEFDASISQVNEKINQSLAFIRRSDELL

SEQ ID NO: 57 - protein, 467 aa, synthetic construct
QNITEEFYQSTCSAVSRGYFSALRTGWYTSVITIELSNIKEPKCNGTDTKVKLIKQELDKYKNAVTELQLLMQSGGPGSGGGGSGGGGSRFLGFPLGVGSAIASGIAVSKVLHLEGEVNKIKNALLSTNKAVVSLSNGVSVLTSKVLDLKNYINNQLLPIVNQQSCRISPIETVIEFQQKNSRLLEITREFSVNAGVTTPLSTYMLTNSELLSLINDMPITNDQKKLMSSNVPIVRQQSYSIMSIIKEEVLAYVVQLPIYGVIDTPCWKLHTSPLCTTNIKEGSNICLTRTDRGWYCDNAGSVSFFPQADTCKVQSNRVFCDTMNSLTLPSEVSLCNTDIFNSKYDCKIMTSKTDISSSVITSLGAIVSCYGKTKCTASNKNRGIIKTFSNGCDYVSNKGVDTVSVGNTLYYVNKLEGKNLYVKGEPIINYYDPLVFPSDEFDASISQVNEKINQSLAFIRRSDELL

SEQ ID NO: 58 - protein, 467 aa, synthetic construct
QNITEEFYQSTCSAVSRGYFSALRTGWYTSVITIELSNIKEPKCNGTDTKVKLIKQELDKYKNAVTELQLLMQSGGPGSGGGGSGGGGSRFPPFLLGVGSAIASGIAVSKVLHLEGEVNKIKNALLSTNKAVVSLSNGVSVLTSKVLDLKNYINNQLLPIVNQQSCRISPIETVIEFQQKNSRLLEITREFSVNAGVTTPLSTYMLTNSELLSLINDMPITNDQKKLMSSNVQIVRQQSYSIMSIIKEEVLAYVVQLPIYGVIDTPCWKLHTSPLCTTNIKEGSNICLTRTDRGWYCDNAGSVSFFPQADTCKVQSNRVFCDTMNSLTLPPEVSLCNTDIFNSKYDCKIMTSKTDISSSVITSLGAIVSCYGKTKCTASNKNRGIIKTFSNGCDYVSNKGVDTVSVGNTLYYVNKLEGKNLYVKGEPIINYYDPLVFPSDEFDASISQVNEKINQSLAFIRRSDELL

SEQ ID NO: 59 - protein, 467 aa, synthetic construct
QNITEEFYQSTCSAVSRGYFSALRTGWYTSVITIELSNIKEPKCNGTDTKVKLIKQELDKYKNAVTELQLLMQSGGPGSGGGGSGGGGSRFPPFPLGVGSAIASGIAVSKVLHLEGEVNKIKNALLSTNKAVVSLSNGVSVLTSKVLDLKNYINNQLLPIVNQQSCRISPIETVIEFQQKNSRLLEITREFSVNAGVTTPLSTYMLTNSELLSLINDMPITNDQKKLMSSNVQIVRQQSYSIMSIIKEEVLAYVVQLPIYGVIDTPCWKLHTSPLCTTNIKEGSNICLTRTDRGWYCDNAGSVSFFPQADTCKVQSNRVFCDTMNSLTLPPEVSLCNTDIFNSKYDCKIMTSKTDISSSVITSLGAIVSCYGKTKCTASNKNRGIIKTFSNGCDYVSNKGVDTVSVGNTLYYVNKLEGKNLYVKGEPIINYYDPLVFPSDEFDASISQVNEKINQSLAFIRRSDELL

SEQ ID NO: 60 - protein, 467 aa, synthetic construct
QNITEEFYQSTCSAVSRGYFSALRTGWYTSVITIELSNIKEPKCNGTDTKVKLIKQELDKYKNAVTELQLLMQSGGPGSGGGGSGGGGSRFLGFPLGVGSAIASGIAVSKVLHLEGEVNKIKNALLSTNKAVVSLSNGVSVLTSKVLDLKNYINNQLLPIVNQQSCRISPIETVIEFQQKNSRLLEITREFSVNAGVTTPLSTYMLTNSELLSLINDMPITNDQKKLMSSNVPIVRQQSYSIMSIIKEEVLAYVVQLPIYGVIDTPCWKLHTSPLCTTNIKEGSNICLTRTDRGWYCDNAGSVSFFPQADTCKVQSNRVFCDTMNSLTLPPEVSLCNTDIFNSKYDCKIMTSKTDISSSVITSLGAIVSCYGKTKCTASNKNRGIIKTFSNGCDYVSNKGVDTVSVGNTLYYVNKLEGKNLYVKGEPIINYYDPLVFPSDEFDASISQVNEKINQSLAFIRRSDELL

SEQ ID NO: 61 - protein, 467 aa, synthetic construct
QNITEEFYQSTCSAVSRGYFSALRTGWYTSVITIELSNIKEPKCNGTDTKVKLIKQELDKYKNAVTELQLLMQSGGPGSGGGGSGGGGSRFPPFLLGVGSAIASGIAVSKVLHLEGEVNKIKNALLSTNKAVVSLSNGVSVLTSKVLDLKNYINNQLLPIVNQQSCRISPIETVIEFQQKNSRLLEITREFSVNAGVTTPLSTYMLTNSELLSLINDMPITNDQKKLMSSNVPIVRQQSYSIMSIIKEEVLAYVVQLPIYGVIDTPCWKLHTSPLCTTNIKEGSNICLTRTDRGWYCDNAGSVSFFPQADTCKVQSNRVFCDTMNSLTLPPEVSLCNTDIFNSKYDCKIMTSKTDISSSVITSLGAIVSCYGKTKCTASNKNRGIIKTFSNGCDYVSNKGVDTVSVGNTLYYVNKLEGKNLYVKGEPIINYYDPLVFPSDEFDASISQVNEKINQSLAFIRRSDELL

SEQ ID NO: 62 - protein, 467 aa, synthetic construct
QNITEEFYQSTCSAVSRGYFSALRTGWYTSVITIELSNIKEPKCNGTDTKVKLIKQELDKYKNAVTELQLLMQSGGPGSGGGGSGGGGSRFPPFPLGVGSAIASGIAVSKVLHLEGEVNKIKNALLSTNKAVVSLSNGVSVLTSKVLDLKNYINNQLLPIVNQQSCRISPIETVIEFQQKNSRLLEITREFSVNAGVTTPLSTYMLTNSELLSLINDMPITNDQKKLMSSNVPIVRQQSYSIMSIIKEEVLAYVVQLPIYGVIDTPCWKLHTSPLCTTNIKEGSNICLTRTDRGWYCDNAGSVSFFPQADTCKVQSNRVFCDTMNSLTLPPEVSLCNTDIFNSKYDCKIMTSKTDISSSVITSLGAIVSCYGKTKCTASNKNRGIIKTFSNGCDYVSNKGVDTVSVGNTLYYVNKLEGKNLYVKGEPIINYYDPLVFPSDEFDASISQVNEKINQSLAFIRRSDELL

SEQ ID NO: 63 - protein, 467 aa, synthetic construct
QNITEEFYQSTCSAVSRGYFSALRTGWYTSVITIELSNIKEPKCNGTDTKVKLIKQELDKYKNAVTELQLLMQSGGPGSGGGGSGGGGSRFPPFPLGVGSAIASGIAVSKVLHLEGEVNKIKNALLSTNKAVVSLSNGVSVLTSKVLDLKNYINNQLLPIVNQPSCRISNIETVIEFQQKNSRLLEITREFSVNAGVTTPLSTYMLTNSELLSLINDMPITNDQKKLMSSNVPIVRQQSYSIMSIIKEEVLAYVVQLPIYGVIDTPCWKLHTSPLCTTNIKEGSNICLTRTDRGWYCDNAGSVSFFPQADTCKVQSNRVFCDTMNSLTLPPEVSLCNTDIFNSKYDCKIMTSKTDISSSVITSLGAIVSCYGKTKCTASNKNRGIIKTFSNGCDYVSNKGVDTVSVGNTLYYVNKLEGKNLYVKGEPIINYYDPLVFPSDEFDASISQVNEKINQSLAFIRRSDELL

SEQ ID NO: 64 - protein, 467 aa, synthetic construct
QNITEEFYQSTCSAVSRGYFSALRTGWYTSVITIELSNIKEPKCNGTDTKVKLIKQELDKYKNAVTELQLLMQSGGPGSGGGGSGGGGSRFPPFPLGVGSAIASGIAVSKVLHLEGEVNKIKNALLSTNKAVVSLSNGVSVLTSKVLDLKNYINNQLLPIVNQQSCRPSNIETVIEFQQKNSRLLEITREFSVNAGVTTPLSTYMLTNSELLSLINDMPITNDQKKLMSSNVPIVRQQSYSIMSIIKEEVLAYVVQLPIYGVIDTPCWKLHTSPLCTTNIKEGSNICLTRTDRGWYCDNAGSVSFFPQADTCKVQSNRVFCDTMNSLTLPPEVSLCNTDIFNSKYDCKIMTSKTDISSSVITSLGAIVSCYGKTKCTASNKNRGIIKTFSNGCDYVSNKGVDTVSVGNTLYYVNKLEGKNLYVKGEPIINYYDPLVFPSDEFDASISQVNEKINQSLAFIRRSDELL

SEQ ID NO: 65 - protein, 467 aa, synthetic construct
QNITEEFYQSTCSAVSRGYFSALRTGWYTSVITIELSNIKEPKCNGTDTKVKLIKQELDKYKNAVTELQLLMQSGGPGSGGGGSGGGGSRFPPFPLGVGSAIASGIAVSKVLHLEGEVNKIKNALLSTNKAVVSLSNGVSVLTSKVLDLKNYINNQLLPIVNQQSCRIPNIETVIEFQQKNSRLLEITREFSVNAGVTTPLSTYMLTNSELLSLINDMPITNDQKKLMSSNVPIVRQQSYSIMSIIKEEVLAYVVQLPIYGVIDTPCWKLHTSPLCTTNIKEGSNICLTRTDRGWYCDNAGSVSFFPQADTCKVQSNRVFCDTMNSLTLPPEVSLCNTDIFNSKYDCKIMTSKTDISSSVITSLGAIVSCYGKTKCTASNKNRGIIKTFSNGCDYVSNKGVDTVSVGNTLYYVNKLEGKNLYVKGEPIINYYDPLVFPSDEFDASISQVNEKINQSLAFIRRSDELL

SEQ ID NO: 66 - protein, 467 aa, synthetic construct
QNITEEFYQSTCSAVSRGYFSALRTGWYTSVITIELSNIKEPKCNGTDTKVKLIKQELDKYKNAVTELQLLMQSGGPGSGGGGSGGGGSRFPPFPLGVGSAIASGIAVSKVLHLEGEVNKIKNALLSTNKAVVSLSNGVSVLTSKVLDLKNYINNQLLPIVNQQSCRIPPIETVIEFQQKNSRLLEITREFSVNAGVTTPLSTYMLTNSELLSLINDMPITNDQKKLMSSNVPIVRQQSYSIMSIIKEEVLAYVVQLPIYGVIDTPCWKLHTSPLCTTNIKEGSNICLTRTDRGWYCDNAGSVSFFPQADTCKVQSNRVFCDTMNSLTLPPEVSLCNTDIFNSKYDCKIMTSKTDISSSVITSLGAIVSCYGKTKCTASNKNRGIIKTFSNGCDYVSNKGVDTVSVGNTLYYVNKLEGKNLYVKGEPIINYYDPLVFPSDEFDASISQVNEKINQSLAFIRRSDELL

SEQ ID NO: 67 - protein, 467 aa, synthetic construct
QNITEEFYQSTCSAVSRGYFSALRTGWYTSVITIELSNIKEPKCNGTDTKVKLIKQELDKYKNAVTELQLLMQSGGPGSGGGGSGGGGSRFLGFPLGVGSAIASGIAVSKVLHLPGEVNKIKNALLSTNKAVVSLSNGVSVLTSKVLDLKNYINNQLLPIVNQQSCRISNIETVIEFQQKNSRLLEITREFSVNAGVTTPLSTYMLTNSELLSLINDMPITNDQKKLMSSNVPIVRQQSYSIMSIIKEEVLAYVVQLPIYGVIDTPCWKLHTSPLCTTNIKEGSNICLTRTDRGWYCDNAGSVSFFPQADTCKVQSNRVFCDTMNSLTLPPEVSLCNTDIFNSKYDCKIMTSKTDISSSVITSLGAIVSCYGKTKCTASNKNRGIIKTFSNGCDYVSNKGVDTVSVGNTLYYVNKLEGKNLYVKGEPIINYYDPLVFPSDEFDASISQVNEKINQSLAFIRRSDELL

SEQ ID NO: 68 - protein, 467 aa, synthetic construct
QNITEEFYQSTCSAVSRGYFSALRTGWYTSVITIELSNIKEPKCNGTDTKVKLIKQELDKYKNAVTELQLLMQSGGPGSGGGGSGGGGSRFPPFLLGVGSAIASGIAVSKVLHLPGEVNKIKNALLSTNKAVVSLSNGVSVLTSKVLDLKNYINNQLLPIVNQQSCRISNIETVIEFQQKNSRLLEITREFSVNAGVTTPLSTYMLTNSELLSLINDMPITNDQKKLMSSNVPIVRQQSYSIMSIIKEEVLAYVVQLPIYGVIDTPCWKLHTSPLCTTNIKEGSNICLTRTDRGWYCDNAGSVSFFPQADTCKVQSNRVFCDTMNSLTLPPEVSLCNTDIFNSKYDCKIMTSKTDISSSVITSLGAIVSCYGKTKCTASNKNRGIIKTFSNGCDYVSNKGVDTVSVGNTLYYVNKLEGKNLYVKGEPIINYYDPLVFPSDEFDASISQVNEKINQSLAFIRRSDELL

SEQ ID NO: 69 - protein, 467 aa, synthetic construct
QNITEEFYQSTCSAVSRGYFSALRTGWYTSVITIELSNIKEPKCNGTDTKVKLIKQELDKYKNAVTELQLLMQSGGPGSGGGGSGGGGSRFPPFPLGVGSAIASGIAVSKVLHLPGEVNKIKNALLSTNKAVVSLSNGVSVLTSKVLDLKNYINNQLLPIVNQQSCRISNIETVIEFQQKNSRLLEITREFSVNAGVTTPLSTYMLTNSELLSLINDMPITNDQKKLMSSNVPIVRQQSYSIMSIIKEEVLAYVVQLPIYGVIDTPCWKLHTSPLCTTNIKEGSNICLTRTDRGWYCDNAGSVSFFPQADTCKVQSNRVFCDTMNSLTLPPEVSLCNTDIFNSKYDCKIMTSKTDISSSVITSLGAIVSCYGKTKCTASNKNRGIIKTFSNGCDYVSNKGVDTVSVGNTLYYVNKLEGKNLYVKGEPIINYYDPLVFPSDEFDASISQVNEKINQSLAFIRRSDELL

SEQ ID NO: 70 - protein, 467 aa, synthetic construct
QNITEEFYQSTCSAVSRGYFSALRTGWYTSVITIELSNIKEPKCNGTDTKVKLIKQELDKYKNAVTELQLLMQSGGPGSGGGGSGGGGSRFLGFPLGVGSAIASGIAVSKVLHLPGEVNKIKNALLSTNKAVVSLSNGVSVLTSKVLDLKNYINNQLLPIVNQQSCRISPIETVIEFQQKNSRLLEITREFSVNAGVTTPLSTYMLTNSELLSLINDMPITNDQKKLMSSNVPIVRQQSYSIMSIIKEEVLAYVVQLPIYGVIDTPCWKLHTSPLCTTNIKEGSNICLTRTDRGWYCDNAGSVSFFPQADTCKVQSNRVFCDTMNSLTLPPEVSLCNTDIFNSKYDCKIMTSKTDISSSVITSLGAIVSCYGKTKCTASNKNRGIIKTFSNGCDYVSNKGVDTVSVGNTLYYVNKLEGKNLYVKGEPIINYYDPLVFPSDEFDASISQVNEKINQSLAFIRRSDELL

SEQ ID NO: 71 - protein, 467 aa, synthetic construct
QNITEEFYQSTCSAVSRGYFSALRTGWYTSVITIELSNIKEPKCNGTDTKVKLIKQELDKYKNAVTELQLLMQSGGPGSGGGGSGGGGSRFPPFLLGVGSAIASGIAVSKVLHLPGEVNKIKNALLSTNKAVVSLSNGVSVLTSKVLDLKNYINNQLLPIVNQQSCRISPIETVIEFQQKNSRLLEITREFSVNAGVTTPLSTYMLTNSELLSLINDMPITNDQKKLMSSNVPIVRQQSYSIMSIIKEEVLAYVVQLPIYGVIDTPCWKLHTSPLCTTNIKEGSNICLTRTDRGWYCDNAGSVSFFPQADTCKVQSNRVFCDTMNSLTLPPEVSLCNTDIFNSKYDCKIMTSKTDISSSVITSLGAIVSCYGKTKCTASNKNRGIIKTFSNGCDYVSNKGVDTVSVGNTLYYVNKLEGKNLYVKGEPIINYYDPLVFPSDEFDASISQVNEKINQSLAFIRRSDELL

SEQ ID NO: 72 - protein, 467 aa, synthetic construct
QNITEEFYQSTCSAVSRGYFSALRTGWYTSVITIELSNIKEPKCNGTDTKVKLIKQELDKYKNAVTELQLLMQSGGPGSGGGGSGGGGSRFPPFPLGVGSAIASGIAVSKVLHLPGEVNKIKNALLSTNKAVVSLSNGVSVLTSKVLDLKNYINNQLLPIVNQQSCRISPIETVIEFQQKNSRLLEITREFSVNAGVTTPLSTYMLTNSELLSLINDMPITNDQKKLMSSNVPIVRQQSYSIMSIIKEEVLAYVVQLPIYGVIDTPCWKLHTSPLCTTNIKEGSNICLTRTDRGWYCDNAGSVSFFPQADTCKVQSNRVFCDTMNSLTLPPEVSLCNTDIFNSKYDCKIMTSKTDISSSVITSLGAIVSCYGKTKCTASNKNRGIIKTFSNGCDYVSNKGVDTVSVGNTLYYVNKLEGKNLYVKGEPIINYYDPLVFPSDEFDASISQVNEKINQSLAFIRRSDELL

SEQ ID NO: 73 - protein, 467 aa, synthetic construct
QNITEEFYQSTCSAVSRGYFSALRTGWYTSVITIELSNIKEPKCNGTDTKVKLIKQELDKYKNAVTELQLLMQSGGPGSGGGGSGGGGSRFLGFPLGVGSAIASGIAVSKVLHLPGEVNKIKNALLSTNKAVVSLSNGVSVLTSKVLDLKNYINNQLLPIVNQQSCRISNIETVIEFQQKNSRLLEITREFSVNAGVTTPLSTYMLTNSELLSLINDMPITNDQKKLMSSNVPIVRQQSYSIMSIIKEEVLAYVVQLPIYGVIDTPCWKLHTSPLCTTNIKEGSNICLTRTDRGWYCDNAGSVSFFPQADTCKVQSNRVFCDTMNSLTLPSEVSLCNTDIFNSKYDCKIMTSKTDISSSVITSLGAIVSCYGKTKCTASNKNRGIIKTFSNGCDYVSNKGVDTVSVGNTLYYVNKLEGKNLYVKGEPIINYYDPLVFPSDEFDASISQVNEKINQSLAFIRRSDELL

SEQ ID NO: 74 - protein, 467 aa, synthetic construct
QNITEEFYQSTCSAVSRGYFSALRTGWYTSVITIELSNIKEPKCNGTDTKVKLIKQELDKYKNAVTELQLLMQSGGPGSGGGGSGGGGSRFLGFPLGVGSAIASGIAVSKVLHLPGEVNKIKNALLSTNKAVVSLSNGVSVLTSKVLDLKNYINNQLLPIVNQQSCRISNIETVIEFQQKNSRLLEITREFSVNAGVTTPLSTYMLTNSELLSLINDMPITNDQKKLMSSNVQIVRQQSYSIMSIIKEEVLAYVVQLPIYGVIDTPCWKLHTSPLCTTNIKEGSNICLTRTDRGWYCDNAGSVSFFPQADTCKVQSNRVFCDTMNSLTLPPEVSLCNTDIFNSKYDCKIMTSKTDISSSVITSLGAIVSCYGKTKCTASNKNRGIIKTFSNGCDYVSNKGVDTVSVGNTLYYVNKLEGKNLYVKGEPIINYYDPLVFPSDEFDASISQVNEKINQSLAFIRRSDELL

SEQ ID NO: 75 - protein, 467 aa, synthetic construct
QNITEEFYQSTCSAVSRGYFSALRTGWYTSVITIELSNIKEPKCNGTDTKVKLIKQELDKYKNAVTELQLLMQSGGPGSGGGGSGGGGSRFLGFPLGVGSAIASGIAVSKVLHLPGEVNKIKNALLSTNKAVVSLSNGVSVLTSKVLDLKNYINNQLLPIVNQQSCRISPIETVIEFQQKNSRLLEITREFSVNAGVTTPLSTYMLTNSELLSLINDMPITNDQKKLMSSNVQIVRQQSYSIMSIIKEEVLAYVVQLPIYGVIDTPCWKLHTSPLCTTNIKEGSNICLTRTDRGWYCDNAGSVSFFPQADTCKVQSNRVFCDTMNSLTLPSEVSLCNTDIFNSKYDCKIMTSKTDISSSVITSLGAIVSCYGKTKCTASNKNRGIIKTFSNGCDYVSNKGVDTVSVGNTLYYVNKLEGKNLYVKGEPIINYYDPLVFPSDEFDASISQVNEKINQSLAFIRRSDELL

SEQ ID NO: 76 - protein, 467 aa, synthetic construct
QNITEEFYQSTCSAVSRGYFSALRTGWYTSVITIELSNIKEPKCNGTDTKVKLIKQELDKYKNAVTELQLLMQSGGPGSGGGGSGGGGSRFLGFPLGVGSAIASGIAVSKVLHLPGEVNKIKNALLSTNKAVVSLSNGVSVLTSKVLDLKNYINNQLLPIVNQQSCRISPIETVIEFQQKNSRLLEITREFSVNAGVTTPLSTYMLTNSELLSLINDMPITNDQKKLMSSNVQIVRQQSYSIMSIIKEEVLAYVVQLPIYGVIDTPCWKLHTSPLCTTNIKEGSNICLTRTDRGWYCDNAGSVSFFPQADTCKVQSNRVFCDTMNSLTLPPEVSLCNTDIFNSKYDCKIMTSKTDISSSVITSLGAIVSCYGKTKCTASNKNRGIIKTFSNGCDYVSNKGVDTVSVGNTLYYVNKLEGKNLYVKGEPIINYYDPLVFPSDEFDASISQVNEKINQSLAFIRRSDELL

SEQ ID NO: 77 - protein, 467 aa, synthetic construct
QNITEEFYQSTCSAVSRGYFSALRTGWYTSVITIELSNIKEPKCNGTDTKVKLIKQELDKYKNAVTELQLLMQSGGPGSGGGGSGGGGSRFPPFLLGVGSAIASGIAVSKVLHLPGEVNKIKNALLSTNKAVVSLSNGVSVLTSKVLDLKNYINNQLLPIVNQQSCRISPIETVIEFQQKNSRLLEITREFSVNAGVTTPLSTYMLTNSELLSLINDMPITNDQKKLMSSNVQIVRQQSYSIMSIIKEEVLAYVVQLPIYGVIDTPCWKLHTSPLCTTNIKEGSNICLTRTDRGWYCDNAGSVSFFPQADTCKVQSNRVFCDTMNSLTLPPEVSLCNTDIFNSKYDCKIMTSKTDISSSVITSLGAIVSCYGKTKCTASNKNRGIIKTFSNGCDYVSNKGVDTVSVGNTLYYVNKLEGKNLYVKGEPIINYYDPLVFPSDEFDASISQVNEKINQSLAFIRRSDELL

SEQ ID NO: 78 - protein, 467 aa, synthetic construct
QNITEEFYQSTCSAVSRGYFSALRTGWYTSVITIELSNIKEPKCNGTDTKVKLIKQELDKYKNAVTELQLLMQSGGPGSGGGGSGGGGSRFPPFPLGVGSAIASGIAVSKVLHLPGEVNKIKNALLSTNKAVVSLSNGVSVLTSKVLDLKNYINNQLLPIVNQQSCRISPIETVIEFQQKNSRLLEITREFSVNAGVTTPLSTYMLTNSELLSLINDMPITNDQKKLMSSNVQIVRQQSYSIMSIIKEEVLAYVVQLPIYGVIDTPCWKLHTSPLCTTNIKEGSNICLTRTDRGWYCDNAGSVSFFPQADTCKVQSNRVFCDTMNSLTLPPEVSLCNTDIFNSKYDCKIMTSKTDISSSVITSLGAIVSCYGKTKCTASNKNRGIIKTFSNGCDYVSNKGVDTVSVGNTLYYVNKLEGKNLYVKGEPIINYYDPLVFPSDEFDASISQVNEKINQSLAFIRRSDELL

SEQ ID NO: 79 - protein, 467 aa, synthetic construct
QNITEEFYQSTCSAVSRGYFSALRTGWYTSVITIELSNIKEPKCNGTDTKVKLIKQELDKYKNAVTELQLLMQSGGPGSGGGGSGGGGSRFPPFPLGVGSAIASGIAVSKVLHLPGEVNKIKNALLSTNKAVVSLSNGVSVLTSKVLDLKNYINNQLLPIVNQPSCRISNIETVIEFQQKNSRLLEITREFSVNAGVTTPLSTYMLTNSELLSLINDMPITNDQKKLMSSNVPIVRQQSYSIMSIIKEEVLAYVVQLPIYGVIDTPCWKLHTSPLCTTNIKEGSNICLTRTDRGWYCDNAGSVSFFPQADTCKVQSNRVFCDTMNSLTLPPEVSLCNTDIFNSKYDCKIMTSKTDISSSVITSLGAIVSCYGKTKCTASNKNRGIIKTFSNGCDYVSNKGVDTVSVGNTLYYVNKLEGKNLYVKGEPIINYYDPLVFPSDEFDASISQVNEKINQSLAFIRRSDELL

SEQ ID NO: 80 - protein, 467 aa, synthetic construct
QNITEEFYQSTCSAVSRGYFSALRTGWYTSVITIELSNIKEPKCNGTDTKVKLIKQELDKYKNAVTELQLLMQSGGPGSGGGGSGGGGSRFPPFPLGVGSAIASGIAVSKVLHLPGEVNKIKNALLSTNKAVVSLSNGVSVLTSKVLDLKNYINNQLLPIVNQQSCRPSNIETVIEFQQKNSRLLEITREFSVNAGVTTPLSTYMLTNSELLSLINDMPITNDQKKLMSSNVPIVRQQSYSIMSIIKEEVLAYVVQLPIYGVIDTPCWKLHTSPLCTTNIKEGSNICLTRTDRGWYCDNAGSVSFFPQADTCKVQSNRVFCDTMNSLTLPPEVSLCNTDIFNSKYDCKIMTSKTDISSSVITSLGAIVSCYGKTKCTASNKNRGIIKTFSNGCDYVSNKGVDTVSVGNTLYYVNKLEGKNLYVKGEPIINYYDPLVFPSDEFDASISQVNEKINQSLAFIRRSDELL

SEQ ID NO: 81 - protein, 467 aa, synthetic construct
QNITEEFYQSTCSAVSRGYFSALRTGWYTSVITIELSNIKEPKCNGTDTKVKLIKQELDKYKNAVTELQLLMQSGGPGSGGGGSGGGGSRFPPFPLGVGSAIASGIAVSKVLHLPGEVNKIKNALLSTNKAVVSLSNGVSVLTSKVLDLKNYINNQLLPIVNQQSCRIPNIETVIEFQQKNSRLLEITREFSVNAGVTTPLSTYMLTNSELLSLINDMPITNDQKKLMSSNVPIVRQQSYSIMSIIKEEVLAYVVQLPIYGVIDTPCWKLHTSPLCTTNIKEGSNICLTRTDRGWYCDNAGSVSFFPQADTCKVQSNRVFCDTMNSLTLPPEVSLCNTDIFNSKYDCKIMTSKTDISSSVITSLGAIVSCYGKTKCTASNKNRGIIKTFSNGCDYVSNKGVDTVSVGNTLYYVNKLEGKNLYVKGEPIINYYDPLVFPSDEFDASISQVNEKINQSLAFIRRSDELL

SEQ ID NO: 82 - protein, 467 aa, synthetic construct
QNITEEFYQSTCSAVSRGYFSALRTGWYTSVITIELSNIKEPKCNGTDTKVKLIKQELDKYKNAVTELQLLMQSGGPGSGGGGSGGGGSRFPPFPLGVGSAIASGIAVSKVLHLPGEVNKIKNALLSTNKAVVSLSNGVSVLTSKVLDLKNYINNQLLPIVNQQSCRIPPIETVIEFQQKNSRLLEITREFSVNAGVTTPLSTYMLTNSELLSLINDMPITNDQKKLMSSNVPIVRQQSYSIMSIIKEEVLAYVVQLPIYGVIDTPCWKLHTSPLCTTNIKEGSNICLTRTDRGWYCDNAGSVSFFPQADTCKVQSNRVFCDTMNSLTLPPEVSLCNTDIFNSKYDCKIMTSKTDISSSVITSLGAIVSCYGKTKCTASNKNRGIIKTFSNGCDYVSNKGVDTVSVGNTLYYVNKLEGKNLYVKGEPIINYYDPLVFPSDEFDASISQVNEKINQSLAFIRRSDELL

SEQ ID NO: 83 - protein, 467 aa, synthetic construct
QNITEEFYQSTCSAVSRGYFSALRTGWYTSVITIELSNIKEPKCNGTDTKVKLIKQELDKYKNAVTELQLLMQSGGPGSGGGGSGGGGSRFPPFPLGVGSAIASGIAVSKVLHLPGEVNKIKNALLSTNKAVVSLSNGVSVLTSKVLDLKNYINNQLLPIVNQPSCRISPIETVIEFQQKNSRLLEITREFSVNAGVTTPLSTYMLTNSELLSLINDMPITNDQKKLMSSNVPIVRQQSYSIMSIIKEEVLAYVVQLPIYGVIDTPCWKLHTSPLCTTNIKEGSNICLTRTDRGWYCDNAGSVSFFPQADTCKVQSNRVFCDTMNSLTLPPEVSLCNTDIFNSKYDCKIMTSKTDISSSVITSLGAIVSCYGKTKCTASNKNRGIIKTFSNGCDYVSNKGVDTVSVGNTLYYVNKLEGKNLYVKGEPIINYYDPLVFPSDEFDASISQVNEKINQSLAFIRRSDELL

SEQ ID NO: 84 - protein, 467 aa, synthetic construct
QNITEEFYQSTCSAVSRGYFSALRTGWYTSVITIELSNIKEPKCNGTDTKVKLIKQELDKYKNAVTELQLLMQSGGGGSGGGGSGGGGSRFPPFPLGVGSAIASGIAVSKVLHLPGEVNKIKNALLSTNKAVVSLSNGVSVLTSKVLDLKNYINNQLLPIVNQQSCRISNIETVIEFQQKNSRLLEITREFSVNAGVTTPLSTYMLTNSELLSLINDMPITNDQKKLMSSNVPIVRQQSYSIMSIIKEEVLAYVVQLPIYGVIDTPCWKLHTSPLCTTNIKEGSNICLTRTDRGWYCDNAGSVSFFPQADTCKVQSNRVFCDTMNSLTLPPEVSLCNTDIFNSKYDCKIMTSKTDISSSVITSLGAIVSCYGKTKCTASNKNRGIIKTFSNGCDYVSNKGVDTVSVGNTLYYVNKLEGKNLYVKGEPIINYYDPLVFPSDEFDASISQVNEKINQSLAFIRRSDELL

SEQ ID NO: 85 - protein, 467 aa, synthetic construct
QNITEEFYQSTCSAVSRGYFSALRTGWYTSVITIELSNIKEPKCNGTDTKVKLIKQELDKYKNAVTELQLLMQSGGGGSGGGGSGGGGSRFPPFPLGVGSAIASGIAVSKVLHLEGEVNKIKNALLSTNKAVVSLSNGVSVLTSKVLDLKNYINNQLLPIVNQQSCRISNIETVIEFQQKNSRLLEITREFSVNAGVTTPLSTYMLTNSELLSLINDMPITNDQKKLMSSNVPIVRQQSYSIMSIIKEEVLAYVVQLPIYGVIDTPCWKLHTSPLCTTNIKEGSNICLTRTDRGWYCDNAGSVSFFPQADTCKVQSNRVFCDTMNSLTLPPEVSLCNTDIFNSKYDCKIMTSKTDISSSVITSLGAIVSCYGKTKCTASNKNRGIIKTFSNGCDYVSNKGVDTVSVGNTLYYVNKLEGKNLYVKGEPIINYYDPLVFPSDEFDASISQVNEKINQSLAFIRRSDELL

SEQ ID NO: 86 - protein, 467 aa, synthetic construct
QNITEEFYQSTCSAVSRGYFSALRTGWYTSVITIELSNIKEPKCNGTDTKVKLIKQELDKYKNAVTELQLLMQSGGGGSGGGGSGGGGSRFPPFPLGVGSAIASGIAVSKVLHLPGEVNKIKNALLSTNKAVVSLSNGVSVLTSKVLDLKNYINNQLLPIVNQQSCRISPIETVIEFQQKNSRLLEITREFSVNAGVTTPLSTYMLTNSELLSLINDMPITNDQKKLMSSNVPIVRQQSYSIMSIIKEEVLAYVVQLPIYGVIDTPCWKLHTSPLCTTNIKEGSNICLTRTDRGWYCDNAGSVSFFPQADTCKVQSNRVFCDTMNSLTLPPEVSLCNTDIFNSKYDCKIMTSKTDISSSVITSLGAIVSCYGKTKCTASNKNRGIIKTFSNGCDYVSNKGVDTVSVGNTLYYVNKLEGKNLYVKGEPIINYYDPLVFPSDEFDASISQVNEKINQSLAFIRRSDELL

SEQ ID NO: 87 - protein, 467 aa, synthetic construct
QNITEEFYQSTCSAVSRGYFSALRTGWYTSVITIELSNIKEPKCNGTDTKVKLIKQELDKYKNAVTELQLLMQSGGGGSGGGGSGGGGSRFPPFPLGVGSAIASGIAVSKVLHLEGEVNKIKNALLSTNKAVVSLSNGVSVLTSKVLDLKNYINNQLLPIVNQQSCRISPIETVIEFQQKNSRLLEITREFSVNAGVTTPLSTYMLTNSELLSLINDMPITNDQKKLMSSNVPIVRQQSYSIMSIIKEEVLAYVVQLPIYGVIDTPCWKLHTSPLCTTNIKEGSNICLTRTDRGWYCDNAGSVSFFPQADTCKVQSNRVFCDTMNSLTLPPEVSLCNTDIFNSKYDCKIMTSKTDISSSVITSLGAIVSCYGKTKCTASNKNRGIIKTFSNGCDYVSNKGVDTVSVGNTLYYVNKLEGKNLYVKGEPIINYYDPLVFPSDEFDASISQVNEKINQSLAFIRRSDELL

SEQ ID NO: 88 - protein, 467 aa, synthetic construct
QNITEEFYQSTCSAVSRGYFSALRTGWYTSVITIELSNIKEPKCNGTDTKVKLIKQELDKYKNAVTELQLLMQSGGGGSPGGGSGGGGSRFLGFPLGVGSAIASGIAVSKVLHLEGEVNKIKNALLSTNKAVVSLSNGVSVLTSKVLDLKNYINNQLLPIVNQQSCRISPIETVIEFQQKNSRLLEITREFSVNAGVTTPLSTYMLTNSELLSLINDMPITNDQKKLMSSNVPIVRQQSYSIMSIIKEEVLAYVVQLPIYGVIDTPCWKLHTSPLCTTNIKEGSNICLTRTDRGWYCDNAGSVSFFPQADTCKVQSNRVFCDTMNSLTLPPEVSLCNTDIFNSKYDCKIMTSKTDISSSVITSLGAIVSCYGKTKCTASNKNRGIIKTFSNGCDYVSNKGVDTVSVGNTLYYVNKLEGKNLYVKGEPIINYYDPLVFPSDEFDASISQVNEKINQSLAFIRRSDELL

SEQ ID NO: 89 - protein, 467 aa, synthetic construct
QNITEEFYQSTCSAVSRGYFSALRTGWYTSVITIELSNIKEPKCNGTDTKVKLIKQELDKYKNAVTELQLLMQSGGGGPGGGGSGGGGSRFPPFLLGVGSAIASGIAVSKVLHLEGEVNKIKNALLSTNKAVVSLSNGVSVLTSKVLDLKNYINNQLLPIVNQQSCRISPIETVIEFQQKNSRLLEITREFSVNAGVTTPLSTYMLTNSELLSLINDMPITNDQKKLMSSNVPIVRQQSYSIMSIIKEEVLAYVVQLPIYGVIDTPCWKLHTSPLCTTNIKEGSNICLTRTDRGWYCDNAGSVSFFPQADTCKVQSNRVFCDTMNSLTLPPEVSLCNTDIFNSKYDCKIMTSKTDISSSVITSLGAIVSCYGKTKCTASNKNRGIIKTFSNGCDYVSNKGVDTVSVGNTLYYVNKLEGKNLYVKGEPIINYYDPLVFPSDEFDASISQVNEKINQSLAFIRRSDELL

SEQ ID NO: 90 - protein, 467 aa, synthetic construct
QNITEEFYQSTCSAVSRGYFSALRTGWYTSVITIELSNIKEPKCNGTDTKVKLIKQELDKYKNAVTELQLLMQSGGGGSGGGPSGGGGSRFPPFPLGVGSAIASGIAVSKVLHLEGEVNKIKNALLSTNKAVVSLSNGVSVLTSKVLDLKNYINNQLLPIVNQQSCRISPIETVIEFQQKNSRLLEITREFSVNAGVTTPLSTYMLTNSELLSLINDMPITNDQKKLMSSNVPIVRQQSYSIMSIIKEEVLAYVVQLPIYGVIDTPCWKLHTSPLCTTNIKEGSNICLTRTDRGWYCDNAGSVSFFPQADTCKVQSNRVFCDTMNSLTLPPEVSLCNTDIFNSKYDCKIMTSKTDISSSVITSLGAIVSCYGKTKCTASNKNRGIIKTFSNGCDYVSNKGVDTVSVGNTLYYVNKLEGKNLYVKGEPIINYYDPLVFPSDEFDASISQVNEKINQSLAFIRRSDELL

SEQ ID NO: 91 - protein, 488 aa, synthetic construct
QNITEEFYQSTCSAVSRGYFSALRTGWYTSVITIELSNIKEPKCNGTDTKVKLIKQELDKYKNAVTELQLLMQNTPAANNRARREAPQYMNYTINTTKNLNVSISKKRKRRFLGFLLGVGSAIASGIAVSKVLHLPGEVNKIKNALLSTNKAVVSLSNGVSVLTSKVLDLKNYINNQLLPIVNQQSCRISNIETVIEFQQKNSRLLEITREFSVNAGVTTPLSTYMLTNSELLSLINDMPITNDQKKLMSSNVPIVRQQSYSIMSIIKEEVLAYVVQLPIYGVIDTPCWKLHTSPLCTTNIKEGSNICLTRTDRGWYCDNAGSVSFFPQADTCKVQSNRVFCDTMNSLTLPPEVSLCNTDIFNSKYDCKIMTSKTDISSSVITSLGAIVSCYGKTKCTASNKNRGIIKTFSNGCDYVSNKGVDTVSVGNTLYYVNKLEGKNLYVKGEPIINYYDPLVFPSDEFDASISQVNEKINQSLAFIRRSDELL

SEQ ID NO: 92 - protein, 488 aa, synthetic construct
QNITEEFYQSTCSAVSRGYFSALRTGWYTSVITIELSNIKEPKCNGTDTKVKLIKQELDKYKNAVTELQLLMQNTPAANNRARREAPQYMNYTINTTKNLNVSISKKRKRRFLGFLLGVGSAIASGIAVSKVLHLPGEVNKIKNALLSTNKAVVSLSNGVSVLTSKVLDLKNYINNQLLPIVNQQSCRISPIETVIEFQQKNSRLLEITREFSVNAGVTTPLSTYMLTNSELLSLINDMPITNDQKKLMSSNVPIVRQQSYSIMSIIKEEVLAYVVQLPIYGVIDTPCWKLHTSPLCTTNIKEGSNICLTRTDRGWYCDNAGSVSFFPQADTCKVQSNRVFCDTMNSLTLPPEVSLCNTDIFNSKYDCKIMTSKTDISSSVITSLGAIVSCYGKTKCTASNKNRGIIKTFSNGCDYVSNKGVDTVSVGNTLYYVNKLEGKNLYVKGEPIINYYDPLVFPSDEFDASISQVNEKINQSLAFIRRSDELL

SEQ ID NO: 93 - protein, 488 aa, synthetic construct
QNITEEFYQSTCSAVSRGYFSALRTGWYTSVITIELSNIKEPKCNGTDTKVKLIKQELDKYKNAVTELQLLMQNTPAANNRARREAPQYMNYTINTTKNLNVSISKKRKRRFLGFPLGVGSAIASGIAVSKVLHLPGEVNKIKNALLSTNKAVVSLSNGVSVLTSKVLDLKNYINNQLLPIVNQQSCRISPIETVIEFQQKNSRLLEITREFSVNAGVTTPLSTYMLTNSELLSLINDMPITNDQKKLMSSNVPIVRQQSYSIMSIIKEEVLAYVVQLPIYGVIDTPCWKLHTSPLCTTNIKEGSNICLTRTDRGWYCDNAGSVSFFPQADTCKVQSNRVFCDTMNSLTLPPEVSLCNTDIFNSKYDCKIMTSKTDISSSVITSLGAIVSCYGKTKCTASNKNRGIIKTFSNGCDYVSNKGVDTVSVGNTLYYVNKLEGKNLYVKGEPIINYYDPLVFPSDEFDASISQVNEKINQSLAFIRRSDELL

SEQ ID NO: 94 - protein, 488 aa, synthetic construct
QNITEEFYQSTCSAVSRGYFSALRTGWYTSVITIELSNIKEPKCNGTDTKVKLIKQELDKYKNAVTELQLLMQNTPAANNGSASEAPQYMNYTINTTKNLNVSISKKGKGRFLGFLLGVGSAIASGIAVSKVLHLPGEVNKIKNALLSTNKAVVSLSNGVSVLTSKVLDLKNYINNQLLPIVNQQSCRISNIETVIEFQQKNSRLLEITREFSVNAGVTTPLSTYMLTNSELLSLINDMPITNDQKKLMSSNVPIVRQQSYSIMSIIKEEVLAYVVQLPIYGVIDTPCWKLHTSPLCTTNIKEGSNICLTRTDRGWYCDNAGSVSFFPQADTCKVQSNRVFCDTMNSLTLPPEVSLCNTDIFNSKYDCKIMTSKTDISSSVITSLGAIVSCYGKTKCTASNKNRGIIKTFSNGCDYVSNKGVDTVSVGNTLYYVNKLEGKNLYVKGEPIINYYDPLVFPSDEFDASISQVNEKINQSLAFIRRSDELL

SEQ ID NO: 95 - protein, 488 aa, synthetic construct
QNITEEFYQSTCSAVSRGYFSALRTGWYTSVITIELSNIKEPKCNGTDTKVKLIKQELDKYKNAVTELQLLMQNTPAANNGSASEAPQYMNYTINTTKNLNVSISKKGKGRFLGFLLGVGSAIASGIAVSKVLHLPGEVNKIKNALLSTNKAVVSLSNGVSVLTSKVLDLKNYINNQLLPIVNQQSCRISPIETVIEFQQKNSRLLEITREFSVNAGVTTPLSTYMLTNSELLSLINDMPITNDQKKLMSSNVPIVRQQSYSIMSIIKEEVLAYVVQLPIYGVIDTPCWKLHTSPLCTTNIKEGSNICLTRTDRGWYCDNAGSVSFFPQADTCKVQSNRVFCDTMNSLTLPPEVSLCNTDIFNSKYDCKIMTSKTDISSSVITSLGAIVSCYGKTKCTASNKNRGIIKTFSNGCDYVSNKGVDTVSVGNTLYYVNKLEGKNLYVKGEPIINYYDPLVFPSDEFDASISQVNEKINQSLAFIRRSDELL

SEQ ID NO: 96 - protein, 488 aa, synthetic construct
QNITEEFYQSTCSAVSRGYFSALRTGWYTSVITIELSNIKEPKCNGTDTKVKLIKQELDKYKNAVTELQLLMQNTPAANNGSASEAPQYMNYTINTTKNLNVSISKKGKGRFLGFPLGVGSAIASGIAVSKVLHLPGEVNKIKNALLSTNKAVVSLSNGVSVLTSKVLDLKNYINNQLLPIVNQQSCRISPIETVIEFQQKNSRLLEITREFSVNAGVTTPLSTYMLTNSELLSLINDMPITNDQKKLMSSNVPIVRQQSYSIMSIIKEEVLAYVVQLPIYGVIDTPCWKLHTSPLCTTNIKEGSNICLTRTDRGWYCDNAGSVSFFPQADTCKVQSNRVFCDTMNSLTLPPEVSLCNTDIFNSKYDCKIMTSKTDISSSVITSLGAIVSCYGKTKCTASNKNRGIIKTFSNGCDYVSNKGVDTVSVGNTLYYVNKLEGKNLYVKGEPIINYYDPLVFPSDEFDASISQVNEKINQSLAFIRRSDELL

SEQ ID NO: 97 - protein, 449 aa, synthetic construct
QNITEEFYQSTCSAVSRGYFSALRTGWYTSVITIELSNIKEPKCNGTDTKVKLIKQELDKYKNAVTELQLLMQSTPATGSGSAIASGIAVSKVLHLEGEVNKIKNALLSTNKAVVSLSNGVSVLTSKVLDLKNYINNQLLPIVNQQSCRISNIETVIEFQQKNSRLLEITREFSVNAGVTTPLSTYMLTNSELLSLINDMPITNDQKKLMSSNVPIVRQQSYSIMSIIKEEVLAYVVQLPIYGVIDTPCWKLHTSPLCTTNIKEGSNICLTRTDRGWYCDNAGSVSFFPQADTCKVQSNRVFCDTMNSLTLPPEVSLCNTDIFNSKYDCKIMTSKTDISSSVITSLGAIVSCYGKTKCTASNKNRGIIKTFSNGCDYVSNKGVDTVSVGNTLYYVNKLEGKNLYVKGEPIINYYDPLVFPSDEFDASISQVNEKINQSLAFIRRSDELL

SEQ ID NO: 98 - protein, 449 aa, synthetic construct
QNITEEFYQSTCSAVSRGYFSALRTGWYTSVITIELSNIKEPKCNGTDTKVKLIKQELDKYKNAVTELQLLMQSTPATGSGSAIASGIAVSKVLHLEGEVNKIKNALLSTNKAVVSLSNGVSVLTSKVLDLKNYINNQLLPIVNQQSCRISPIETVIEFQQKNSRLLEITREFSVNAGVTTPLSTYMLTNSELLSLINDMPITNDQKKLMSSNVPIVRQQSYSIMSIIKEEVLAYVVQLPIYGVIDTPCWKLHTSPLCTTNIKEGSNICLTRTDRGWYCDNAGSVSFFPQADTCKVQSNRVFCDTMNSLTLPPEVSLCNTDIFNSKYDCKIMTSKTDISSSVITSLGAIVSCYGKTKCTASNKNRGIIKTFSNGCDYVSNKGVDTVSVGNTLYYVNKLEGKNLYVKGEPIINYYDPLVFPSDEFDASISQVNEKINQSLAFIRRSDELL

SEQ ID NO: 99 - protein, 449 aa, synthetic construct
QNITEEFYQSTCSAVSRGYFSALRTGWYTSVITIELSNIKEPKCNGTDTKVKLIKQELDKYKNAVTELQLLMQSTPATGSGSAIASGIAVSKVLHLPGEVNKIKNALLSTNKAVVSLSNGVSVLTSKVLDLKNYINNQLLPIVNQQSCRISPIETVIEFQQKNSRLLEITREFSVNAGVTTPLSTYMLTNSELLSLINDMPITNDQKKLMSSNVPIVRQQSYSIMSIIKEEVLAYVVQLPIYGVIDTPCWKLHTSPLCTTNIKEGSNICLTRTDRGWYCDNAGSVSFFPQADTCKVQSNRVFCDTMNSLTLPPEVSLCNTDIFNSKYDCKIMTSKTDISSSVITSLGAIVSCYGKTKCTASNKNRGIIKTFSNGCDYVSNKGVDTVSVGNTLYYVNKLEGKNLYVKGEPIINYYDPLVFPSDEFDASISQVNEKINQSLAFIRRSDELL

SEQ ID NO: 100 - protein, 466 aa, synthetic construct
QNITEEFYQSTCSAVSRGYFSALRTGWYTSVITIELSNIKEPKCNGTDTKVKLIKQELDKYKNAVTELQLLMQNTPAANNRARGSGSGRSLGFLLGVGSAIASGIAVSKVLHLEGEVNKIKNALLSTNKAVVSLSNGVSVLTSKVLDLKNYINNQLLPIVNQQSCRISPIETVIEFQQKNSRLLEITREFSVNAGVTTPLSTYMLTNSELLSLINDMPITNDQKKLMSSNVPIVRQQSYSIMSIIKEEVLAYVVQLPIYGVIDTPCWKLHTSPLCTTNIKEGSNICLTRTDRGWYCDNAGSVSFFPQADTCKVQSNRVFCDTMNSLTLPPEVSLCNTDIFNSKYDCKIMTSKTDISSSVITSLGAIVSCYGKTKCTASNKNRGIIKTFSNGCDYVSNKGVDTVSVGNTLYYVNKLEGKNLYVKGEPIINYYDPLVFPSDEFDASISQVNEKINQSLAFIRRSDELL

SEQ ID NO: 101 - protein, 466 aa, synthetic construct
QNITEEFYQSTCSAVSRGYFSALRTGWYTSVITIELSNIKEPKCNGTDTKVKLIKQELDKYKNAVTELQLLMQNTPAANNRARGSGSGRSLGFLLGVGSAIASGIAVSKVLHLPGEVNKIKNALLSTNKAVVSLSNGVSVLTSKVLDLKNYINNQLLPIVNQQSCRISPIETVIEFQQKNSRLLEITREFSVNAGVTTPLSTYMLTNSELLSLINDMPITNDQKKLMSSNVPIVRQQSYSIMSIIKEEVLAYVVQLPIYGVIDTPCWKLHTSPLCTTNIKEGSNICLTRTDRGWYCDNAGSVSFFPQADTCKVQSNRVFCDTMNSLTLPPEVSLCNTDIFNSKYDCKIMTSKTDISSSVITSLGAIVSCYGKTKCTASNKNRGIIKTFSNGCDYVSNKGVDTVSVGNTLYYVNKLEGKNLYVKGEPIINYYDPLVFPSDEFDASISQVNEKINQSLAFIRRSDELL

SEQ ID NO: 102 - protein, 449 aa, synthetic construct
QNITEEFYQSTCSAVSRGYFSALRTGWYTSVITIELSNIKEPKCNGTDTKVKLIKQELDKYKNAVTELQLLMFLGFPLGVGSAIASGIAVSKVLHLEGEVNKIKNALLSTNKAVVSLSNGVSVLTSKVLDLKNYINNQLLPIVNQQSCRISNIETVIEFQQKNSRLLEITREFSVNAGVTTPLSTYMLTNSELLSLINDMPITNDQKKLMSSNVPIVRQQSYSIMSIIKEEVLAYVVQLPIYGVIDTPCWKLHTSPLCTTNIKEGSNICLTRTDRGWYCDNAGSVSFFPQADTCKVQSNRVFCDTMNSLTLPPEVSLCNTDIFNSKYDCKIMTSKTDISSSVITSLGAIVSCYGKTKCTASNKNRGIIKTFSNGCDYVSNKGVDTVSVGNTLYYVNKLEGKNLYVKGEPIINYYDPLVFPSDEFDASISQVNEKINQSLAFIRRSDELL

SEQ ID NO: 103 - protein, 449 aa, synthetic construct
QNITEEFYQSTCSAVSRGYFSALRTGWYTSVITIELSNIKEPKCNGTDTKVKLIKQELDKYKNAVTELQLLMFLGFPLGVGSAIASGIAVSKVLHLEGEVNKIKNALLSTNKAVVSLSNGVSVLTSKVLDLKNYINNQLLPIVNQQSCRISPIETVIEFQQKNSRLLEITREFSVNAGVTTPLSTYMLTNSELLSLINDMPITNDQKKLMSSNVPIVRQQSYSIMSIIKEEVLAYVVQLPIYGVIDTPCWKLHTSPLCTTNIKEGSNICLTRTDRGWYCDNAGSVSFFPQADTCKVQSNRVFCDTMNSLTLPPEVSLCNTDIFNSKYDCKIMTSKTDISSSVITSLGAIVSCYGKTKCTASNKNRGIIKTFSNGCDYVSNKGVDTVSVGNTLYYVNKLEGKNLYVKGEPIINYYDPLVFPSDEFDASISQVNEKINQSLAFIRRSDELL

SEQ ID NO: 104 - protein, 449 aa, synthetic construct
QNITEEFYQSTCSAVSRGYFSALRTGWYTSVITIELSNIKEPKCNGTDTKVKLIKQELDKYKNAVTELQLLMFLGFPLGVGSAIASGIAVSKVLHLPGEVNKIKNALLSTNKAVVSLSNGVSVLTSKVLDLKNYINNQLLPIVNQQSCRISPIETVIEFQQKNSRLLEITREFSVNAGVTTPLSTYMLTNSELLSLINDMPITNDQKKLMSSNVPIVRQQSYSIMSIIKEEVLAYVVQLPIYGVIDTPCWKLHTSPLCTTNIKEGSNICLTRTDRGWYCDNAGSVSFFPQADTCKVQSNRVFCDTMNSLTLPPEVSLCNTDIFNSKYDCKIMTSKTDISSSVITSLGAIVSCYGKTKCTASNKNRGIIKTFSNGCDYVSNKGVDTVSVGNTLYYVNKLEGKNLYVKGEPIINYYDPLVFPSDEFDASISQVNEKINQSLAFIRRSDELL

SEQ ID NO: 105 - DNA, 1401 bp, synthetic construct
  source 1..1401: mol_type = other DNA
cagaacatcaccgaggagttctaccagagcacctgcagcgctgtgtctagaggctacttcagcgcccttagaaccggctggtacaccagcgtgatcaccatcgagctctccaatatcaaagaacctaagtgcaacggtacagatacgaaggtgaagctgatcaagcaggagctggataagtacaagaacgccgtgacagagttgcagctgctgatgcagagcggcggacctggcagcggcggaggcggaagcggcggcggcggctctagattcctgggcttcctgctcggcgtgggcagcgctattgccagcggcatcgccgtgtccaaggtgctgcacctggaaggcgaggtgaacaagatcaaaaatgccctgctgagcacaaacaaggccgtggtgagcctgagcaatggcgtctccgtgctgacaagcaaagttctggacctgaagaactacatcaacaaccagctgctgcctattgtgaaccagcaaagctgtagaatcagcaacatcgagacagtgatcgaatttcagcagaaaaacagccggctgctggaaatcacaagagagttctccgtgaatgccggcgtcaccacaccactgtctacatacatgctgaccaattctgagctgctgagcctgatcaatgacatgcctatcaccaacgaccagaagaagctgatgagctccaacgtgcagatcgtgcggcagcagagctacagcatcatgagcatcatcaaggaggaagtgctcgcctacgtcgtgcaactgcccatctacggagtcatcgacacaccttgttggaagctgcacaccagccccctgtgtaccaccaacatcaaggaaggctctaacatctgcctgacccggaccgatagaggctggtattgtgacaacgctggcagcgtgtccttcttccctcaggccgatacatgcaaggtgcagtctaacagagtgttctgcgacaccatgaacagcctgacactgcctagcgaggtgagcctgtgcaacaccgatatcttcaacagcaagtacgactgcaaaatcatgaccagcaaaaccgacatcagcagcagcgtcatcacctctctgggcgccatcgtgagttgctacggcaagaccaagtgcaccgcctctaataagaaccggggcatcatcaagacttttagcaacggctgcgactacgtgtctaacaagggcgtggacaccgtgtccgtgggaaataccctgtactacgtgaacaaactggaaggaaagaacctgtacgtgaaaggagagcccatcatcaattattacgaccccctggtgtttccatctgatgagttcgacgccagcatctctcaggtgaacgagaagattaaccaaagcctggccttcatcagaaggtccgacgagctgctg

SEQ ID NO: 106 - DNA, 1401 bp, synthetic construct
  source 1..1401: mol_type = other DNA
caaaacatcaccgaggagttctaccagagtacctgtagcgccgttagcagaggttatttcagcgctctgcggacaggctggtatacaagcgtgattacaatcgagctgagcaacatcaaggagacaaagtgcaacggcaccgatacaaaggtcaaactgatcaagcaggagctggataagtacaagaacgctgtgacagagctgcagctgctgatgcagagcggaggacctggcagcggcggcggcggatctggcggcggaggctctaggttcctgggcttccctctgggcgttggaagcgccatcgccagcggcatcgccgtgtctaaggtgctgcacctggaaggcgaggtgaacaaaatcaagaacgccctcctgagcaccaacaaggccgtggtgtccctttctaatggcgtgtccgtgctgacctctaaggtgctggacctgaagaactacatcaacaaccagctgctgcctatcgtgaatcaacagagctgcagaatctccaacattgaaaccgtgattgagtttcagcagaaaaatagcagactgctggaaatcacccgggaattttctgtgaacgccggcgtgaccacccctctgagcacctacatgctgaccaacagcgaactgctgtccctgatcaacgatatgcctatcaccaacgaccagaagaagctgatgagcagcaacgtgcaaatcgtgcggcagcagtcctacagcatcatgagcatcatcaaggaagaggtgctggcctacgtggtccagctgcctatctacggcgtgatcgacacaccatgttggaagctgcacaccagccctctgtgcacaacaaacatcaaagagggcagcaatatctgcctgacaagaacagatagaggctggtactgcgacaacgctggcagcgtctccttcttcccccaggccgacacttgcaaggtccagagcaacagagtgttctgcgacaccatgaacagcctcacactgcctagcgaggtgagcctgtgtaataccgacatcttcaactctaaatacgactgcaagatcatgacctccaagaccgacatctctagcagcgtgatcacatctctgggcgccatcgtttcttgctacggaaagaccaagtgcaccgcctctaacaagaatagaggcatcatcaaaacctttagcaatggctgtgactacgtgtccaataaaggcgtggacaccgtgagcgtgggcaacaccctgtactacgtgaacaagctggaaggcaagaacctgtacgtgaagggagaacccatcatcaactactacgatcccctggtgttccccagcgacgagttcgacgccagcatcagccaggtgaacgagaagatcaaccagtctctggccttcattagacggagcgatgagctgctc

SEQ ID NO: 107 - DNA, 1401 bp, synthetic construct
  source 1..1401: mol_type = other DNA
cagaacatcaccgaggagttctaccagtctacctgttctgctgtgtccagaggctacttcagcgccctgagaaccggctggtacaccagcgtgatcaccatcgagctgagcaacatcaaggaaaccaagtgcaacggcaccgatacaaaggtcaagctgatcaagcaggagctggataagtacaagaacgccgttacagagctgcagctgctgatgcagagcggcggacctggcagcggaggcggcggcagcggcggcggaggcagcaggtttctgggcttcctgctgggagtgggtagcgctatcgcctctggcatcgccgtctccaaggtgctgcacctggaaggcgaagtaaacaagatcaagaacgccctgcttagcactaacaaggccgtggtcagcctgagcaatggcgtgagtgtgctgacctccaaagtgctggacctgaagaattacatcaacaaccagctgctgccaattgtgaaccagcaaagctgcagaatcagcaatatcgagacagtgattgagtttcagcagaaaaacagcagactgctggaaatcacccgggaattttctgtgaacgccggagtgaccacccctctgtccacctacatgctgacaaattctgagctgctgagcctgatcaacgacatgcctatcaccaatgaccagaagaagctgatgagctccaacgtgcccatcgtgcggcagcaaagctacagcatcatgtcaatcatcaaagaggaagtgctggcttatgtggtgcagctgcctatctacggcgtgatcgacaccccatgttggaagctgcacaccagccccctgtgtaccacaaacatcaaggagggaagcaacatctgcctgacaagaacagatagaggctggtactgcgacaacgctggctctgtcagcttcttccctcaggccgatacctgcaaggtgcagagcaaccgggtgttctgcgacacaatgaacagcctgaccctgcctagcgaggttagcctctgtaataccgacatcttcaacagcaaatatgactgcaagatcatgaccagcaagacagatatcagcagctctgtgatcacatctctgggcgccatcgtgtcctgctacggaaagaccaagtgcaccgccagcaataaaaacagaggaatcatcaagaccttcagcaacggctgcgactacgtgtctaacaaaggcgtggacacagtgtccgtgggcaacaccctgtactacgtgaacaaactggaaggcaagaacctgtacgtgaagggcgagcctatcattaactactacgaccccctcgtgttccccagcgacgagttcgacgccagcatttctcaggtgaacgagaagatcaatcaaagcctggccttcatccggagaagcgatgagctgctg

SEQ ID NO: 108 - DNA, 1401 bp, synthetic construct
  source 1..1401: mol_type = other DNA
cagaacatcaccgaggaattttaccagagcacctgcagcgccgtgtctagaggctacttcagcgccctgcggaccggctggtacaccagcgtgatcacaatcgagctgagcaacatcaaggaaaccaagtgcaacggcaccgataccaaggttaagctgatcaagcaggagctggataagtacaagaacgctgtgaccgagctgcagctgctgatgcagagcggcggacctggcagcggcggaggtggctctggaggcggcggaagcagattcctgggcttcctgctgggagtgggaagcgccatcgccagcggcatcgccgtgtccaaagtgctccacctggaaggcgaggttaacaagataaagaacgcgctgctgtctacaaacaaggccgtggtgtctctgtccaatggcgtgtctgtgctgaccagcaaagtgctggacctgaagaactacatcaacaaccagctgctgcctattgtgaaccaacaatcttgtagaatcagcaacatcgagacggtgattgagtttcagcagaagaacagccggctgctggaaatcactcgggagttcagcgtgaatgctggcgtcaccacccctctgagcacatacatgctgacaaatagcgagctgctcagcctcatcaacgacatgcctatcaccaatgatcagaaaaagctgatgagctccaacgtgcagatcgtgcggcagcagtcatatagcatcatgagcatcatcaaggaagaggtgctggcctacgtcgtgcaactgccaatctacggcgtgatcgacaccccttgctggaagctgcacacaagccctctgtgcacaacaaacatcaaagagggcagcaatatctgcctgaccagaaccgacagaggatggtattgcgacaacgccggctccgtgtccttcttcccccaggccgacacatgcaaagttcagagcaacagagtgttctgcgataccatgaacagccttacactgccccccgaggtgtccctgtgtaacacagacatcttcaacagcaagtacgactgcaagatcatgaccagcaagaccgacatctctagcagcgtgattacaagcctgggcgccatcgtgagttgttacggcaagacaaagtgcaccgccagcaacaagaatagaggcatcatcaagaccttcagcaatggctgtgactacgtgtccaacaaaggcgtggacaccgtgagtgtcggcaacaccctgtactacgtgaacaaactggaaggcaaaaacctgtacgtgaagggcgaacccatcatcaactactacgatcctctggtgttcccatctgatgagttcgacgcctctatcagccaggtgaacgagaagatcaatcagagcctggcttttatcaggagaagcgacgagctgctg

SEQ ID NO: 109 - DNA, 1401 bp, synthetic construct
  source 1..1401: mol_type = other DNA
cagaacatcaccgaggaattttaccagagcacctgtagcgccgtgtcccgcggctacttcagcgccctgagaacaggctggtataccagcgtgatcacaatcgagctgtctaatatcaaggagcctaagtgcaacggcacagataccaaggtgaaactgatcaaacaggagctggataagtacaagaacgccgtcaccgagctgcagctgctgatgcagtccggaggccctggatctggcgggggcggcagcggcggaggcggaagcagattcctgggcttccctctgggcgtcggcagcgccatcgcctctggcatcgccgtgtctaaggtgctgcacctggaaggagaagttaacaaaatcaagaatgccctgctcagcaccaacaaggccgtggtgagcctgagcaacggagtatccgtgctgaccagcaaagtgctggacctgaagaactacatcaacaaccagctgctgcccattgtgaaccaacaaagctgtaggatcagcaatatcgagacagtgattgagtttcagcagaagaactcccggctgctggaaatcaccagagagttcagcgttaacgccggcgtgaccacaccactgagcacatacatgctgaccaacagcgagctcctcagcctgatcaacgacatgcctatcacaaatgaccagaagaagctgatgagctctaacgtgcagatcgtgcggcagcagagctacagcatcatgagcatcatcaaggaggaagtgctggcttatgttgtgcagctgcctatctacggcgtgatcgacacgccctgctggaagctgcacacctctcctctgtgcacaaccaacatcaaagaaggctctaatatctgcctgacaagaaccgatagaggctggtactgcgacaacgctggctccgtgtcattcttcccccaggctgacacctgcaaagtgcaatctaacagagtgttctgcgataccatgaacagcctgacactgccatctgaggtgtccctgtgtaataccgacatcttcaacagcaaatacgactgcaagatcatgacctccaagaccgacatcagcagcagcgtgatcacaagcctgggcgccatcgtgtcttgctacggcaagaccaagtgcaccgccagcaacaagaaccggggcatcatcaagaccttcagcaacggctgtgactacgtcagcaataaaggcgtggacacagtgtccgtgggcaacaccctgtactacgtgaacaagctggaaggcaagaacctgtacgtgaagggcgagcctattatcaactactacgatcctctggtgttccccagcgatgagttcgacgccagcatctctcaggtgaatgagaagatcaatcagagcctggcctttatccggagaagcgacgaactgctt

SEQ ID NO: 110 - DNA, 1401 bp, synthetic construct
  source 1..1401: mol_type = other DNA
cagaacatcacagaggagttctaccagtctacctgcagcgccgtcagccggggctacttcagcgccctgagaaccggctggtacacctccgtgatcacaatcgagctgtccaatatcaaagaaaccaagtgcaacggaacagatacaaaggtgaagctgatcaagcaggagctggacaagtataagaacgccgtgaccgagctgcagctgctcatgcagagcggcggacctggcagcggcgggggcggcagcggcggcggaggatctagattcctgggctttccactgggcgtgggcagcgccatcgcttctggcatcgccgtgtccaaggtgctccacctggaaggggaggtgaacaagatcaagaacgccctgctgagcaccaacaaggccgtggtgtctctgtccaatggcgtaagcgtgctaaccagcaaagtgctggacctgaagaactacatcaataaccagctgctgcccattgtgaaccagcagtcctgcagaatcagcaacattgagacagtgatcgagtttcagcaaaagaacagccggctgctggaaatcaccagggagttcagcgtcaacgccggcgtgacaacccctctgtctacatacatgctgacaaacagcgagctgctgagcctgatcaacgacatgcctattacaaatgatcagaaaaagctgatgagctctaatgtgcccatcgtgcggcagcagtcttattctatcatgtccatcatcaaggaggaagtgctggcttacgtggtccaactgcctatctacggcgtgatcgacaccccttgttggaagctgcacacttcacctctctgtaccaccaacatcaaagagggctctaatatctgcctgaccagaaccgacagaggctggtactgcgacaacgctggcagcgtctccttcttccctcaggccgatacatgtaaagtgcagagcaatagagtgttctgcgataccatgaacagcctgacactgccaagcgaggtgagcctgtgcaacaccgatatcttcaacagcaagtacgactgcaagatcatgacgagcaaaaccgacatctccagcagcgtgatcaccagcctcggcgccatcgtgtcttgctacggcaagaccaagtgcaccgccagcaacaagaaccggggcatcatcaagaccttcagcaacggttgtgactacgtgtctaacaaaggcgtggacaccgtgagcgtgggaaataccctgtactacgtgaacaagctggaaggaaagaacctgtacgttaagggcgaacctatcatcaactactacgaccccctggtgtttcccagcgacgagttcgacgccagcatcagccaggtgaacgaaaagatcaaccaaagcctggccttcatcagaagatccgatgagctgctg

SEQ ID NO: 111 - DNA, 1401 bp, synthetic construct
  source 1..1401: mol_type = other DNA
cagaacatcacggaagagttctaccagagcacatgcagcgccgtgagcagaggatacttcagcgccctgagaaccggctggtatacaagcgtcatcacaatcgagctgtctaatatcaaggagacaaaatgcaacggcaccgacaccaaggtgaagctgattaagcaggagctggataagtacaagaacgctgtgacagagttgcagctgctgatgcagtctggtggacctggctccggcggcggcggcagcggcggaggcggaagcagattcctgggcttccccctgggcgtgggcagcgctatcgccagcggcatcgctgtgtctaaggtgctgcacctggaaggcgaggtgaacaagatcaagaatgccctgctgagcaccaacaaggccgtcgtgtctctgagcaacggcgtgtccgtgctgacaagcaaggtgctggacctgaagaactacatcaacaaccagctgctgcccatcgtcaatcagcagagctgcagaatctctaacatcgaaaccgtgatcgagtttcagcaaaagaactctagactgctggaaatcactcgggaatttagcgtgaacgctggcgttacaacccctctctctacatacatgctgacaaacagcgagcttctgagcctgatcaatgatatgcctatcaccaacgaccagaaaaagctgatgagcagcaacgtgcagatcgtgcggcagcaaagctacagcatcatgagcatcatcaaagaggaagtgctggcctacgtggtgcagctgcctatctacggcgtgatcgacaccccatgctggaagctgcacaccagccccctgtgcaccaccaacattaaggaaggcagcaacatctgcctgaccagaaccgatagaggctggtactgcgacaacgccggatcggttagcttcttccctcaggccgacacctgtaaagtgcaatccaaccgggtgttctgcgacaccatgaacagcctgaccctgccacctgaggtgtccctatgtaacacagacatcttcaacagcaagtatgattgcaagatcatgacctctaagaccgacatcagctccagcgtgatcacctccctgggcgccatcgtgtcttgttacggcaaaacaaagtgcaccgccagtaacaagaacagaggcattatcaagaccttcagcaatggctgtgattacgtgtctaacaaaggcgtggacacagtgtctgtgggaaataccctgtactacgtgaacaagctggaaggcaagaatctgtacgtgaaaggagagcctatcatcaactactacgaccccctggtgtttcctagcgacgagttcgacgcctccatcagccaggtgaatgagaagatcaaccagtccctggccttcattaggcggagcgatgagctgctg

SEQ ID NO: 112 - DNA, 1401 bp, synthetic construct
  source 1..1401: mol_type = other DNA
cagaacatcacagaggagttctaccagagcacctgcagcgccgtgagccggggctacttctctgctctgagaaccggctggtacaccagcgtgatcacaatcgagctgagcaatatcaaggaacccaagtgcaacggcaccgacacgaaggtgaagctgatcaagcaggagctggataagtacaagaacgctgttacagagctgcagctgctgatgcagagcggcggtcctggctcaggcggaggcggcagcggcggcggcggaagcagattcctgggatttctgctgggcgtgggcagcgctatcgccagcggcatcgccgtgagcaaggtgctgcacctggaaggcgaggtgaacaagatcaagaacgccctgctgtctaccaacaaggccgttgtgtctctgagcaacggagtctccgtgctgacctccaaagtgctggacctgaagaactacatcaacaaccagctgctgcccatcgtgaatcagcaatcttgtagaatcagcaatattgaaaccgtgatcgagtttcagcagaagaacagcagactgctggaaatcactcgggaatttagcgtgaacgccggagtgaccacaccactgagcacatacatgctgacaaattctgagctgctgtccctgatcaatgatatgcctatcaccaacgaccagaaaaagctgatgagcagcaacgtgcccattgtgcggcagcagagctacagcatcatgtctatcatcaaagaggaagtgcttgcctacgtggtgcaactgcctatctacggagtgatcgacacaccttgctggaagctgcacaccagccctctgtgcaccaccaacatcaaagagggatctaatatctgcctgaccagaaccgacagaggctggtattgtgacaacgccggcagcgtgtccttcttccctcaggccgacacatgcaaggtgcaatctaacagggtgttctgcgacaccatgaactccctgaccctgccatctgaagtgtcgctgtgtaacacagatatcttcaacagcaaatatgattgcaagatcatgacatctaagaccgacatcagctccagcgtgattaccagcctgggcgccatcgtgtcctgctacggcaaaaccaagtgtaccgcttctaacaagaatagaggcatcatcaagaccttcagcaacggctgcgactacgtgtctaacaaaggcgtcgacaccgtgtccgtcggcaacaccctgtactacgtgaacaagctggagggcaagaatctgtacgttaagggcgagcctatcatcaactattacgatcctctggtgttccccagcgatgagttcgacgccagcatcagccaggtgaacgagaagatcaaccagagcctggccttcatccggagaagcgacgagctgctg

SEQ ID NO: 113 - DNA, 1401 bp, synthetic construct
  source 1..1401: mol_type = other DNA
cagaacatcaccgaagagttctaccagagcacctgcagcgctgttagccgcggatacttcagcgccctgcggaccggctggtatacaagcgtgattacaatcgagctgagcaacatcaaggaacccaagtgcaacggcacagatacaaaggtgaagctgatcaagcaggagctggataagtacaagaacgccgtgacagagctgcagctgctgatgcagagcggcggacctggcagcggaggaggcggcagcggaggcggcggctccagattcctgggcttcctgctcggcgtcggctctgctatcgcctctggaatcgccgtgtctaaggtgctgcacctggaaggcgaggtgaacaaaatcaaaaacgccctgctgtctacaaacaaggccgtggtttccctgtctaacggcgtgtctgtgctgacctctaaggtgctggacctgaagaattacatcaacaaccagctgctgcctattgtgaaccagcagtcttgcagaatcagcaacatcgagacagtgatcgagtttcagcaaaagaacagccggctgcttgagatcactcgggaatttagcgtgaatgccggcgtgaccacacctctgtctacctacatgctgaccaacagcgagctgctatccctgatcaacgacatgcctatcaccaatgatcagaaaaagctgatgagcagcaacgtgcagatcgtcagacagcagagctacagcatcatgtctatcatcaaggaagaagtgctggcctacgtggtgcaactgcctatctacggcgttatcgacaccccttgttggaagctccacaccagccccctgtgtacaaccaacattaaagagggcagcaacatctgcctgaccagaaccgatagaggctggtactgcgacaacgctggcagcgtgagttttttcccccaggccgacacatgcaaggtgcagagcaatagagtgttctgcgacaccatgaactccctgacactgccacctgaggtgtccctgtgtaataccgacattttcaacagcaagtatgattgcaaaatcatgaccagcaaaaccgacatcagctctagcgtcatcaccagcctgggcgccatcgtgagctgctacggcaagaccaagtgcaccgccagcaacaagaacagaggcatcatcaagaccttcagcaatggttgtgactacgtgtccaacaagggcgtggacaccgtgagcgtgggcaacaccctgtactacgtgaacaagctggaaggaaagaacctgtacgtgaagggcgaacctatcatcaactactacgaccccctggtgttcccatctgatgagttcgacgcctccatcagccaggtgaacgagaaaatcaatcaatctctggccttcatccggagaagcgacgagctgctg

SEQ ID NO: 114 - DNA, 1401 bp, synthetic construct
  source 1..1401: mol_type = other DNA
caaaacatcaccgaagagttctaccagtctacctgttctgccgtgagcagaggctatttcagcgccctgagaaccggctggtatacaagcgttatcacaattgaactgagcaatatcaaggaaaccaagtgcaacggcaccgatacaaaggtcaagctgatcaaacaggagctggacaagtacaagaacgccgtgaccgagctgcagctgctgatgcagagcggcggccctggcagcggaggcggaggcagcggtggcggcggcagcagattcctgggcttcctgcttggagtgggcagcgccatcgcttctggcatcgccgttagcaaagtgctgcacctggaaggcgaggtgaacaagatcaaaaacgccctgctgagcaccaacaaggccgtggtgtctctgtccaacggagtgtccgtcctgacctccaaggtgctggatctgaagaactacatcaacaaccagctgctgcctatcgtaaaccagcagtcttgtagaatcagcaatatcgagaccgtgatcgagttccagcagaagaacagccggctgctggagatcaccagagagttttcggtgaatgctggcgtcacaacacccctgagtacatacatgctgaccaacagcgaactgctgagcctgatcaacgacatgcctatcaccaatgaccagaaaaagctgatgagctccaacgtgccaattgtgcggcagcaaagctacagcatcatgagcatcatcaaggaggaagtgctggcctacgtcgtgcaactgccaatctacggcgtgatcgacaccccttgctggaagctgcacacctctcctctgtgcaccacaaacatcaaagagggctcaaacatctgcctgacacggaccgacagaggctggtactgcgacaacgccggctccgtgtccttcttcccccaggccgacacatgcaaggtgcagagcaacagagtgttctgcgatacaatgaacagcctcaccctgccccccgaggtgtccctgtgtaataccgacatcttcaactccaaatacgactgcaagatcatgaccagcaagaccgatatcagcagctctgtgatcaccagcctgggagccattgtgagctgctacggcaagaccaaatgcaccgccagcaataaaaatagaggaatcatcaagacattcagcaacggctgtgactacgtgagcaacaagggcgtggacacagtgagcgtgggcaacaccctgtactacgtgaacaagctggaaggcaagaatctgtacgtgaagggagaacctattatcaactactatgatcctctggtgtttcctagcgatgagttcgacgcctctatctctcaggtgaacgagaagatcaaccagtctcttgcttttatcaggcggagcgacgagctgctg

SEQ ID NO: 115 - DNA, 1401 bp, synthetic construct
  source 1..1401: mol_type = other DNA
cagaacatcacagaggagttctaccagagcacatgcagcgctgtgtctagaggctacttcagcgctctgagaacaggctggtacacctccgtcataaccatcgagctgagcaacatcaaggaacctaagtgtaatggtacagatacaaaggtgaaactgatcaagcaggagctcgacaagtacaagaatgctgtgaccgagctgcagctgctgatgcagtctggaggacctggctctggcggaggcggcagcggaggcggcggcagcagattcctgggctttccactaggcgtgggctccgccatcgcctctggcatcgccgtgtccaaggtgctgcacctggaaggcgaagtgaacaaaatcaagaacgccctgctgagcaccaacaaggccgtggtgagcctcagcaacggagtgagcgtgctgaccagcaaggtgctggatctgaagaattacatcaacaaccagctgctgcctatcgtaaatcaacagagctgcagaatctctaacatcgagacagtgattgagttccagcagaaaaactccagactgcttgaaatcacaagggaatttagcgtgaacgccggagtcaccacccccctgtctacatacatgctgaccaactctgagctgctgtctctgatcaacgacatgcctatcaccaatgatcagaagaagctgatgagctctaacgtgcctatcgtgcggcagcaaagctacagcatcatgagcatcatcaaagaggaagttctggcttatgtcgtgcagctgcccatctacggcgtgatcgacaccccttgctggaagctgcacaccagccctctgtgtaccaccaacatcaaggaaggcagcaacatctgcctgacacggaccgacagaggctggtattgcgacaacgccggcagcgtgtcattcttcccccaggccgacacctgcaaggtgcaaagcaatagagtgttctgcgacacaatgaacagcctgaccctgcccagcgaggtgtctctgtgcaacactgatatcttcaacagcaaatacgactgcaagatcatgaccagcaagaccgacatcagcagcagcgtgatcacaagcctgggcgccatcgtgtcttgttacggaaagaccaagtgcaccgcctctaacaagaaccggggcattatcaaaacattcagcaatggctgtgattacgtgtccaacaaaggcgtcgacaccgtgtccgtgggaaataccctgtactacgtgaacaagctggagggcaagaacctgtacgtgaagggcgagcctatcattaactactacgatcctctggtgttcccaagcgacgagttcgacgccagcatcagccaggtgaacgagaagatcaatcagtccctggcctttatcagacggagcgacgagctgctg

SEQ ID NO: 116 - DNA, 1401 bp, synthetic construct
  source 1..1401: mol_type = other DNA
cagaacatcacagaagagttctaccagtctacctgtagcgccgtgagccgcggctacttcagcgctctgagaaccggctggtatacatctgtgatcaccatcgagctgagcaacatcaaagagcctaagtgcaacggcaccgacaccaaggtgaagctgatcaagcaggagctggataagtacaagaacgctgtgaccgagctgcagctgctgatgcagagtggaggacctggcagtggcggcggcggatctggcggcggcggctctagattcctgggcttcccactgggcgtgggcagcgccatcgctagcggcatcgccgtgtccaaggtgctgcacctggaaggcgaggtgaacaaaatcaagaacgccctgctctccaccaacaaggccgtggtctctctgtccaatggcgtgtccgttctgacctctaaggtgctggacctgaagaactacatcaacaaccagctgctgcccatcgtgaaccagcagtcctgcagaatcagcaacatcgagacagtgatcgagtttcagcaaaaaaacagcagactgctggaaatcactcgggaatttagcgtgaatgccggcgtcacaacccctctgagcacctacatgctgacaaacagcgagctgctgagcctgatcaatgatatgcctatcaccaacgaccagaagaagctgatgagctctaacgtgcaaatcgtgcggcagcaaagctacagcatcatgagcatcatcaaagaggaagtgctggcctacgtggtgcagctgcctatctacggcgtgattgacaccccatgctggaagctgcacaccagccctctgtgcaccaccaatatcaaggaaggcagcaacatctgcctgacccggaccgatagaggctggtactgcgacaacgctggcagcgtgtccttcttcccccaggccgacacatgcaaggtgcagagcaatagagtgttctgcgacaccatgaacagcttaacactgcctcctgaggtgtccctctgtaacaccgacatcttcaactctaaatacgactgcaagattatgaccagcaaaacagatatcagcagctccgtgatcacatctctgggagccatcgtgtcttgctacggaaagacaaagtgtaccgccagcaataagaacagaggcatcatcaagacattcagcaatggttgtgattacgtgtctaacaagggtgtggacaccgtgtctgttggcaacaccctgtactacgtcaataagctggaaggaaaaaacctgtacgttaagggcgaacctataatcaattattacgaccccctcgtgtttcccagcgatgagttcgacgccagcatcagccaggtgaacgagaagatcaaccagagcctggccttcatcagacggagcgacgagctgctg

SEQ ID NO: 117 - DNA, 1401 bp, synthetic construct
  source 1..1401: mol_type = other DNA
cagaatatcaccgaggagttctaccagagcacctgtagcgccgtgtccagaggctacttcagcgccctgagaaccggctggtatactagcgtgatcaccatcgagctctctaatatcaaagagacaaaatgcaacggcaccgatacaaaagtgaagctgatcaagcaggagctggacaagtataagaacgccgtgaccgaactgcagctgctgatgcagtctggcggccctggcagcggcggcggaggcagtggaggaggcggaagccggttcctggggttccccctgggcgtcggcagcgctatcgcctctggcatcgccgtcagcaaggtgctgcacctggaaggcgaagtgaacaaaatcaagaacgctctgctgagcaccaacaaggccgtggtgtctctttctaacggcgtgtccgtgctgacatctaaagtgctggatctgaagaattacatcaacaaccagctgctgcctatcgtgaaccaacaatcttgcagaatcagcaacatcgagacagtgatagagtttcagcagaagaacagccgcctgctggaaatcacaagggaatttagcgtgaatgctggcgtgaccacacctctgtctacatacatgctgaccaatagcgagttactgagcctcatcaacgacatgcctatcaccaacgaccagaaaaagctgatgtctagcaacgtgcccatcgtgcggcagcagagctactcaatcatgagcatcatcaaagaggaagtgctggcctacgtcgtgcagctgcctatctacggcgtgattgacacaccttgctggaagctgcacaccagccctctgtgcaccaccaacatcaaggaaggctctaacatctgcctgacaagaaccgatcggggatggtactgcgacaacgccggctctgtgagcttcttcccacaggccgacacatgtaaggtgcagagcaacagagtgttctgcgacaccatgaacagcctgaccctgccacctgaggtgtccctgtgtaacaccgacatcttcaacagcaagtacgactgcaagattatgaccagcaagaccgacatcagtagcagcgtcatcacctctctgggcgctatcgtgtcctgctacggcaagacaaagtgcaccgccagcaataagaatagaggcatcatcaagaccttctccaatggctgtgattacgtttccaacaagggagtggacacagtgagcgttggaaacaccctctactacgtgaacaagctggagggcaagaacctgtacgtgaaaggcgagcccatcattaactactacgatcctctggtgtttcccagcgatgagttcgacgccagcatcagccaagtgaacgagaagatcaaccagagcctggccttcatcagacggagcgacgagctgctg

SEQ ID NO: 118 - DNA, 1401 bp, synthetic construct
  source 1..1401: mol_type = other DNA
cagaacattaccgaggagttctaccagagcacatgcagcgccgtctcccgcggctacttctctgccctgagaaccggctggtatacaagcgtgatcaccatcgagctgagcaacatcaaggaacccaagtgcaacggcaccgacaccaaagtaaaactgatcaaacaggagctggacaagtacaagaatgctgtgacagagctgcagctgctgatgcagagcggcggtcctggcagcggaggcggcggaagcggcggcggcggctctagattcctgggattcctgctcggagttggcagcgctatcgccagcggaatcgccgtgtccaaggtgctgcacctggaaggcgaagtgaacaagatcaagaatgctctgctcagcaccaacaaggccgtggtgagcctgagcaacggcgtgtctgtgctgacctctaaggtgctggatctgaagaactacatcaacaaccagctgctgcctatcgtcaaccaacagtcttgcagaatcagcaatattgaaaccgtgatcgaatttcagcaaaagaacagcagactgctggaaatcaccagagaattttctgtgaacgctggcgtcacaacccctctgtccacatacatgctgacaaatagcgagctgctgtctctgatcaatgacatgcctattacaaacgaccagaaaaagctgatgagcagcaacgtgccaatcgtgcggcagcaaagctacagcatcatgtctatcatcaaggaagaggtgctggcctacgtcgtgcagctgcctatctacggcgtgatcgacaccccttgctggaagctgcacaccagccctctgtgcaccaccaacatcaaggagggaagcaacatctgcctgactcggaccgatagaggctggtactgcgataacgccggcagcgttagcttcttcccccaggccgacacctgtaaggtgcagagcaaccgggtgttctgcgatacaatgaacagcctgaccctgccacctgaggtgtccctctgtaataccgatatcttcaacagcaaatacgactgtaagatcatgacctctaagacagacatcagcagcagcgtgatcacaagcctgggcgccatcgtgagttgctacggcaagaccaagtgtaccgccagcaacaagaacagaggcatcatcaagaccttctccaatggatgtgattacgtgtccaacaaaggcgtggacaccgtgtccgtgggcaacaccctgtattacgtgaacaagctggagggcaaaaatctgtacgtgaagggcgagcccattatcaactactacgaccccctggtgttccctagcgacgagttcgacgcctctatctcacaggtgaacgagaagatcaaccagagcctggcctttatcagacggagcgacgagctgctg

SEQ ID NO: 119 - DNA, 1401 bp, synthetic construct
  source 1..1401: mol_type = other DNA
cagaacatcaccgaggagttctaccagagcacatgcagcgccgttagccggggctacttcagcgccctgagaaccggctggtacacctccgtgattacaatcgagctgtccaatatcaaagagcctaagtgtaacggcaccgataccaaggtgaagctgattaaacaggagctggataagtacaagaacgccgtgaccgagctgcagctgctcatgcagagcggaggaccaggcagcggcggaggcggttctggcggcggaggcagcagattcccccccttcctgctcggcgtgggctctgctatcgccagcgggatcgccgtgtccaaggtgctgcacctggaaggcgaggtgaataaaatcaagaacgccctgctgagcaccaacaaggccgtcgtgtctctgagcaacggcgtcagcgtcctgaccagcaaggtgctggacctgaagaattacatcaacaaccagctgctgcctatcgtgaatcaacaaagctgcagaatcagcaacatcgagacagtgatcgaatttcagcaaaagaatagccggctgctggaaatcactagagagttcagcgtgaatgctggcgtgacaacccctctgagcacctacatgctgaccaactccgagctgctgagcctgatcaacgacatgcctatcaccaacgaccagaagaagctcatgtctagcaacgtgcagatcgtgcggcagcagagctacagcatcatgagcatcatcaaggaggaagtgctggcttatgtggtccagctgccaatctacggcgtgatcgacaccccttgctggaagctgcacaccagccctctttgtaccaccaacatcaaagaaggcagcaacatctgcctgacaagaacagatagaggctggtactgcgacaacgccggaagcgtgtcttttttcccccaggccgacacctgtaaagtgcagagcaacagagtgttctgcgacacaatgaacagtctgaccctgcctagcgaggtgtctctgtgcaataccgacatctttaacagcaagtatgattgcaagatcatgacctctaaaacagacatctcgtctagcgtgatcacatctctgggcgccatcgtgtcctgctacggcaagacaaagtgcaccgcctctaacaaaaacaggggcatcatcaagaccttcagcaacggctgtgattacgtgtccaacaagggcgtggacaccgtgtccgtcggcaacacactgtactacgttaacaagctggaaggaaagaacctgtacgtgaaaggcgaacctattatcaactactacgaccccctggtgttccctagcgacgagttcgacgccagcatcagccaggtgaacgagaagatcaaccagagcctggccttcatccggagaagcgatgagctgctg

SEQ ID NO: 120 - DNA, 1401 bp, synthetic construct
  source 1..1401: mol_type = other DNA
cagaacatcaccgaggagttctaccagagcacatgcagcgccgtgtccagagggtatttctccgctctgagaaccggctggtacaccagcgtgatcacaatcgagctgagcaacatcaaagagacaaagtgcaacggaacagacaccaaggtcaagctgatcaagcaggagctggataagtacaagaatgctgtgaccgaactgcagctgctgatgcagtccggcggtcctggctccggcggcggcggcagcggcggaggaggatctcggttccctcctttcctgctcggcgtgggcagcgctatcgccagcggaatcgccgtgtctaaagtgctgcacctggaaggcgaggtgaacaaaatcaagaacgccctgctgagcaccaacaaggccgtggtgtctctgagcaacggcgtttctgttctgaccagcaaagtgctggacctgaagaactacatcaacaaccagctgctgcccatcgtgaaccagcagagttgcagaatcagcaacattgagacagtgatcgagtttcagcaaaagaacagcagactgcttgaaatcaccagagagtttagcgtgaatgccggcgttacaacccctctgtctacctacatgctgacaaacagcgagctactcagcctgatcaacgacatgcctatcaccaatgaccagaaaaagctgatgagctccaacgtgcccatcgtgcggcaacagagctacagcatcatgagcatcatcaaggaagaggtgctggcctacgtggtgcagctgcctatctacggcgtgatcgacacaccatgttggaagctgcacaccagccctctgtgtaccacaaatatcaaggagggcagcaacatctgcctgacccggaccgacagaggctggtactgcgacaacgccggatctgtgtccttcttcccacaggccgatacctgtaaagtgcaaagcaatagagtgttttgcgacaccatgaactctctgaccctgccttctgaagtgtctctgtgcaataccgatatcttcaactcaaagtacgactgcaagatcatgaccagcaagacagatattagcagcagcgtcatcacaagcctgggcgccatcgtgtcctgctacggcaagacaaagtgcaccgccagcaacaagaacagaggcatcatcaagaccttcagcaacggctgtgattacgtgtccaacaagggcgtcgacactgtgagcgtcggcaacaccctgtactatgtgaacaagctggaaggcaagaatctctatgtgaagggcgaacccattatcaattactacgatcctctggtgttccccagcgacgagttcgacgcctctatcagccaggtgaacgagaagatcaaccagagcctggccttcatccggcgcagcgacgagctgctg

SEQ ID NO: 121 - DNA, 1401 bp, synthetic construct
  source 1..1401: mol_type = other DNA
cagaacattacagaagagttctaccagagcacatgcagcgccgtgtctagaggctacttcagcgctctgagaaccggctggtacacctccgtgatcacaatcgagctgtctaatatcaaggaaaccaaatgcaacggcaccgataccaaggtgaagctgatcaaacaggagctggataagtataagaacgctgttacagagctgcagctgctgatgcagagcggcggtcctggcagcggcggcggcggatctggcggaggcggcagccggttcccccccttcctcctcggcgttggaagcgccatcgcctctggaatcgccgtgtccaaggtgctgcacctggaaggcgaggtgaacaagatcaagaacgccctgctgagcaccaacaaggccgtggtgtccctgagcaatggcgtgtccgtgctgaccagcaaggtgctggacctgaagaactacatcaacaaccagctcctgcctatcgtgaatcaacaatcttgtagaatcagcaacatagagacagtgatcgagtttcagcagaagaacagcagactgctggaaatcacccgggaattttctgtcaatgctggagtgactacccctctgtctacctacatgctgacaaacagtgaactgctgagcctgatcaatgacatgcctattacaaacgaccagaaaaagctgatgagcagcaacgtgcaaatcgtgcggcagcagagctacagcatcatgagcatcatcaaggaggaagtgctggcctacgtcgtgcagctgcctatctacggcgtgatcgacacaccttgctggaagctgcacaccagccctctgtgcacgaccaacatcaaggagggcagcaacatctgcctgacaagaaccgatagaggctggtattgcgacaacgccggcagcgtctccttcttccctcaggccgacacctgtaaagtgcagagcaatagagtgttctgcgacaccatgaacagcctgacactgccaccagaagtgtcactttgtaataccgatatcttcaactctaagtacgactgcaagatcatgaccagcaagaccgatatcagctctagcgtgatcacctctctgggcgccatcgttagctgctacggcaagacaaagtgcaccgccagcaacaagaacagaggcatcatcaagaccttcagcaatggatgtgactacgtgtccaacaaaggcgtggacaccgtgagcgtgggcaacaccctgtactacgtgaacaaactggagggaaaaaacctgtacgtgaagggcgagcccattatcaactactacgaccccctggtctttcctagcgacgagttcgacgccagcatctctcaggtgaacgagaagatcaaccagtctctggctttcatcaggcggagcgatgagctgctg

SEQ ID NO: 122 - DNA, 1401 bp, synthetic construct
  source 1..1401: mol_type = other DNA
cagaacatcaccgaggagttctaccagagcacctgtagcgctgtgtcccggggctacttctctgccctgcggaccggctggtacaccagcgtgatcacaatcgagctgagcaacatcaaggaacccaagtgcaatggcaccgacaccaaggtgaagctgatcaagcaggagttggataagtacaagaacgccgtgaccgagctgcagctgctgatgcagagcggcggtcctggctctggaggaggcggctctggcggaggcggcagcagattcccccccttcctgctgggcgtgggctctgctatcgcctctggcatcgccgtgtctaaggtgctgcacctggaaggcgaagtgaacaaaatcaagaacgcactgctgagcaccaacaaggccgtcgtgagcctgtctaatggcgtgagcgtgctgaccagcaaagtgctggacctgaagaattacatcaacaaccaactgctgcccatcgtgaatcaacaaagctgtagaatcagcaacatcgaaaccgtgatcgagtttcagcagaagaacagcagactccttgagatcacccgggaatttagcgtgaacgccggcgtgacaactccactgtccacctacatgctgacaaacagcgagctgctgagcctgatcaacgacatgcctatcacaaatgatcagaaaaagctgatgagcagcaacgtccctatcgttagacagcagtcttatagcatcatgtctatcatcaaggaagaggtgctggcctacgtggtgcagctgcctatctacggcgtgatcgacaccccttgctggaagctgcacaccagccctctgtgcaccacaaacatcaaagagggcagcaacatctgcctgaccagaaccgatagaggatggtactgcgacaacgctggcagcgtgtccttcttcccacaggccgacacatgcaaggtgcagagcaatagagtgttctgcgacaccatgaacagcctgacactgcctagcgaggtgagtctgtgcaacacagacatcttcaacagcaagtacgactgcaagatcatgacctctaagaccgacatcagcagcagcgtgatcacaagcctcggcgccatcgtgtcctgctacggcaaaaccaagtgtacagccagcaacaagaaccggggaatcattaagacattcagcaacggctgtgattacgtgagtaacaagggcgtcgacacagtgtccgttggaaataccctgtactacgtgaacaagctggaaggcaagaacctgtacgtgaaaggcgagcctataattaactactatgatcctctggtgttccccagcgacgagtttgacgccagcatttcccaggtgaacgagaagatcaaccagtctctggccttcatcagaaggtccgatgagctgctg

SEQ ID NO: 123 - DNA, 1401 bp, synthetic construct
  source 1..1401: mol_type = other DNA
caaaacattaccgaggaattttaccagtctacatgcagcgccgtgtctagaggctacttcagcgccctgaggacaggctggtacaccagcgtgatcaccatcgagctgagcaatatcaaggagcctaagtgtaacggcacagatacaaaggtcaagctgatcaagcaggagctggacaagtataagaacgccgtgaccgagctccagctgctgatgcagagcggaggacctggcagcggcggtggcggctctggaggcggaggctctagattccccccattcctgctcggcgtgggctccgccatcgccagtgggatcgccgtgtccaaagtgctgcacctggaaggcgaggtgaacaaaatcaagaacgcactgctgtctaccaacaaggccgtggtgtccctgagcaacggcgtgtctgtgctgacaagcaaggtgctggatctgaagaactacatcaacaaccagctgctgccaatcgtgaaccagcagagctgcagaatcagcaacattgaaaccgtgatcgagtttcagcaaaagaacagcagactgctggaaatcacccgggagttcagcgttaatgctggcgtgacaacacctctgagcacctacatgctgactaacagcgagctgctgagcctgatcaacgacatgcctatcaccaatgatcagaaaaagctgatgtctagcaatgtgcaaatcgtgcggcagcagagctacagcatcatgagcatcatcaaggaagaggttctggcctacgtcgtgcagctgcctatctacggcgtgatcgacacaccttgttggaagctgcacaccagccctctgtgtaccaccaacatcaaggaaggcagcaacatctgcctgacaagaacagatagaggctggtattgcgacaacgccggatctgtctccttcttccctcaggccgatacctgcaaggtgcagagcaaccgggtgttctgcgataccatgaactccctgaccctgccccccgaggtgagcctgtgcaacacagacatcttcaacagcaaatacgactgcaagatcatgaccagcaagaccgacatcagctcatccgtgatcacaagcctgggcgctatcgtgtcttgttacggcaagaccaagtgcaccgccagcaacaaaaatagaggcatcatcaaaaccttcagcaacggctgcgactacgtgtccaacaaaggcgtcgacaccgtgtccgtgggcaacaccctgtactacgtgaacaagctggagggaaagaacctctatgtgaagggagaacctattatcaattactacgaccccctggtgttccccagcgacgagttcgacgccagcatcagccaggtgaacgagaagatcaaccagagcctcgcttttatccggagaagcgacgagctgctg

SEQ ID NO: 124 - DNA, 1401 bp, synthetic construct
  source 1..1401: mol_type = other DNA
cagaacattaccgaagagttctaccagagcacctgtagcgccgtgtccagaggctacttcagcgccctgagaaccggatggtacactagcgtgatcaccatcgagctgagcaatatcaaggaacagaaatgcaatggcaccgatacaaaggtcaagctgatcaagcaggagctggacaagtacaagaacgccgtgacagagctgcaactgctgatgcagagtggaggtcctggcagcggaggcggcggatctggcggcggcggctctagattcccccccttcctgctgggagtcggctctgctattgccagcggcatcgccgtgtctaaggtgctccacctggagggcgaggtcaacaagatcaagaacgctctgctgagcacaaacaaggccgtggtgagcctgagcaacggcgtaagcgtgctgacctccaaggtgctggacctgaagaactacatcaacaaccaactcctgccaatcgtgaaccagcagagctgtagaatctctaacatcgaaaccgtgatcgagttccagcaaaagaacagccggctgctggaaatcaccagagagttcagcgttaacgcgggcgtgaccacacctctgtctacatacatgctgacaaatagcgagctgctgagcctgatcaacgacatgcctatcacaaacgatcagaagaagctgatgagctctaatgtgcctatcgtgcggcagcagagctacagcattatgagcatcatcaaggaagaggtgctggcctacgtggtgcagctgcccatctacggagtgatcgacaccccctgctggaagctgcacaccagccccctgtgcaccaccaacatcaaagagggcagcaacatctgcctgacccggaccgatagaggctggtattgtgataacgccggttctgtgagcttctttcctcaggccgacacctgcaaggtgcagagcaacagagtgttctgcgacaccatgaacagcctcacactgcctcctgaggtgtccctttgtaataccgacatcttcaactccaaatacgactgcaagatcatgaccagcaagacagacatcagctctagcgtgataacatccctgggcgccatcgtgtcatgctacggcaagaccaagtgcacagccagcaacaagaaccggggcatcatcaaaacattctccaatggctgcgactacgtgagcaataaaggcgtcgacaccgtgagcgtgggcaacaccctgtactacgttaacaaactggaaggcaaaaacctgtatgtgaaaggagaacctatcatcaactactacgatcctctggtgttcccatctgatgaatttgacgcctctatctcccaggtgaacgagaagatcaatcagtccctggcttttatccgcagaagcgacgagctgctg

SEQ ID NO: 125 - DNA, 1401 bp, synthetic construct
  source 1..1401: mol_type = other DNA
cagaacatcaccgaggagttctaccagtctacctgcagcgccgtgagccggggctacttcagcgccctgcggactggctggtacacctccgtcattaccatcgagctgagcaacatcaaagaacctaagtgtaacggcacagacaccaaggtgaagctgatcaagcaggagctggataagtacaagaatgctgtcaccgagctgcagctgctgatgcagagcggcggacctggcagcgggggcggaggatctggtggaggcggcagccgcttcctgggcttccccctgggagttggctctgctatcgcctccggaatcgctgtgtctaaggtgctgcacctggaaggcgaagtgaacaaaatcaaaaacgctctgctgtctacaaacaaggccgtggtgagtctgtctaacggcgtgagcgtgctgaccagcaaggtcctggacctgaagaactacatcaacaaccagctgctgcctatcgtgaaccaacaaagctgtagaatcagcaatatcgagacagtgatcgagtttcagcagaagaacagcagactgctggaaatcaccagagagttcagcgtgaacgccggcgttacaacacctctgagcacatacatgctgacaaacagcgagctgctgagtctgatcaacgacatgcctatcaccaatgatcagaaaaagctgatgagcagcaacgtgcccattgtgcggcagcagagctacagcatcatgagcatcatcaaggaagaggtgcttgcctacgtcgtgcagctgcccatctacggcgtgatcgacaccccctgctggaagctgcacaccagccctctctgtacaaccaatatcaaggaaggcagcaacatctgcctgacaagaaccgatagaggctggtactgcgacaacgccggatctgtgagttttttcccacaggccgacacctgtaaagtgcagtccaacagagtgttttgcgacacaatgaatagcctgacactgccacctgaggtgtccctgtgcaacaccgacatcttcaactctaaatacgactgcaagatcatgaccagcaaaaccgacatcagcagcagcgtgatcacatctctgggcgccatcgtgtcctgctacggcaagaccaagtgcaccgccagcaacaagaatagaggcatcatcaagaccttctccaatggctgcgattacgtgagcaacaaaggcgtggacaccgtgagcgtgggcaacaccctgtactacgtgaataagctggaaggcaagaacctttatgtgaagggcgagcccattattaactactatgatcctctggtgttccctagcgacgagttcgacgcctctatctcccaggtgaacgagaagatcaatcaaagcctggccttcatcagacggtctgatgagctgctg

SEQ ID NO: 126 - DNA, 1401 bp, synthetic construct
  source 1..1401: mol_type = other DNA
caaaacatcaccgaagagttctaccagagcacctgtagcgctgtcagccggggctacttcagcgccctgagaaccggctggtacactagcgtcatcaccatcgagctgagcaatatcaaagaacccaagtgcaatgggaccgacaccaaggtgaagctgatcaagcaggagctggataagtacaagaacgcagttacagagctccagctgctgatgcagtccggcggacctggctcaggcggcggaggcagcggaggcggcggaagcaggttccctccattcctgctgggcgtgggcagtgctatcgccagcggcatcgccgtgtccaaggtgctgcacctggagggcgaagtgaacaagatcaagaacgccctgctgagcacaaacaaggccgtcgtgtctctgagcaacggcgtttctgtgctgacatctaaggtgctcgatctgaagaactacatcaacaaccagctgctgcctatcgtgaatcaacaaagctgcagaatcagcaacatcgagacagtgatcgagttccagcagaagaacagcagactgctggaaatcacaagagagttcagcgtgaacgccggcgtgaccacccctctgtctacctacatgctgaccaatagcgagctgctcagcctaatcaacgacatgcctattacaaatgaccagaaaaagctgatgtctagcaacgtgcctatcgtgcggcagcagagctacagcatcatgagcatcatcaaggaagaagtgctggcctacgtggtgcagctgcctatctacggcgtgatcgacactccctgctggaaactgcacaccagccctctgtgtacgacaaatatcaaggaaggctccaatatctgcctgaccagaaccgatagaggctggtattgcgacaacgccggctctgtgagcttcttcccccaggctgacacatgcaaggtgcagagcaacagagtgttctgcgatacaatgaacagcctgaccctgccccccgaggtgtccctgtgcaacacagacatcttcaacagcaagtacgactgcaagatcatgacctctaagaccgacatctctagctccgtgatcaccagcttgggagccatcgtgtcctgctacggcaagaccaaatgtaccgccagcaacaaaaaccggggaattatcaagacatttagcaatggttgtgactacgtgtccaacaagggcgtggacaccgtgtctgttggcaacaccctgtactacgtgaacaagctggaaggcaaaaacctgtacgtgaaaggcgagcctatcatcaactactatgatcctctggtgtttccaagcgacgagttcgacgcctctatcagccaggtgaacgagaagatcaaccagagcctggcctttatacggagatctgatgagctgctg

SEQ ID NO: 127 - DNA, 1401 bp, synthetic construct
  source 1..1401: mol_type = other DNA
cagaacatcactgaagagttctaccagtccacctgcagcgctgtgagtaggggctacttctctgccctgagaacaggctggtacacctccgtgatcaccatcgagctgagcaatattaaggaacctaagtgtaatggcaccgataccaaggtgaaactgatcaagcaggagctggacaagtacaagaacgccgtgacagagctgcagcttcttatgcagagcggcggccccggcagcggaggcggcggatctggaggcggcggttccagattccctccattcccactgggcgttggaagcgccatcgcctctggcatcgccgtttccaaggtgctgcacctggaaggagaagtgaacaagatcaagaatgccctgctgagcaccaacaaggccgtggtgagcctgtctaacggcgtgtctgtcctgaccagcaaggtgctggatctgaagaactacatcaacaaccagctgctgcctatcgtgaatcaacagagctgtagaatctctaatatcgagacagtgatcgagtttcagcagaagaacagcagactgctggaaatcacacgggagttcagcgtgaacgccggcgtgaccacccctctgagcacatacatgctgaccaactctgagctgctgtccctgattaacgacatgcctatcaccaacgatcagaaaaagctgatgagcagcaacgtgcccatcgtgcggcagcaaagctacagcatcatgagcatcatcaaagaggaagtgctggcctacgtcgtgcagctgcccatctacggcgtcatcgacacaccttgctggaagctgcacaccagccctctgtgcacaaccaatattaaggaaggcagcaacatctgcctgaccagaacagatagaggctggtattgcgacaacgccggctctgtttcattcttcccccaggccgacacctgtaaagtgcaatctaaccgggtgttttgcgacaccatgaactccttgaccctgccacctgaggtgagcctgtgcaacacagacattttcaactccaagtacgactgcaagatcatgacaagcaaaaccgacatctctagcagcgtgatcaccagcctcggcgctatcgtgagctgctacggcaagacaaagtgcaccgccagcaacaagaatagaggcatcatcaagaccttcagcaacggctgtgactacgtgagcaacaaaggcgtggacaccgtgtctgtgggcaacaccctgtactacgtgaacaagctggaaggaaaaaacctgtacgtaaagggcgagcctatcatcaactactatgatcctctggtgttccccagcgacgagttcgacgctagcatctcacaggtgaacgagaagatcaaccagtctctcgcttttatccggagaagcgatgagctgctg

SEQ ID NO: 128 - DNA, 1401 bp, synthetic construct
  source 1..1401: mol_type = other DNA
cagaacatcaccgaggagttctaccagagcacctgtagcgccgtgagcagaggctacttcagcgccctgagaacaggatggtacaccagcgtgatcaccatcgagctgagcaacatccccgagacaaagtgcaacggcaccgacaccaaagtcaagctgatcaagcaggagctggataagtataagaacgccgtgaccgagctgcagctgctgatgcagtctggcggacctggcagcggcggtggcggaagcggcggcggcggcagtaggttccctccattccccctgggagtgggctctgctatcgcctctggcatcgctgtttccaaggtgctgcacctggaaggcgaggtgaacaaaatcaagaacgctctgctgagcaccaacaaggccgtggtcagcctgagcaatggcgtgagcgtcctcacgagcaaggtgctggatctgaagaactacatcaacaaccagctgctgcctatcgtgaatcaacaaagttgcagaatcagcaacattgaaaccgtgatcgagtttcagcaaaagaacagcagactgctggaaatcacccgggaattttctgtgaacgccggcgttacaacacctctgagcacctacatgctgacaaactccgagctgctgtctctgatcaacgacatgcctatcaccaatgaccagaaaaagctgatgagcagcaacgtgcccatcgttagacagcagagctacagcatcatgtccatcatcaaggaagaagtgctggcctacgtggtgcagctgcccatctacggcgtgatcgacaccccttgttggaagctgcacaccagccctctgtgcaccacaaacatcaaggaaggcagcaacatctgcctgactcggaccgatagaggatggtattgcgataacgcaggcagcgtctccttcttccctcaggccgacacatgcaaggtgcagagcaatagagtgttctgcgacaccatgaactccctgaccctgcctcctgaggtgtctctctgtaataccgacatcttcaacagcaaatacgactgcaagatcatgacatctaaaacagatatctctagcagcgtgatcacaagcctgggcgccattgtgtcttgctacggaaagacaaagtgtaccgccagcaacaagaaccggggaatcatcaaaaccttcagcaacggctgcgactacgtgtccaacaagggcgtggacacagtgtccgtgggcaacaccctgtactacgtgaacaagctggaaggcaagaacctgtacgtgaaaggcgagcctattatcaattactacgaccccctggtgtttccatctgatgagttcgacgccagcatcagccaggtgaatgagaagattaatcagagcctcgccttcatccggagaagcgacgagctgctg

SEQ ID NO: 129 - DNA, 1401 bp, synthetic construct
  source 1..1401: mol_type = other DNA
cagaacatcaccgaagagttctaccagagcacctgcagcgccgtgtctagaggctacttctccgctctgagaacgggatggtacaccagcgtgattacaatcgagcttagcaacatcaaggaaaccaagtgcaacggcacccccaccaaagtgaagctcatcaagcaggagctggataagtacaagaacgccgtgaccgagctgcagctgctgatgcagagcggcggccctggctctggcggcggcggcagcggtggaggcggatctaggttccctccattccccctgggagttggctctgctatcgccagcggcattgccgttagcaaggtgctgcacctggaaggcgaggtgaacaagatcaagaacgctctgctgtccaccaacaaggccgtggtgtctctgagcaacggcgtgagcgtgctgacatctaaagtgctggacctgaagaattacatcaacaaccaactgctgcctatcgtcaatcagcaatcttgtagaatcagcaacatcgagacagtgatcgagtttcagcagaaaaactccagactgctggaaatcactcgggaatttagcgtgaacgccggcgtcaccacacctctgagcacctacatgctgacaaacagcgagctcctgagcctgatcaatgatatgcctatcaccaacgaccagaagaagctgatgagcagcaacgtgcctatcgtgcggcagcagtcctacagcatcatgagcatcatcaaggaagaagtgctggcttatgtggtccagctgccaatctacggcgtgatcgacacaccctgctggaagctccacaccagccctctgtgtaccaccaacatcaaggagggctctaatatctgcctgacaagaacagatagaggctggtactgcgacaacgccggctctgtgtcattcttcccacaggccgatacctgtaaagtgcaaagcaacagagtgttctgcgacaccatgaacagcctgaccctgcctcctgaggtgtccctgtgcaacacagacatcttcaacagcaagtatgattgcaagattatgaccagcaagaccgacatctccagcagcgtgatcacaagcctgggtgccatcgtgtcctgctacggcaaaacaaagtgcacagccagtaacaagaaccggggaatcatcaagaccttctctaatggatgtgactacgtgagcaataaaggcgtggacaccgtgagcgtgggcaacaccctgtactacgtgaacaagctggaaggcaagaacctgtacgtcaaaggcgaacccatcatcaattactacgaccccctggtgtttcctagcgacgagttcgacgcctccatcagccaggtgaacgagaagatcaatcagtctctggccttcatccggagaagcgatgagctgctg

SEQ ID NO: 130 - DNA, 1401 bp, synthetic construct
  source 1..1401: mol_type = other DNA
cagaacatcacagaggagttctaccagagcacgtgcagcgccgtgtctcggggctacttcagcgccctgagaaccggatggtacaccagcgtgatcacaatcgagctgagcaacatcaaggaaacaaagtgtaatggcaccgacacaaaggtcaagctgatcaagcaggagctggataaatacaagaacgctgtgaccgagctgcagctgctgatgcagagcggaggacctgggagcggcggaggcggcagcggcggcggcggctctagattcctgggattccccctgggcgtcggcagcgctatcgcctccggcatcgccgtgtctaaggtgctgcacctggaaggcgaggtgaacaagatcaagaatgctctgctgagcacaaacaaggccgtggtgtctctgagcaacggcgtgagcgtgctgaccagcaaggtgctcgacctgaagaactacatcaacaaccagctgctgcctatcgtcaaccagcagagctgcagaatctcccctatcgagacagtgatcgagtttcagcaaaagaacagccggctgctggaaatcacccgggaatttagcgtcaacgcaggcgttacaacccctctgtctacatacatgctgacaaacagcgagctgctgtcccttatcaacgatatgcctatcaccaacgaccagaaaaagctgatgagcagcaacgtgcagattgtgcggcagcagtcctacagcatcatgagcatcatcaaagaggaagtgctggcctacgtggttcaactgcccatctacggagtgatcgacaccccctgctggaagctgcacaccagccctctgtgtaccactaacatcaaggaaggctccaatatctgcctgaccagaacagatagaggctggtattgcgacaatgccggcagcgtgtccttcttccctcaggccgacacctgtaaagtgcagagcaacagagtgttctgcgacaccatgaacagcctcaccctgccttctgaagtgtctctgtgcaacaccgatatcttcaacagcaagtacgattgcaagatcatgaccagcaagacagacatcagcagctctgtgatcaccagcctgggcgccatcgtgtcctgctacggaaaaaccaagtgcaccgccagcaacaaaaatagaggcatcattaagacattcagcaatggttgtgactacgtgtccaacaagggagtggacaccgtgtcggtgggcaacactctgtattacgtgaacaagctggaaggcaaaaatctgtacgtgaagggcgagccaattatcaactactacgaccccctggtgtttccaagcgacgagttcgacgcctctatttcacaagtgaacgagaagatcaatcagagcctcgccttcatcagaaggagcgatgagctgctg

SEQ ID NO: 131 - DNA, 1401 bp, synthetic construct
  source 1..1401: mol_type = other DNA
cagaacatcacagaagagttctaccagagcacatgtagcgctgtttccagaggctacttcagcgctctgaggacgggctggtatacatctgttatcacaatcgaactgagcaacattaaggaacccaagtgcaacggtacagacaccaaggtgaagctgatcaaacaggagctggataaatacaagaacgccgtgaccgagctgcagctgctgatgcagagcggcggtcctggctctggcggaggcggcagcggaggcggaggaagcagattcctgggcttcccactgggagtcggcagcgccattgcctctggcatcgccgtgtctaaggtgctgcacctggaaggcgaggtgaataaaatcaagaacgccctgctctctaccaacaaagccgtggtgagcctgagcaatggagtgtccgtgctgacaagcaaggtgctggacctgaagaattacatcaacaaccagctgctgcctatcgtcaatcaacagagctgtagaatctctcctatcgagacagtgattgagtttcagcaaaagaacagcagactgctggaaatcacccgggaatttagcgtgaacgctggcgtgaccacacctctttctacctacatgctgaccaactctgagctcctgtctctgatcaacgacatgcctattaccaacgaccagaaaaagctgatgagcagcaacgtgcagatcgtgcggcagcagagctacagcatcatgagcatcatcaaggaggaagtcctggcctacgtggtgcaactgcctatctacggcgtgatcgacaccccttgctggaagctgcacaccagccctctgtgcaccaccaacatcaaggaaggctccaatatctgcctgacccggaccgatagaggatggtactgcgataacgcaggctccgtgagcttcttcccccaggccgacacatgcaaagtgcagtcgaatagagtgttctgcgacaccatgaacagcctgaccctacccagcgaggtgtccctctgtaacacagacatcttcaacagcaagtatgattgcaagatcatgaccagcaagaccgatatcagcagctctgtgatcacctccctgggcgccatcgtgtcctgctacggcaaaacaaagtgcacagccagcaacaagaatcggggcatcatcaagacttttagcaacggctgtgactacgtgtccaacaagggcgtggacaccgtgagcgtgggcaataccctgtactacgtcaacaagctggaaggcaagaacctgtacgtgaagggcgagcctatcatcaactactacgaccccctggtgttcccatctgatgagttcgacgccagcatcagccaggttaacgagaagatcaaccagagtctggccttcatcagaagaagcgacgagctgctg

SEQ ID NO: 132 - DNA, 1401 bp, synthetic construct
  source 1..1401: mol_type = other DNA
cagaacatcaccgaggagttctaccagagcacatgctctgccgtgagcagaggctacttcagcgccctgagaaccggctggtacaccagcgtcatcacaatcgagctgtccaacatcaaggagcctaagtgcaacggcacggatacaaaggttaagctgatcaaacaggagctcgacaagtacaagaacgccgtgacagagctgcagctgctgatgcagagcggagggcctggcagcggcggcggtggcagcggcggcggaggcagcaggttcctgggcttccccctgggcgtgggcagcgccatcgctagcggcatcgctgtgagcaaggtgctgcacctggaaggcgaggtgaacaaaatcaagaacgccctgctgtctaccaacaaggccgtggtcagccttagcaacggcgtgtctgttctgacctccaaggtgctggatctcaagaactacatcaacaaccagctgctccctatcgtgaaccagcaatcttgtagaatctctccaatcgagacagtgatcgagtttcagcagaagaacagccggctgctggagatcactcgggagttcagcgtgaacgccggcgtgaccacccctctgagcacctacatgctgaccaacagtgaactgctgtcacttatcaacgacatgcctatcacaaatgaccagaaaaagctgatgagcagcaatgtgcaaatcgtgcggcagcagagctacagcatcatgagcatcattaaggaagaggtgctggcctacgtggtgcagctgcccatctacggcgtgatcgacaccccttgctggaagctgcacacatctccactgtgcaccaccaacatcaaggaaggcagcaatatctgcctgacaagaacagatagaggctggtactgcgacaacgctggcagcgtgagcttcttccctcaggccgacacctgtaaagtgcagagcaatagagtcttttgcgacacaatgaacagcctgaccctgccccccgaggtgtctctgtgtaataccgacatcttcaacagcaagtatgattgcaagatcatgaccagcaagaccgatattagcagctctgtgatcacctccctgggcgccatcgtgtcctgctacggaaaaacaaagtgcaccgccagcaacaagaacagaggaatcatcaaaaccttcagcaatggatgtgattacgtgtccaacaaaggcgtggacaccgtgtccgttggcaacaccctgtactatgtgaacaagctggaaggcaagaacctgtacgtgaagggcgaacctattatcaactactacgaccctctggtgttccccagcgacgagttcgacgcctctatctctcaggtgaatgagaagattaaccaaagcctggcttttatccggagaagcgacgagctgctg

SEQ ID NO: 133 - DNA, 1401 bp, synthetic construct
  source 1..1401: mol_type = other DNA
cagaacatcaccgaggagttctaccagtctacctgcagcgccgtgagccggggctatttcagcgccctgaggaccggctggtacaccagcgtgattacaatcgagctgagcaatatcaaggaacctaagtgtaatggaacagacaccaaggtcaagctgatcaagcaggagctggataagtacaagaacgctgttacagagctgcagctgctgatgcagagcggcggacctggtagcggaggcggcggctctggcggcggcggaagcagattcctgggcttccccctgggagtgggatctgccatcgcctccggcatcgccgtgagcaaggtgctgcacctggaaggcgaagtgaacaaaatcaagaacgctctgctgagcacaaacaaggcagtcgtgtccctgtctaatggcgtgagtgttctgacctctaaagtgctcgacctgaagaactacatcaacaaccagctgctccctatagtgaatcaacaaagctgcagaatctctcccatcgaaaccgtgatcgagttccagcaaaagaacagcagactgctggaaatcacacgggaattttccgttaatgctggagtgaccacccctctgtccacatacatgttgaccaatagcgagctgctgtcgctgatcaacgatatgcctatcaccaacgaccagaaaaagctgatgagcagcaacgtgcctatcgtcagacagcagagctacagcatcatgagcatcatcaaagaggaagtgctggcctacgtggtgcagctgcctatctacggcgtaatcgacacaccctgctggaagctacacacctcaccactgtgtacaacaaacatcaaggagggctctaacatctgcctgaccagaaccgatagaggctggtactgcgacaacgccggctccgtgtccttcttccctcaggccgacacctgtaaagtgcagagcaaccgggtgttctgcgacaccatgaactctttaaccctccccagcgaggtgagcctgtgcaacacagatatcttcaacagcaaatacgactgcaagatcatgaccagcaagaccgacatcagctctagcgtgattacctccctgggcgccatcgtgagctgctacggcaagaccaaatgcacagccagcaacaagaatagaggcatcatcaagactttttctaacggctgtgattacgtgtctaacaagggcgtggacacagtgagcgtgggcaacaccctgtactatgtgaacaagctggagggcaagaacctgtacgtgaagggcgagcctatcatcaactactatgaccccctggtgtttccaagcgacgagttcgacgccagcatcagccaggtgaacgagaagatcaaccagtcactggccttcatccggagaagcgatgagctgctg

SEQ ID NO: 134 - DNA, 1401 bp, synthetic construct
  source 1..1401: mol_type = other DNA
cagaacatcaccgaggagttctaccaaagcacatgcagcgccgtcagcaggggatatttcagcgccctgcggaccggctggtacaccagcgtgatcaccatcgagctgagcaacatcaaagaacccaagtgcaacggcacagataccaaggtgaagctgatcaaacaggagcttgataagtacaagaacgctgttacagagctccagctgctgatgcagagcggcggtcctggcagcggcggcggcggatctggcggaggcggcagcagattccctccattcctgctgggcgttggaagcgctatcgcctctggcattgccgtgtcgaaggtgctgcacctggaaggcgaggtgaataagatcaagaacgccctgctgtccaccaacaaggccgtggtgtctctgtctaatggcgtgagcgtgctgacctctaaggtgctcgacctgaagaattacatcaacaaccagctgctgcctatcgtgaaccagcaaagctgcagaatctcccctattgaaaccgtgatagagtttcagcagaagaacagcagactgctggaaatcacccgggagttcagcgtgaacgccggcgtgacaacacctctgtccacatacatgctgacaaacagtgaactgctgagcctcatcaacgacatgcctatcacaaatgaccagaaaaagctgatgagcagcaacgtgcagatcgtgcggcagcaaagctacagcatcatgtctatcatcaaggaagaagtgctggcttacgtggtgcagctgcctatctacggcgtgatcgacaccccttgttggaagctgcacaccagccctctgtgcacaaccaacatcaaagagggcagcaacatctgcctgaccagaaccgatagaggctggtattgcgacaacgcaggctccgtgtccttcttcccccaggccgatacctgtaaagtgcagagcaatagagtgttctgcgacaccatgaacagcctgacactgccccccgaggtgagcctgtgtaacacagatatcttcaacagcaagtatgactgcaagatcatgacctctaaaaccgatatctcctctagcgtgattacaagcctgggagccatcgtttcctgctacggcaagaccaaatgcaccgccagcaacaagaacagaggcatcatcaaaactttttccaatggatgtgactacgtcagcaacaagggcgtcgacaccgtgagcgtgggcaacaccctgtactacgtgaacaagctggagggaaagaacctgtacgtgaagggcgagcctatcatcaactactacgaccccctggtgtttccatctgacgagttcgacgccagcatcagccaggtgaacgagaagatcaaccagtctctggccttcatccggagaagcgacgagttgctg

SEQ ID NO: 135 - DNA, 1401 bp, synthetic construct
  source 1..1401: mol_type = other DNA
cagaacatcacagaagagttctaccagagcacatgcagcgccgtctctcgcggctacttcagcgctctgagaaccggctggtacaccagcgtcattaccatcgagctgtctaacatcaaggaacccaagtgcaacggcaccgacaccaaagtgaagctgatcaaacaggagctggataagtacaagaacgctgtgaccgagctgcagctgctgatgcagagcggaggtcctggcagcggcggcggaggatctggcggcggcggaagcagattccctccattccccctgggcgtgggctccgccatcgccagcggcatcgccgtgtccaaggtgctgcacctggagggagaagtgaacaagattaagaacgctctgctgtcaaccaacaaggccgtggtcagtctgagcaacggcgtgtctgtgctgacaagcaaagtgctggacctgaagaattacatcaacaaccagctgctgcctatcgttaatcaacagagctgcagaattagtcctatcgaaaccgtgatcgagtttcagcagaagaacagccggctgctggaaatcacacgggaattttccgtgaacgccggcgttacaacacctctgagcacctacatgctgacaaacagcgagctcctcagcctgatcaatgacatgcctatcacaaacgaccagaaaaagctgatgagcagcaacgtgcagatcgtgcggcagcaatcctacagcatcatgagcatcatcaaggaagaggtgcttgcctacgtggtgcagctgcccatctacggcgtgatcgacaccccttgctggaagctgcacaccagccctctgtgcaccaccaatatcaaagagggcagcaacatttgcctgacaagaacagatagagggtggtattgcgacaacgcaggcagcgtcagcttcttcccccaggccgacacctgtaaagtgcaaagcaacagagtgttctgcgacaccatgaactctctgaccctccctcctgaggtgtccctgtgtaacaccgatatcttcaactccaaatacgattgcaagatcatgaccagcaagacagacatcagctcttctgtgatcaccagcctgggcgccatcgtgagctgctacggcaagaccaagtgtaccgcctctaacaagaacagaggcatcatcaagaccttcagcaatggctgtgattacgtgtccaataagggcgtggacactgtcagcgtgggaaatactctgtattacgtgaacaagctggaaggaaagaacctgtacgtgaagggcgagccaatcatcaactactacgaccccctggtgtttccatctgatgagttcgacgccagcatcagccaggtgaacgagaagatcaaccagagcctggccttcatccggaggagcgacgagctgctg

SEQ ID NO: 136 - DNA, 1401 bp, synthetic construct
  source 1..1401: mol_type = other DNA
cagaacattaccgaggagttctaccagtctacatgcagcgccgtcagcagaggttatttctctgctctgagaactggctggtacaccagcgtgatcaccatcgagctgtctaatatcaaagagcccaagtgcaacggcaccgacaccaaggtgaagctcatcaagcaggagctggataagtacaagaacgctgttacagagctccagctgctgatgcagagcggcggacctggcagcggcggcggaggctctggaggcggaggctccagattcctgggatttcccctgggagtcggcagcgccatcgcctccggcatcgccgtgagcaaggtgctgcacctggaaggagaagtgaacaagatcaaaaatgccctgctgagcaccaacaaggccgtggtgagcctgagcaacggcgtgagcgtgctgacaagcaaggtgctggacctgaaaaactacatcaacaatcagctgctgcctatcgtgaatcaacaaagctgcagaatcagccctattgagacagtgatcgagttccagcagaaaaatagcagactgctggaaatcacccgggaatttagcgtgaacgctggcgtgacaacccctctgtccacctacatgctgaccaacagcgagctgctgtcactgatcaacgacatgcctatcacgaatgatcagaagaagctgatgagcagcaatgtgccaatcgttagacagcagagctacagcatcatgagcatcatcaaggaagaagtgctggcctacgtggtgcagctgcctatctacggcgtgatcgacaccccttgctggaagctgcacaccagccccctgtgcaccaccaacatcaaagaaggctctaacatctgcctgacaaggacagatagaggctggtactgcgataacgctggctccgtgagcttcttcccccaggccgacacctgtaaggttcaatctaacagagtgttctgcgatacaatgaactctctgaccctgcctcctgaggtgtccctgtgtaacacagacattttcaactctaaatacgactgcaagattatgaccagcaagaccgacatcagctccagcgtgatcacaagcctgggcgccatcgtgtcttgttacggcaaaacaaagtgcaccgcctctaataagaaccggggcatcatcaagaccttcagcaacggctgtgactacgtgagcaacaagggcgtcgacaccgtgtccgtgggcaacaccctctactacgtgaacaagctggagggcaagaacctgtatgtcaagggcgagcctatcatcaactactacgaccccctggtgtttccaagtgatgagttcgatgccagcatcagccaggtgaacgagaagatcaaccagagcctggccttcatccggcggagcgacgagctgctg

SEQ ID NO: 137 - DNA, 1401 bp, synthetic construct
  source 1..1401: mol_type = other DNA
cagaacatcacagaggagttctaccagagcacctgtagcgccgtgtccagaggctacttctctgctctgagaacaggctggtatacatctgtgatcaccatcgagctgtccaacatcaaggagcccaagtgcaacggcaccgacaccaaggtgaagctgatcaagcaggagctggataagtataagaacgctgtgaccgagctgcagctgctgatgcagagcggcggtcctggctctggaggaggcggatctggcggcggcggctctaggttcccccctttcctgctcggcgtcggcagcgctatcgccagcggcatcgccgtgtctaaggtgctgcacctggagggcgaggtgaacaagattaagaacgccctgctgagcaccaacaaggccgtcgtgtctctgagcaacggcgtgagcgtcctgaccagcaaagtgctggacctgaagaattacatcaacaaccagctgctgccaatcgtgaatcaacagtcatgcagaatcagccctattgaaaccgtgatcgagtttcagcagaagaacagcagactgctggaaatcactcgggaatttagcgttaatgccggagtgaccacacctctgagcacctacatgctgacaaatagcgagctcctgagcctgatcaacgacatgcctatcaccaatgatcagaaaaagctgatgtcttctaacgtgcctatcgtgcggcagcaatcctacagcatcatgagcatcatcaaggaagaggtgctggcctacgtggtgcagctgcctatctacggagttatcgacacaccatgttggaagctgcacaccagccccctgtgtaccaccaacattaaggaaggctccaacatctgcctgacaagaaccgatagaggatggtactgcgacaacgccggcagcgtgagttttttccctcaggctgatacatgcaaggtgcagagcaatagagtgttctgcgacaccatgaactccttgacactgcctcctgaggtgtccctgtgcaacacagacatcttcaactcaaagtacgactgcaaaatcatgaccagcaagacagatatcagcagcagcgttatcacaagcctgggcgccatcgtgtcctgctacggcaaaaccaaatgcaccgccagcaacaagaacagaggcatcatcaaaaccttcagcaacggatgtgactacgtgagcaacaagggcgtggacaccgtgagcgtgggcaacaccctgtactacgtgaacaaactggaaggcaagaacctgtacgtgaaaggcgaacccataatcaactactacgaccctctggtgttccccagcgatgagttcgacgcctctatctctcaggtgaatgagaagatcaatcaatctctggccttcatccggcggagcgacgagctgttg

SEQ ID NO: 138 - DNA, 1401 bp, synthetic construct
  source 1..1401: mol_type = other DNA
caaaacatcaccgaggagttctaccagtctacctgtagcgccgtcagcagaggatacttctctgccctgagaaccggctggtatacaagcgtgatcaccattgagctgagcaacatcaaagaacccaagtgtaacggcaccgacaccaaggtgaagctgatcaaacaggagctggacaagtacaagaacgccgtgaccgagctgcagctgctgatgcagagcggaggccctggctcaggcggcggcggcagcggcggcggaggcagccggttccctcctttccccctgggcgtgggctccgctatcgccagcggaatcgctgtctctaaggtgctgcacctggaaggcgaggtgaacaagatcaagaacgccctgctgagcaccaacaaggccgtggtgtccctgtctaatggcgtatccgtgttgaccagcaaagtgctggatctgaagaactacatcaacaaccagctgctgcctattgtgaatcagcagtcctgcagaatctctcctattgaaaccgtgatcgagtttcagcagaaaaattccagactgctggaaatcacccgggagttcagcgttaatgctggcgtgaccacacctctgagcacctacatgctgaccaacagcgagctgctttctctgatcaatgatatgcctatcaccaacgaccagaagaagctgatgagcagcaacgtgcccatcgtgcggcagcaaagctacagcatcatgagcatcatcaaggaagaggtgctggcctacgttgtgcagctgcctatctacggcgtgatcgacacaccctgctggaagctgcacaccagccccctctgtacaaccaacatcaaggaaggaagcaacatctgcctgacaagaacagacagaggctggtactgcgacaacgccggcagcgtgtccttcttcccccaggccgatacatgcaaggtgcagagcaacagagtgttctgcgacaccatgaactccctgacactgccacctgaggtgagcctgtgcaacaccgatatcttcaacagcaagtacgactgcaaaatcatgacaagcaagaccgacatcagcagcagcgtgatcacaagcctgggcgccatcgtgagctgctacggaaagacaaagtgcaccgcctctaacaagaaccggggcatcatcaagacattcagcaatggatgtgattacgtgtctaacaagggcgtggacaccgtgtctgtgggcaacaccctgtattacgtcaacaaactggagggcaagaacctgtacgtgaaaggcgagcctattatcaattactacgatcctctggtgtttccatctgatgagttcgacgccagcatcagccaggtgaacgagaagatcaatcaaagcctcgcttttatcaggcgcagcgacgagctgctg

SEQ ID NO: 139 - DNA, 1401 bp, synthetic construct
  source 1..1401: mol_type = other DNA
cagaacatcacggaagagttctaccagtccacatgcagcgccgttagcagaggctacttctctgccctgagaaccggctggtataccagcgtgattaccatcgagctgagcaacatcaaggaacccaagtgcaacggcaccgacacaaaggttaaactgatcaagcaagagctggataagtacaagaacgccgtcaccgagctgcagctgctgatgcaaagcggcggtcctggatctggaggcggaggatctggcggcggaggcagcagattccctccattccccctgggcgtgggcagcgctatcgctagcggcattgccgtgtctaaggtgctgcacctggaaggcgaagtgaacaagatcaagaatgctctgctgtctacaaacaaggccgtggtgtccctgtccaatggcgtgtccgtgctgacaagcaaggtgctcgatctgaagaactacatcaacaaccagctgctgcctattgtgaatcagccttcttgcagaatctccaacatcgagacagtgatcgagtttcagcagaagaacagccggctgctggaaatcacccgggaatttagcgtgaacgctggcgtgaccacccctctgagcacatacatgctgaccaacagcgagctgctgagcttgatcaacgacatgcctatcacaaacgaccagaaaaagctgatgagcagcaacgtgcctatcgttagacagcaatcatatagcatcatgagcatcatcaaggaagaagtgctcgcctacgtggtccagctgcccatctacggcgtgatcgacaccccttgctggaagctgcacaccagccctctgtgcaccacaaatatcaaggagggcagcaatatctgcctgaccaggaccgacagaggctggtactgcgacaacgccggctctgtgtcgttcttcccccaggccgatacctgtaaagtgcagagcaaccgggtgttctgcgataccatgaactccctgacactgcctcctgaggtgtctctgtgtaatacagacatcttcaactccaagtacgactgcaagattatgaccagcaagaccgatatcagcagtagcgtgatcaccagcctgggagccatcgtgagctgctacggcaaaacaaagtgtaccgcctctaacaagaacagaggcatcatcaaaaccttcagcaacggctgtgactacgtgtctaacaaaggcgtcgacactgtgagcgtcggaaataccctgtactacgtgaacaagctcgaaggcaaaaatctgtacgtgaagggcgagcctatcatcaactactacgaccccctcgtgtttccatccgatgagttcgacgccagcatcagccaggtgaacgagaagatcaaccagagcctggccttcatccggagaagcgacgagctgctg

SEQ ID NO: 140 - DNA, 1401 bp, synthetic construct
  source 1..1401: mol_type = other DNA
cagaacatcacagaggagttctaccagtctacctgcagcgccgtgtccagaggctacttctctgctctgagaaccggctggtacaccagcgtgatcaccatcgagcttagtaacatcaaggaacctaagtgcaatggtacagacaccaaggtcaagctgatcaagcaggagctggacaagtataagaacgccgtgaccgagctgcagctgctgatgcagagcggcggccccgggtctggaggcggcggctccggaggcggaggatctagattcccacctttccctctgggcgtgggcagcgccattgctagcggcatcgccgttagcaaggttctgcacctggaaggagaagtgaacaaaatcaagaacgccctgctgagcaccaacaaggccgtggtgtccctgtctaacggcgtgtctgtgctgaccagcaaggtgctcgatctgaagaactacatcaacaaccagctgctccctatcgtgaatcaacaaagctgcagacccagcaacatcgagacagtgatcgagtttcagcaaaagaacagccggctgctggaaatcacaagagagtttagcgtgaacgctggcgtcaccacccctctgagcacctacatgctgacaaatagcgagctgctgtctttgatcaacgacatgcctatcaccaacgaccagaaaaagctgatgagcagcaatgtgcctattgtgcggcagcagagctacagcatcatgagcatcatcaaagaagaggtgctcgcctacgtcgtgcagctgcccatctacggcgtgatcgacactccatgttggaaactgcacacatctcctctgtgtaccaccaatatcaaggaaggcagcaacatctgcctgaccagaacagatcggggctggtactgcgacaacgccggctccgtgtccttcttcccccaggccgatacctgtaaagtgcagagcaacagagtgttctgcgacaccatgaacagcctgacactgcctccagaagtgagcctgtgcaacaccgacatcttcaacagcaaatacgactgcaagatcatgacatctaagaccgatatcagctctagcgtcattacatccctgggcgccatcgtgtcctgctacggcaaaaccaagtgcaccgccagcaacaagaaccggggcattatcaagaccttcagcaatggctgtgattatgtgtctaacaaaggcgtggacacagtgagcgtgggaaataccctgtactacgtgaacaagctggaaggcaagaacctgtacgttaagggcgagcctatcatcaattactacgaccccctggtgttccctagcgacgagttcgacgccagcatcagccaggtgaacgagaagatcaaccagagcctggcttttatccgcagaagcgatgagctgctg

SEQ ID NO: 141 - DNA, 1401 bp, synthetic construct
  source 1..1401: mol_type = other DNA
caaaacattaccgaggagttctaccagagcacctgcagcgccgtgagccggggctacttcagcgccctgagaaccggctggtacaccagcgtcatcacaatcgagctgagcaatatcaaggaacctaagtgcaacgggaccgacaccaaggtgaagctgatcaaacaggagctggataagtacaagaacgccgtgacagagctgcagctgctgatgcagagcggcggacctggctccggcggaggaggcagcggcggcggaggcagcagattccctccattcccactgggcgtgggctccgccatcgccagcggcatcgccgtgtccaaggtgctgcacctggaaggcgaagtgaacaagatcaagaacgctctgttaagcacaaacaaggccgttgtgtctctgagcaacggcgtgtctgtgcttacatctaaggtgctggacctgaagaattacatcaacaaccagctgctgcccatcgtgaaccagcaaagctgcagaatccccaacatcgagacagtgatcgagtttcagcagaagaacagcagactgctggaaatcactcgggaatttagcgtcaacgccggcgtgaccacacccctgagcacctacatgctgaccaatagcgagctgctgagcctcatcaatgacatgcctattaccaacgaccagaaaaagctgatgagcagcaacgtgcctattgtgcggcagcagtcctactctatcatgagcatcatcaaggaagaggtgctggcctacgtggtgcagctgccaatctacggcgtgatcgacacaccttgttggaagctgcacacctctcctctgtgtaccaccaacatcaaggagggctctaatatctgcctgacaagaacagatagaggctggtactgcgacaacgctggctcagttagcttcttcccccaggccgacacctgtaaagtgcaaagcaaccgggtgttctgcgataccatgaacagcctgacactgcctcctgaggtgagtctgtgcaacacagacatcttcaatagcaaatacgactgcaagatcatgaccagcaagaccgatatcagcagctctgtgatcacatctctcggcgctatcgtgtcgtgctacggcaagaccaagtgcaccgccagcaacaagaacagaggaatcatcaaaaccttcagcaatggttgtgactacgtgagcaacaagggggtcgacaccgtgtccgtcggcaacaccctgtactacgtgaacaaactggaaggcaaaaacctgtatgtgaagggcgagcctatcatcaactattacgatcctctggtgttccccagcgacgagttcgacgcctctatttctcaggtgaacgagaagatcaaccagtctctggcttttatcagaaggtccgatgagctgctg

SEQ ID NO: 142 - DNA, 1401 bp, synthetic construct
  source 1..1401: mol_type = other DNA
cagaacatcacagaggagttctaccagtctacctgcagcgccgtgtcccggggctacttcagcgccctgagaaccggctggtacaccagcgtgatcacaatcgagctgagcaatatcaaagaacctaagtgtaacggcaccgatacaaaggtgaagctgatcaaacaggagctggacaagtacaagaacgccgtgaccgagctgcagctgctgatgcagagcggcggacctggcagcggcggcggcggctctggcggcggcggttctcggttcccaccattccctctgggagtgggctctgccatcgcctctggcatcgccgtctccaaggtgctgcacctggaaggagaagtgaataagatcaagaacgctctgctgtctacaaacaaggccgtggtgtccctgagcaatggagtgtctgtcctgacctccaaagtgctggatctgaagaactacatcaacaaccagctgctccccatcgtgaaccaacagagctgcagaatccctcctattgaaaccgtgatcgagtttcagcagaagaacagcagactgctggagatcacccgggaatttagcgtgaacgctggcgttacgacacctctgagcacatacatgctgacaaacagcgagctgctgagcctgatcaacgatatgcctatcaccaacgaccagaaaaagctgatgagttctaatgtgcctatcgtgcggcagcaatcctacagcatcatgagcatcatcaaggaagaagtgctggcctacgttgtgcagctgcctatctacggcgtgatcgacaccccttgttggaagctgcacaccagccctctctgtacaaccaacatcaaagagggcagcaacatctgcctgaccagaacagatagaggctggtattgcgacaacgccggcagcgtcagcttcttcccccaggccgacacatgcaaagtgcagagcaatagagtgttctgcgacacaatgaacagcctgaccctgccccctgaggtgagcctgtgcaacaccgacatcttcaacagcaagtacgactgcaagatcatgaccagcaagacagatatcagcagcagcgtgattaccagcctgggcgccatcgtctcttgctacggcaaaaccaagtgcaccgccagcaacaagaacagaggcatcatcaagaccttcagcaacggttgtgattacgtgagcaacaagggagtggacaccgtgtccgtgggaaataccctgtattacgtgaacaagctggaaggcaagaacctgtacgtgaaaggcgagcccattatcaactactatgaccccctcgtgttccccagcgacgagttcgacgccagcatcagccaggtgaacgagaagatcaatcaaagtcttgcttttatcagaaggtccgacgagctgctc

SEQ ID NO: 143 - DNA, 1401 bp, synthetic construct
  source 1..1401: mol_type = other DNA
cagaacatcaccgaggagttctaccagagcacctgtagcgctgtgagccggggctacttcagcgccctgagaacaggctggtacaccagcgtgattacaatcgaactgtctaacatcaaggaacctaagtgcaacggaacagacaccaaggtgaagctgatcaagcaggagctggataagtacaagaacgccgttaccgagctgcagctgctgatgcagagcggcggtcctggcagcggaggaggcggcagcggaggcggcggcagtagattcctgggcttccccctgggagtgggcagcgctatcgcttctggaatcgccgtgtccaaggtcctgcacctgcccggcgaggtgaacaagatcaagaacgccctgctgagcacaaacaaggccgtggtgtccctgtccaacggcgtgagcgtgctgaccagcaaggtgctggacctgaagaactacatcaacaaccagctgctgcctatcgtgaaccagcagtcttgtagaatcagcaatatcgagacagtgatcgagtttcagcaaaagaacagcagactgctggaaatcaccagagagttctctgtgaacgctggcgtgaccacccctctgagtacctacatgctgaccaatagcgaacttctgagcctgatcaatgatatgcctatcacaaacgaccagaagaagctgatgagctccaatgtgcccattgtacggcagcagagctacagcatcatgtctatcattaaggaagaggtgctggcctacgtggtccagctgcctatctacggcgtgatcgacacaccttgttggaagctgcacaccagcccactgtgcacaaccaacatcaaagaagggagtaatatctgcctgaccagaacagatagaggctggtactgcgacaacgccggcagcgtgtccttcttccctcaggccgacacctgcaaggtgcaaagcaaccgggtgttctgcgatacaatgaacagcctgacactgccacctgaggtgtctctctgtaataccgatatctttaacagcaaatacgactgcaaaatcatgacctctaaaaccgacatctcaagctctgtgataaccagcctgggcgccatcgtgagctgctacggcaagacaaagtgcaccgccagcaataaaaacaggggcatcatcaagaccttcagcaacggctgcgactacgtgagcaacaaaggcgtggacaccgtgagcgtgggcaacaccctgtactacgtgaataagctggaaggcaaaaacctctacgtcaagggcgagcccatcatcaactattatgaccctctggtctttcccagcgacgagttcgacgcctctatctctcaggttaacgagaagatcaaccaaagcctggccttcatccggagaagcgatgagctgctg

SEQ ID NO: 144 - DNA, 1401 bp, synthetic construct
  source 1..1401: mol_type = other DNA
caaaacatcaccgaggagttctaccagagcacctgtagcgccgtgtcgcgcggctacttctccgccctgagaacaggctggtacaccagcgtgatcaccatcgagctgtctaacattaaagagcccaagtgcaacggcaccgataccaaggtgaagctaatcaagcaggagctggataagtacaagaacgctgtgacagagctgcagctgctgatgcagtctggaggacctggctctggtggcggcggaagtggaggcggaggcagcagattcccccccttcctgctgggcgtgggcagcgctatcgcctctggcatcgccgttagcaaggtgctgcacctgccaggcgaagtgaacaaaatcaagaacgctctgctgagcaccaacaaggccgtggtctctctgagcaacggcgtgagcgtgctgacatctaaagtgctggacctgaagaattacatcaacaaccagctgctccccattgtgaatcagcagagctgtagaatcagcaacatcgagacagtgatcgagtttcagcagaaaaattcaagactgctggaaatcacacgggaattttccgtgaacgccggcgttacaacccctctgtccacctacatgctgaccaacagcgagctgctgtccctgatcaacgacatgcctatcacaaatgatcagaagaagctgatgagctctaatgtgcctatcgtgcggcagcaatcatatagcatcatgagcatcatcaaggaagaagtgctggcctacgtggtgcaactgcctatctacggcgtgatcgacaccccatgttggaagctgcacacaagtcctctgtgcaccaccaacatcaaggaaggcagcaacatctgcctgactcggacagatagaggctggtattgcgataacgccggaagcgtgtccttcttccctcaggccgacacctgcaaggtccagagcaatagagtgttctgcgacacaatgaacagcctgacactgcctcctgaggtgtccctctgtaacaccgacatcttcaacagcaaatacgactgcaagatcatgaccagcaagaccgacataagcagcagcgtgatcaccagcctgggcgccatcgtgtcctgctacggcaaaaccaaatgcaccgccagcaacaagaacagaggcatcatcaagaccttcagcaacggctgcgactacgtgtctaacaagggcgtggacacagtgtctgtgggcaacaccctgtactacgtcaacaaactggaaggcaagaatctgtacgtcaagggcgagcctatcattaactactacgaccccctggtgttcccaagcgatgagttcgacgccagcatcagccaggtgaacgagaagatcaaccagagcctcgcttttatcagacggagcgacgagctgctg

SEQ ID NO: 145 - DNA, 1401 bp, synthetic construct
  source 1..1401: mol_type = other DNA
cagaacatcacggaagagttctaccagagcacctgtagcgccgtgtctagaggctacttcagcgccctgagaaccggctggtacaccagcgtgatcacaatcgagctgagcaacatcaaggaacccaagtgcaacggaacagacaccaaggtgaagctgattaagcaggagctggacaagtacaagaacgccgtgaccgagctgcagctgctgatgcagagcggcggacctggcagtggaggtggcggctctggcggcggaggcagcaggttcccaccattccccctgggcgtgggctctgctatcgcctccggcatcgccgtgagcaaggtgctccacctgcctggagaagtgaacaaaatcaagaacgccctgctgagcaccaacaaggccgtggtgtccctgtctaacggcgtttctgtgctgaccagcaaggtgctggatctgaagaattacatcaacaaccagctgctgcctatcgtgaaccagcagtcttgtagaatctccaacatcgaaaccgtgatcgaatttcaacaaaagaacagccggctgcttgagatcacaagagagttttcagtgaacgctggcgtgacaacccctctgtctacatacatgctgaccaatagcgagctgctctccctcatcaacgacatgcctatcaccaacgaccagaaaaagctgatgagcagcaatgtgcccatcgtcagacagcagagctacagcatcatgagcatcatcaaggaagaagtcctggcctacgtggtgcagctgcctatctacggcgttatcgacaccccttgttggaagctgcacacaagccctctttgtaccacaaacattaaagagggcagcaacatctgcctgactcggaccgatagaggctggtattgcgacaacgccggcagcgtgagcttcttcccccaggccgacacctgcaaggtgcagagcaaccgggtgttctgcgacaccatgaacagcctgaccctgccacctgaggttagcctgtgcaacaccgatatcttcaactctaaatacgactgcaaaatcatgacctccaaaacagatatcagctccagcgtgattacaagcctgggcgccatcgtgtcctgctacggcaagacaaagtgcaccgcctctaataaaaacagaggaatcatcaagaccttcagcaatggctgtgactacgtgagcaacaagggcgtcgacacagtgtccgtgggaaatacactgtactacgtgaataagctggaaggcaaaaacctgtacgtgaagggcgagcctatcatcaactactatgatcctctggtgtttcccagcgatgagttcgacgctagcatctctcaggtgaacgagaagatcaatcaatccctggctttcatccggagaagcgacgagctgctg

SEQ ID NO: 146 - DNA, 1401 bp, synthetic construct
  source 1..1401: mol_type = other DNA
cagaacatcaccgaggaattttaccagtccacatgcagcgccgtgtccagaggctacttctctgccctccggaccggctggtacaccagcgtgatcaccatcgagctgagcaacatcaaggaacctaagtgtaacggcaccgacactaaggtgaagctgatcaagcaggagctggacaagtacaagaatgctgttacagagctgcagctgctgatgcagagcggcggacctggatctgggggcggcggctctggcggcggcggaagcagattcctgggattccctctgggcgtcggaagcgcaatcgccagcggcatagctgtgtccaaggtgctgcacctgcccggcgaggtgaataaaatcaaaaatgccctgctgagcaccaacaaggccgtggtgtcactgagcaacggcgtgagcgtgctgaccagtaaagtgctggatctgaagaactacatcaacaaccagctgctgcctattgtgaaccagcagtcttgtagaatcagccctatcgagacggtgatcgaatttcagcaaaagaacagcagactgctggaaatcacaagggagttcagcgtcaacgctggcgtgaccacacctctgtctacatacatgctgaccaacagcgagctcctgagcctgatcaatgacatgcctatcaccaacgatcagaagaagctgatgagctctaacgtgcccatcgtgcggcaacagtcctacagcatcatgagcatcatcaaggaggaagtgctggcctacgtggttcaactgcctatctacggcgtgatcgacacaccctgctggaagctgcacaccagccctctgtgcacaacaaacatcaaggagggcagcaacatctgcctgacaagaaccgatagaggctggtactgcgataacgccggcagcgtgtccttcttcccccaggccgacacctgcaaagtgcagtccaacagagtgttctgcgacacaatgaacagcctgaccctgccacctgaggtgtctctttgcaacaccgacatcttcaactctaaatacgactgcaaaatcatgacctcaaagaccgacatcagcagctccgtcattacaagcctgggcgccatcgtgagctgctacggaaaaaccaagtgtaccgccagcaacaagaaccggggcattatcaaaaccttctccaatggctgtgactacgtgagcaacaagggcgtcgacaccgtgtctgtgggcaacaccctgtattacgtgaacaagctggaaggcaagaatctgtatgtgaagggagaacccatcatcaattactacgatcctctggtgtttccaagcgacgagttcgacgcctctattagccaggtgaacgagaagatcaaccagagccttgccttcatccgccggagcgatgagctgctg

SEQ ID NO: 147 - DNA, 1401 bp, synthetic construct
  source 1..1401: mol_type = other DNA
cagaacatcacagaggagttctaccagagcacctgcagcgccgtgagcagaggctacttcagcgctctgagaacaggctggtacacctccgtcatcaccatcgagctgtctaatatcaaggaacccaagtgcaatggcaccgacacaaaggtgaagctgatcaagcaggagctggacaagtacaagaacgccgtgaccgagttgcagctgctgatgcagagcggtggccctggcagtggcggcggcggaagcggaggcgggggcagccggttcccccccttcctgctgggagtgggcagcgctatcgcctctggaatcgccgtgtctaaggtgctgcacctgccaggcgaggttaacaaaatcaagaacgccctgctgagcacaaacaaggccgtcgtgtccctgagcaacggcgtgtctgtgctgacaagcaaggtgctggatctgaagaactacatcaacaaccagctgcttcctatcgtgaatcaacagagctgtagaatcagccctatcgaaaccgtgatcgagtttcagcaaaagaacagcaggctgctggaaatcacccgggagttcagcgtgaacgctggcgtgacaacccctctgagcacctacatgctgacaaactccgagctgctgtccctgatcaacgacatgcctatcacaaatgatcagaaaaagctgatgagcagcaacgtgcctatcgtgcggcagcagagctacagcatcatgagcatcatcaaagaagaggtgctggcctacgtggtgcagctgcctatctacggagtgatcgacacaccttgttggaagctgcacaccagccccctctgtaccaccaacatcaaagaaggcagcaatatctgcctgaccagaaccgatagaggatggtactgcgacaacgccggcagcgtctccttcttcccccaggccgacacctgtaaagttcaaagcaatagagtgttctgcgataccatgaacagcctgaccctgcctcctgaggtgtctctgtgcaacacagacatcttcaattctaaatatgactgcaagatcatgaccagcaagacagatatttcctctagcgtgattaccagcctgggcgccatcgtgagctgctacggcaaaaccaagtgcaccgcctctaacaagaacagaggcatcatcaagacttttagcaacggctgcgactacgtgtctaacaagggcgtcgacacagtgtctgttggcaacaccctgtattacgtgaacaagctcgaaggcaagaacctgtacgtgaagggagagcctatcatcaactactacgaccccctggtgtttccatccgacgagttcgacgccagcataagccaggtgaacgagaagatcaaccagagcctggcattcatccggagatctgatgagctgctg

SEQ ID NO: 148 - DNA, 1401 bp, synthetic construct
  source 1..1401: mol_type = other DNA
cagaatatcacagaggagttctaccaaagcacctgcagcgccgtgagccggggctacttctctgctcttagaacaggctggtacaccagcgtgatcaccatcgagctttctaacatcaaggaacctaagtgcaacggcaccgatacaaaagtcaagctgatcaagcaggagctggataagtacaagaacgccgtgaccgagctccagctgctgatgcagtccggcggacctggaagtggcggaggaggcagcggcggcggaggctccagattccctccattccccctgggcgtgggcagcgctatcgccagcggcatcgccgtgagcaaggtactgcacctgcccggcgaggtgaacaagatcaaaaacgccctgctgtctaccaacaaggccgtggtgagcctgagcaacggcgtgtctgtgctgacctccaaggtgctggacctgaagaactacatcaacaaccagctgctccccattgtgaaccagcagtcttgtagaatcagccccatcgagacagtgatcgaatttcagcagaagaacagcagactgctggaaatcaccagagaattttccgtcaacgccggcgtgacaacccctctgagcacctacatgctgacaaatagcgagctgctgagcctgatcaacgatatgcccattaccaacgaccagaaaaagctgatgagcagcaacgtgcctattgtgcggcagcaatcatatagcatcatgagcatcatcaaagaggaagtgctggcctacgtcgtgcagctgcctatctacggcgtgatcgacacgccgtgctggaagctgcacacctctcctctgtgcaccaccaatatcaaggaaggcagcaatatctgcctgacacggacagatagaggctggtattgcgacaacgctggcagcgtgagcttcttcccacaggccgacacatgtaaagtgcaaagcaatagagtgttctgcgacaccatgaacagcctgaccctgcctcctgaggtgagcctgtgtaataccgacatcttcaacagcaaatacgactgcaagatcatgacctccaagacagacatcagcagctctgttatcacttctctgggcgccatcgtgtcctgctacggcaagaccaagtgcacagcctctaacaaaaacagaggcatcatcaagaccttcagcaatggttgtgactacgtgtccaacaagggagtggacaccgtgtccgttggcaacaccctgtactacgtcaataagctggaaggcaagaacctgtacgtgaagggcgagcctattatcaattactacgatcctctggtgttccccagcgatgagtttgacgcctctatcagccaggtgaacgagaagatcaaccagtctctggccttcatcaggcggagcgacgagctgctg

SEQ ID NO: 149 - DNA, 1401 bp, synthetic construct
  source 1..1401: mol_type = other DNA
cagaacatcacagaagagttctaccagagcacatgcagcgctgtttcccgcggctacttcagcgccctgagaaccggctggtacaccagcgtgatcaccatcgagctgtcaaatatcaaagaacccaagtgtaatggcaccgacaccaaggtgaagctgatcaagcaggagctggataagtacaagaatgctgtgacagagctgcagctgctgatgcagagcggcggtcctggctctggcggaggcggctctggcggcggcggcagcagattcctgggcttccccctgggcgtgggaagcgccatcgcctccggcatcgccgtgagcaaggtgctgcacctgcctggagaggtgaacaagatcaagaacgccctgctgagcaccaacaaggccgtggtgagcctgtctaatggagtgtccgtgctgaccagcaaggtgctggacctgaagaactacatcaacaaccagctgcttccaatcgtgaatcaacaatcttgtagaatcagcaacatcgaaaccgtgatcgagtttcagcagaaaaacagcagactgctggagatcaccagagagttcagcgtgaacgccggcgtcacaacccctctgagcacatacatgctgaccaacagcgagctgctgtctctgatcaacgacatgcctatcaccaatgaccagaagaaactgatgtccagcaacgtgcccattgtgcggcagcagagctacagcatcatgagcatcatcaaggaggaagtgctcgcctacgtggtgcagctgcccatctacggcgtcatcgacaccccttgctggaagctccacacaagccctctctgtaccaccaacatcaaggaaggaagcaacatttgcctgacaagaaccgatcggggatggtattgcgacaacgctggctccgtctccttctttccacaggccgacacctgtaaagtgcagagcaaccgggtgttctgcgatacaatgaacagcctgactctgcctagcgaggtgtccctgtgcaacacggacatcttcaacagcaagtacgactgcaagatcatgacctctaagacagatatctcttcttctgtgattacctcgctgggcgccatcgtgagctgctacggcaaaaccaagtgcacagccagtaacaaaaacagaggcatcatcaagaccttcagcaacggctgcgactacgtgtctaacaaaggcgtcgacacagtgtccgttggaaataccctgtactacgtgaacaagctggaaggcaagaacctgtatgtgaagggcgagcctattatcaactactacgatcctctggtgttccccagcgatgagtttgacgcctctatcagccaggtgaacgagaagatcaatcagagcctggctttcatccggagaagcgacgaactgtta

SEQ ID NO: 150 - DNA, 1401 bp, synthetic construct
  source 1..1401: mol_type = other DNA
cagaacatcaccgaggagttctaccagtctacatgcagcgccgtgtctagaggctacttcagcgccctgcggaccggctggtatacatctgtgatcaccatcgaactgagcaatatcaaggaacctaagtgcaacggcaccgatacaaaggtgaaactgatcaagcaggagctggacaagtacaagaatgccgtgacagagctgcagctgctgatgcagagcggcggacctggcagcggcggcggcggaagcggcggcggaggcagcagattcctgggatttccactgggcgtgggcagcgctatcgcctccggcatcgccgtgagcaaggtcctgcacctgcctggcgaagtgaacaagatcaagaatgctctgctgagcaccaacaaggccgtcgtgtccctgtctaatggcgtgtctgtgctgacctctaaagtgctggacctaaagaactacatcaacaaccaactgctgccaattgtgaaccagcagagctgcagaatctctaatatcgagacagtgatcgagttccagcagaaaaacagccggctgctggaaatcaccagagagtttagtgtgaacgccggagttacaacccctctgtctacatacatgctgaccaacagcgagctgctttctctcatcaatgatatgcctatcacaaacgaccagaaaaagctgatgagcagcaacgtgcagatcgtgcggcagcaaagctacagcatcatgagcatcatcaaagaggaagtgctggcctacgtggtgcagctgcctatctacggcgtgatcgacacaccttgctggaagctgcacaccagccctctctgtaccaccaacattaaggaaggctctaacatctgcctgacaagaaccgatagaggatggtactgcgacaacgctggaagcgtgtccttcttcccccaggccgacacctgtaaagttcaaagcaaccgggtgttctgcgatacgatgaactctctgacactgccccccgaggtgtccctgtgtaataccgacatcttcaacagcaagtatgattgcaagatcatgaccagcaagaccgacatcagctccagcgtcatcaccagcctgggcgccatcgtgtcctgctacggcaaaaccaagtgcaccgcctctaacaagaacagaggaatcatcaaaaccttcagcaatggctgtgactacgtgtcaaacaagggcgtcgacaccgtgtccgtgggcaacacactgtactacgtgaacaagctggaaggcaagaacctgtacgttaagggcgagcctattatcaactactacgaccccctggtgtttcccagcgacgagttcgacgccagcatctcacaggtgaacgagaagatcaaccagagcctcgctttcatccgcagaagcgatgagctgctg

SEQ ID NO: 151 - DNA, 1401 bp, synthetic construct
  source 1..1401: mol_type = other DNA
cagaacatcacagaggagttctaccagtctacatgctctgccgtgtctagaggttacttcagcgccctgagaaccggctggtacaccagcgtgatcaccatcgagctctctaatatcaaggaacccaagtgcaacggcaccgacacaaaggtgaaactgatcaagcaggagctggataagtacaagaacgccgtgaccgagctgcagctgctgatgcagagcggcggtcctggcagcggcggaggcggcagcggaggcggcggcagcagattcctgggatttcccctcggagttggatctgctatcgcctctggcatcgccgtgtccaaggtgctgcacctgcccggcgaagtgaacaagatcaaaaacgccctgctgagcaccaacaaggccgtcgtgtccctgtccaacggcgtgtctgtcctgacctctaaggtgctggacctgaagaactacatcaacaaccagctgctgcctatcgtgaaccaacaatcttgtagaatctctcctattgaaaccgtgatcgagtttcagcagaaaaacagcagactgctggaaatcacccgggagttcagcgtgaacgccggcgttaccacacccctcagcacctacatgctgaccaacagcgagctgctgagcctgatcaacgacatgcctatcaccaatgaccagaagaagctgatgagcagcaacgtgcagatcgtgcggcagcagagctacagcatcatgagcatcatcaaagaagaggtgctggcctacgtggtgcagctgcctatctacggcgtcatcgacacaccttgctggaagctgcacacctcccctctgtgtacaaccaatattaaggaaggcagcaacatctgcctgacacggacagatagaggctggtattgcgacaacgctggcagcgtgtccttcttcccacaggccgatacttgtaaagtgcagagcaatagagtgttctgcgacaccatgaacagcctgacactgcctagcgaggtgtccctgtgcaataccgacatcttcaactctaagtacgactgcaagatcatgaccagcaagaccgatatcagctctagcgtgatcaccagcctgggcgccatcgtgagttgctacggcaagacaaagtgcaccgccagcaacaagaacagaggaatcatcaagaccttcagcaacggatgtgactacgtgagcaacaaaggcgtggacacagtgtccgtcggcaacaccctgtactacgtgaacaagctggagggcaaaaatctgtatgtgaagggcgagccaattatcaactactacgatcctctggtgttccccagcgacgagttcgacgccagcatcagccaggtgaacgagaagatcaatcaaagcctggcttttatcaggcggagcgatgagctgctg

SEQ ID NO: 152 - DNA, 1401 bp, synthetic construct
  source 1..1401: mol_type = other DNA
cagaacattactgaggagttctaccagtctacatgcagcgccgtgagcagaggctacttcagcgccctgcgcaccggctggtatacaagcgtgatcacaatcgagctgagcaacatcaaagagcccaagtgcaacggcaccgacaccaaggtgaagctgatcaagcaggagctggataagtacaagaatgctgtgacagagctgcagctgctgatgcagagcggcggccctggcagcggcggaggaggcagcggcggcggaggctctagattcctgggcttccctctgggagtgggatctgctatcgccagcggcatcgccgtgagcaaggttctgcacctgcccggcgaggtgaacaagatcaaaaacgccctgctgagcaccaacaaggccgtggtgtccctgtccaacggcgtgtccgtgctgacctctaaggtgctggacctcaagaactacatcaacaaccagctactgcctatcgtcaaccagcaaagctgtagaatcagccctatcgaaaccgtgatcgagtttcagcagaagaacagcagactgctggaaatcactcgggaattttctgtgaacgctggcgtgacaacccctctgagcacatacatgctgacgaacagtgaactgctgtcgctgatcaatgacatgcccatcaccaacgaccagaaaaagctgatgagcagcaacgtgcaaatcgttagacagcaatcctacagcatcatgtctatcatcaaggaagaggtgctggcctacgtcgtgcagctgcctatctacggcgtgatcgacacaccttgctggaagctgcacaccagccccctgtgcaccaccaacatcaaggaaggcagtaatatctgcctgaccagaaccgatagaggatggtactgcgacaacgccggcagcgttagcttcttcccccaggccgatacctgcaaggtgcagagcaaccgggtgttctgcgacaccatgaacagcctgaccctgccacctgaggtgtccctgtgtaataccgacatcttcaacagcaaatacgactgcaagattatgaccagcaaaaccgatatcagctccagcgtgataacaagcctgggcgccatcgtgagctgctacggaaagaccaagtgtaccgcctccaacaagaaccggggcatcatcaaaacattcagcaacggttgtgactacgtcagcaataaaggcgtggacacagtgtcggtcggcaacaccctgtactacgtgaacaagctggaaggcaagaacctgtacgtgaagggcgagcctatcatcaattactatgatcctctggtgttcccatctgacgagttcgacgccagcattagccaggtgaatgagaagatcaaccagtccctggcttttatccggagatctgatgagctgctg

SEQ ID NO: 153 - DNA, 1401 bp, synthetic construct
  source 1..1401: mol_type = other DNA
cagaacatcaccgaggaattttaccagtccacatgcagcgctgtatcccgcggctacttcagcgccctgcggaccggctggtatacctctgtgatcaccatcgagctgagcaatatcaaggaacccaagtgcaacggcaccgacacaaaggtgaagctcatcaagcaggagttggataagtacaagaacgccgtgacagagctgcagctgctgatgcagtctggcggacctggctctggcggaggcggctccggcggcggaggcagcagattccctcctttcctgctgggcgtgggatctgctatcgcctccggcattgctgtgagcaaggtgctgcacctgccaggcgaggtgaacaagatcaagaacgccctgctgagcaccaacaaagccgtggtgtctctgagcaatggcgtgtccgtgctgacatctaaggtcctggacctgaagaactacatcaacaaccagctgctgcctatcgtgaatcaacagagctgtagaatcagccctattgagacagtgatcgagtttcagcaaaagaactcccggctgctggaaatcacccgggagttcagcgtgaatgccggcgttacaacacctctgtctacctacatgctgaccaattcggagctgctgagcctgatcaacgacatgcctattacaaacgaccagaaaaagctgatgtctagcaacgtgcaaatcgtgcggcagcagagttatagcatcatgagcatcatcaaggaagaagtgctggcctacgtggtccagctgcctatctacggcgtgatcgacaccccttgctggaagctgcacacctctcctctttgcaccacaaacatcaaagaaggcagcaacatctgcctgaccagaaccgatagaggctggtactgcgacaacgctggcagcgtgagcttcttcccccaggccgatacatgcaaagtgcagagcaacagagtgttctgcgacaccatgaacagcctgaccctgccccccgaggtgagcctgtgtaacaccgatatcttcaactctaaatacgactgcaagatcatgaccagcaaaaccgacatcagcagcagcgtgatcaccagcctgggcgccattgtttcatgctacggcaagaccaagtgtactgccagtaacaagaacaggggcatcatcaagaccttcagcaatggatgtgattacgtcagcaataagggcgtggacacagtgagcgtgggtaacaccctgtactacgtgaacaaactggagggcaagaacctgtacgtgaaaggagagcctatcatcaactactacgaccccctggtgttcccaagcgatgagttcgacgcctccattagccaggtgaacgaaaagatcaaccagagcctggcctttatcagaagaagcgacgagctgctg

SEQ ID NO: 154 - DNA, 1401 bp, synthetic construct
  source 1..1401: mol_type = other DNA
cagaacatcaccgaggagttctaccagagcacctgcagcgccgtgagcaggggatatttcagcgctctgagaacaggctggtatacatctgtgatcaccatcgagctcagcaacatcaaagaacccaagtgcaacggtacagatacgaaggtcaagctgatcaagcaggagctggataagtacaagaacgccgtcaccgagctgcagctgctgatgcagagcggcggacctggcagcggcgggggaggaagtggcggcggcggctccagattccctcctttccccctcggcgtgggctccgccatcgccagcggaatcgccgtgtccaaagtgctgcacctgccaggcgaggtgaacaagatcaagaacgccctgctgagcacaaacaaggccgtggtgtccctgtctaatggcgtaagcgtgctgacctctaaggtgctggacctgaagaactacatcaacaaccagcttctgcctattgtgaaccaacaaagctgcagaatctcacccattgaaaccgtgatcgagttccagcagaagaacagccggctgctggaaatcacaagagagtttagcgtgaatgctggcgtgacaactcctctgagcacctacatgctgacaaatagcgagctgctgagcctgatcaatgatatgcctatcaccaatgaccagaaaaagctgatgagcagcaacgtgcagatcgtgcggcagcagagctacagcatcatgagcatcatcaaggaagaggtgctggcctacgtggtccagctgcccatctacggcgtgatcgacaccccttgttggaagctgcacacgagccctctgtgtaccaccaacatcaaggaaggctctaatatctgcctgaccagaaccgatagaggctggtactgcgacaacgcaggcagcgtgtccttcttcccacaggccgacacctgtaaagttcaatctaaccgggtgttttgcgacaccatgaactctttgaccctgcctccagaggtgtccctgtgtaataccgacatcttcaacagcaaatacgactgcaagatcatgaccagcaagacagacatcagctctagcgtgatcacaagcctgggcgccattgtgtcatgctacggcaagaccaagtgcaccgcctccaacaagaacagaggcatcatcaagaccttcagcaacggctgcgactacgtgtctaacaaaggcgtcgacacagtgagcgtgggcaacaccctgtactacgttaacaaactggaaggcaagaatctgtatgtgaagggagagcctattatcaactactacgatcccctggtgttccccagcgatgagttcgacgcctctatcagccaggtgaacgagaagatcaaccagagcctggcttttatccggagaagcgacgagctgctg

SEQ ID NO: 155 - DNA, 1401 bp, synthetic construct
  source 1..1401: mol_type = other DNA
caaaacatcacagaggaattttaccagagcacatgcagcgctgtctctagaggctacttcagcgccctgagaaccggctggtacaccagcgtcatcaccatcgaactgagcaacatcaaggaacctaagtgtaatggcaccgacacaaaggtcaagctgattaagcaggagctggataagtacaagaacgccgtgacagagctgcagctgctgatgcagtccggcggtcctggcagcggcggcggaggctctggcggaggcggcagcaggttccctccattccccctgggagtgggcagcgctatcgcttctggcatcgccgtgtccaaggtgctgcacctgcccggagaagtgaacaaaatcaaaaacgccctgctgagcaccaacaaggccgttgtgtccctgtctaatggcgtgtctgttctgaccagcaaggtgctggacctgaagaattacatcaacaaccagctgctgcctatcgtgaatcagcctagctgcagaatcagcaacatcgagacagtgatcgagtttcagcaaaagaacagccggctgctggaaatcacaagagagtttagcgtgaacgccggcgtgaccacccctctctctacatacatgctgaccaacagcgagctgctgtccctgatcaacgacatgcctatcaccaacgaccagaaaaagctgatgtcttctaacgtgcccattgtgcggcagcagagctacagcatcatgagcatcatcaaggaggaagtgctcgcctacgtggtgcagctgcctatctacggcgtgatcgacaccccatgttggaagctgcacacctctcctctgtgtacaaccaatatcaaggaaggcagcaacatctgcctgaccagaacagatagaggctggtattgcgacaacgccggaagcgtctccttcttccctcaggccgatacctgtaaagtgcagagcaatagagtgttctgcgatacaatgaacagcctgacactgccacctgaggtgtccctgtgcaacaccgatatcttcaacagcaaatatgactgcaagatcatgaccagcaagaccgacatcagcagctctgtgatcacctccctgggcgccatcgtgtcctgctacggcaaaaccaagtgcaccgccagcaataaaaaccggggcatcatcaaaaccttcagcaacggctgcgactacgtgagcaacaagggcgtggacaccgtgagcgtcggcaacacgctgtactacgtgaacaagctggaaggcaagaacctgtacgtgaagggagagcccatcatcaactactacgaccccctggtgttccccagcgatgagttcgacgccagcattagccaggtgaacgagaagatcaatcaatctctggccttcatccggagaagcgacgagctgctc

SEQ ID NO: 156 - DNA, 1401 bp, synthetic construct
  source 1..1401: mol_type = other DNA
cagaacatcacagaggagttctaccagagcacctgcagcgccgtgagccggggctacttcagcgctctgcggaccggctggtacaccagcgtgatcaccatcgagctgagcaacatcaaggaacccaagtgtaatggtacagatacaaaggtgaagctgatcaagcaggagctggataagtacaagaacgctgtgaccgagctgcagctgctgatgcagtctggaggccccggctctggcggcggcggaagcggaggcggcggaagcagattcccaccattccctctgggcgtgggcagcgccattgccagcggcatcgccgtgtcaaaggtcctgcacctgcctggcgaagtgaacaaaatcaagaacgccctgctcagcaccaacaaggccgtggtgtctctgagcaatggagttagcgtgctgaccagcaaggtgctggacctgaagaactacatcaacaatcagctgctgcctatcgtgaatcaacagagctgcagacctagcaacatcgagacagtgatcgaatttcagcagaagaatagcagactgctggaaatcacccgcgagttttctgtgaatgctggcgtgacaacacctctgtccacctacatgctgaccaacagcgagctgctctctctgatcaacgacatgcctatcaccaatgaccagaaaaagctgatgagcagcaacgtgcctattgtgcggcagcaatcttactccatcatgagcatcatcaaggaagaggtgctggcctacgttgtgcagctgcccatctacggcgttatcgacaccccttgctggaagctgcacaccagtcctctctgtacaaccaacatcaaagaaggcagcaacatctgcctgactagaaccgatagaggctggtattgcgacaacgccggcagcgtgtccttcttcccccaggccgacacctgtaaagtccagagcaacagagtgttctgcgacacaatgaacagcctgacactgcctcctgaggtgagcctgtgcaacaccgacatcttcaacagcaagtacgactgcaagatcatgacatctaagacagatatcagcagctctgtgatcacaagcctgggcgccatcgtgtcttgctacggaaaaaccaagtgcaccgccagcaacaagaaccggggcatcatcaagaccttcagcaacggttgtgactacgtgtccaacaaaggcgtcgacaccgtgtccgtgggcaacaccctgtattacgtgaacaagctggaaggcaagaacctgtacgtcaagggcgagcccatcatcaattactacgatcctctggtgttccccagcgacgagttcgacgcctctatttcccaggtgaacgagaagatcaaccaaagcctggcctttatcagaagatctgatgagctactg

SEQ ID NO: 157 - DNA, 1401 bp, synthetic construct
  source 1..1401: mol_type = other DNA
cagaacatcaccgaggagttctaccagagcacctgtagcgccgtgagccggggctacttctctgccctgagaacaggctggtacaccagcgtgatcaccattgaactgagcaacatcaaagagcctaagtgtaacggcaccgacaccaaggtgaagctgatcaagcaggagctggataagtacaaaaacgccgtgaccgagctgcagctgctgatgcagtctggcgggcctggctccggcggcggcggcagcggcggaggcggatctaggttccctcctttccctctgggagtgggcagcgctatcgccagcggcattgccgtgtccaaggtcctgcacctgccaggcgaggttaacaaaatcaagaacgctctgctgagcaccaacaaggccgtggtgtcactttctaatggagttagcgtgctgaccagcaaagtcctggacctgaagaattacatcaacaaccagctgctgcctatcgtgaatcaacaaagctgcagaatccccaacatcgagacagtgatcgagtttcagcagaagaacagcagactgctcgaaatcacccgggaattttctgtgaacgcgggcgtgacaacacctctgtcaacatacatgctgaccaacagcgagctgctgtctctgatcaatgacatgcctatcacaaatgatcagaaaaagctgatgagcagcaacgtgcctatagttagacagcagagctacagcatcatgtctatcatcaaggaagaggtgctcgcctacgtggtccaactacccatctacggagtgatcgacactccctgctggaagctgcacaccagccccctgtgcaccaccaacatcaaagaaggcagcaacatctgcctgacaagaaccgatagaggctggtattgcgacaacgctggcagcgtgtccttcttcccccaggccgatacctgcaaggtgcagagcaatagagtgttctgcgacaccatgaacagcttgaccctgcctcctgaggtgagcctgtgtaacaccgacatcttcaacagcaagtacgactgcaagatcatgacctccaagacagacatttctagctctgtgatcacctctctgggcgccatcgtgtcctgctacggcaagacaaagtgcaccgcctctaacaagaaccggggaatcatcaagaccttcagcaatggttgtgactacgtgagcaacaagggcgtcgacacagtgtccgtgggcaacacactctactacgtgaacaagctggaaggcaagaacctgtacgtgaaaggcgaacccatcatcaactactatgatcctctggtgtttccatctgatgagttcgacgccagcatcagccaggtgaacgagaagatcaaccagagcctggccttcatccggagaagcgacgagctgctg

SEQ ID NO: 158 - DNA, 1401 bp, synthetic construct
  source 1..1401: mol_type = other DNA
cagaacattacagaggagttctaccagagcacctgcagcgccgtgtcccgcggctacttcagcgctctgcggaccggatggtacaccagcgtgatcaccatcgagctgagcaacatcaaggaacccaagtgcaatggcaccgatacaaaggtaaagctgattaagcaggagctggataagtacaagaacgccgtgaccgagctgcagctgctgatgcagagcggcggacctggcagcggcgggggaggctctggaggcggcggcagcagattcccccccttccctctcggcgtgggctccgccatcgccagcggcatcgccgtgtcaaaggtgctgcacctgccaggcgaggtgaacaagatcaaaaacgccctgctaagcaccaacaaggccgttgtgtccctgtccaacggcgtgagcgtcctgacctctaaagtgctggacctgaagaactacatcaacaaccagctcctgccaatcgtgaaccagcagtcttgcagaatcccccctatcgagacagtgatcgagtttcagcagaaaaattctagactgctggaaatcacccgggaatttagcgtgaatgctggagtcaccacacctctgagcacctacatgctgacaaatagcgagctgctgagcctgatcaatgacatgcctataacaaacgaccaaaagaagctcatgagcagcaatgtgcctatcgttagacagcaatcctacagcatcatgagcatcatcaaggaagaagtgctggcttatgtggtgcagctgcctatctacggcgtgatcgacacgccctgctggaagctgcacacatctcctctgtgtacaaccaacatcaaagagggctctaacatctgcctgaccagaacagatagaggatggtactgcgacaacgccggcagcgtgtccttcttcccccaggccgacacctgtaaagtccagagcaaccgggtgttctgcgacaccatgaactctctgaccctgcctcctgaggtgtccctgtgcaacacagacatcttcaacagcaagtacgactgcaagatcatgaccagcaagacagacattagcagcagcgtgatcaccagcctgggcgccatcgtgagctgctacggcaaaacaaagtgtaccgccagcaacaagaacagaggcatcatcaagaccttcagcaatggatgtgattacgtgtctaacaaaggcgtggacaccgtgtccgttggcaacaccctgtactacgtgaacaagctggaaggcaagaatctgtacgtgaagggcgaacctatcatcaactactatgatcctctggtgtttccatctgatgagttcgacgcctctatcagccaggtgaacgagaagatcaaccaatctctggccttcatccggaggagcgacgagctgctg

SEQ ID NO: 159 - DNA, 1401 bp, synthetic construct
  source 1..1401: mol_type = other DNA
caaaacattacagaagagttttaccagagcacatgcagcgccgtgagccggggctacttcagcgctctgaggaccggctggtacacttctgtgatcaccatcgagctgtctaatatcaaggaacctaagtgcaacggtacagataccaaggtgaagctgatcaaacaggagcttgacaagtacaagaacgctgtcaccgagctgcagctgctgatgcagtcaggcggccccggcagcggcggaggaggcagcggcggcggcggcagcagattccctccattccctctgggagttggcagcgctatcgcctctggcatcgccgtgtctaaggtactgcacctgccaggcgaggtgaacaagatcaagaacgccctgctgagcaccaacaaggccgtcgtgagcctgtccaacggagtgtccgtgctgacaagcaaggtgctggacctgaagaattacatcaacaaccagctgctccctatcgtgaaccagcccagctgcagaatcagccctatcgagacagtgattgagtttcagcagaagaactctagactgctggaaatcacccgggagttcagcgtcaatgccggcgttacaacccctctttctacctacatgctgacaaacagcgagctgctgagcctgatcaacgacatgcccatcaccaatgatcagaaaaagctgatgtccagcaacgtgcctatcgtgcggcagcagagctacagcatcatgagcatcatcaaggaagaagtgctggcctacgtggtgcaactgcccatctacggcgtgatcgacaccccctgctggaagctgcacacctcgcctctgtgcaccaccaacataaaagagggcagcaacatctgcctgaccagaaccgatagaggctggtattgcgacaacgccggaagcgtgagcttcttcccccaggccgatacctgtaaagtgcagagcaatcgggtgttctgcgacaccatgaacagcctgaccctgcctccagaagtgtctctgtgtaataccgacatcttcaactctaagtacgactgcaaaattatgacaagcaagacagacatcagcagctctgtgatcacaagcctaggcgccatcgtgagttgctacggaaagaccaagtgtaccgcctctaacaagaacagaggcatcatcaagacattttctaacggctgtgactacgtgtctaacaagggagtggacacagtctccgtgggcaacacgctgtactacgtgaataaactggaaggcaagaacctgtatgtgaaaggcgagcctatcatcaactactacgatcctctggtgttccctagcgacgagttcgatgccagcatctcccaggtgaacgagaagataaaccaatccctggccttcatcagaagaagcgacgagctgctg

SEQ ID NO: 160 - DNA, 1401 bp, synthetic construct
  source 1..1401: mol_type = other DNA
cagaacatcaccgaggagttctaccagagcacctgttctgccgtgtcccggggctacttcagcgcccttagaaccggctggtacaccagcgtgattacaatcgagctgagcaacatcaaggaacctaagtgcaatggcaccgataccaaggttaagctgatcaagcaggagctggacaagtacaagaacgctgtgaccgagctgcagctcctgatgcagtcaggcggaggaggcagcggaggcggcggctccggcggcggaggaagcagattcccccccttccctctgggcgtgggctctgcaatcgccagcggcatcgccgttagcaaggtgctgcacctgcccggcgaggtgaacaaaatcaaaaacgccctgctgagcacaaacaaggccgtggtgtctctgagcaatggcgtctccgtgctgacatctaaggtgctggatctgaagaactacatcaacaaccagctgctccccatcgtgaatcaacagagttgcagaatttctaacatcgagacagtgatcgagtttcagcagaaaaatagcagactgctggaaatcacccgggaattttctgttaatgctggcgtgacaacccctctgtctacctacatgctgaccaacagcgagctcctgagcctgatcaacgacatgcctatcaccaatgaccagaagaagctgatgagcagcaacgtgcctatcgtgcggcagcaaagctacagcatcatgagcatcataaaagaagaagtgctggcctacgtggtccagctgccaatctacggcgtgatcgacacaccttgttggaagctgcacaccagccctctgtgtacgacaaacatcaaggaaggcagcaacatctgcctgactcggaccgatagaggatggtattgcgacaacgccggctctgtgtccttcttcccacaggccgatacatgcaaagtgcagtccaacagagtgttctgcgacaccatgaacagcctgacactgcctcctgaggtgtccctgtgcaacacagacatcttcaacagcaagtacgactgcaagatcatgacaagcaagaccgacatcagcagttctgtgatcaccagcctgggagccatcgtgagctgctacggcaaaaccaagtgcaccgcctctaacaagaatagaggcatcatcaaaacattcagcaacggttgtgactatgtcagcaacaaaggcgtggacaccgtgtccgtgggcaacaccctgtactacgtgaacaagctggaaggcaagaacctgtacgtgaagggcgagcctattatcaactactatgatcctctggtgttccccagcgacgagttcgacgccagcatcagccaggtgaacgagaagatcaatcaaagcctggcttttatcagaaggtctgatgagctgctg

SEQ ID NO: 161 - DNA, 1401 bp, synthetic construct
  source 1..1401: mol_type = other DNA
cagaacatcaccgaggagttctaccagagcacctgtagcgctgtgtcccggggctacttcagcgctctgagaacaggctggtacaccagcgtgatcaccatcgagctttctaatatcaaggaacccaagtgcaatggtacagacaccaaggtgaagctgatcaagcaggagctggataagtacaagaatgccgtcacagagctgcagctgctgatgcagtccggcggcggcggcagcggaggcggcggcagcggcggaggaggctctagattccctccattccccctgggcgtcggcagcgccattgcctctggaatcgccgtgagcaaggtgctgcacctggagggcgaggtgaacaagatcaagaacgccctgctgagcacaaacaaggccgtggtcagcctgagtaacggcgtgtccgtcctcacttccaaggtgctggacctgaagaactacatcaacaaccagctgctgcctatcgtgaaccaacaaagctgccgcatcagcaatatcgaaaccgttatcgagtttcagcagaaaaacagccggctgctggaaatcacacgggaatttagcgtgaatgctggcgtgacaacccctctgtctacatacatgctgacaaacagcgagctgctgtccctgatcaacgacatgcctattaccaatgatcagaagaagctgatgagcagcaacgtgcctatcgtgagacagcagagctacagcatcatgagcatcatcaaggaggaagtgctggcttacgtggtgcagctgcccatctacggcgttatcgacaccccatgttggaagctgcacaccagccctctgtgtaccaccaacatcaaggaaggcagcaacatctgcctgacaagaaccgatagaggctggtattgcgacaacgccggatctgtgagcttcttcccccaggccgatacctgcaaggtccaaagcaacagagtgttctgcgacacaatgaacagcctgaccctgcctcctgaggtgtctctgtgcaataccgatatcttcaactccaaatacgactgcaagatcatgaccagcaagaccgacatctctagcagcgtgatcacatctctgggcgccatcgtgtcctgctacggcaaaaccaagtgcaccgccagcaacaagaaccggggaattatcaagaccttcagcaatggatgtgactacgtgagcaacaaaggcgtggacaccgtgtctgtgggcaacaccctgtactacgttaacaaacttgaaggcaagaacctgtacgtgaaaggcgagcctatcattaattactatgatcccctggtgtttcctagcgatgagttcgacgcctctatctcccaggtgaacgagaaaatcaaccagagcctggccttcatcagaagatccgacgagctgctg

SEQ ID NO: 162 - DNA, 1401 bp, synthetic construct
  source 1..1401: mol_type = other DNA
cagaacatcacagaggagttctaccaaagcacctgcagcgccgtgtctagaggctacttcagcgccctgagaacaggctggtataccagcgtgatcaccatcgagctgtccaacatcaaagagcctaagtgcaacggcaccgacaccaaggtcaagctgatcaagcaggagttggataagtacaagaacgccgtgaccgagctgcagctgctcatgcagagcggcgggggcggctccggcggcggaggcagcggcggaggcggcagcagattccctcctttccccctgggcgttggcagcgctatcgcttctggcatcgccgtgtctaaggtgctgcacctgcctggcgaggtgaacaagatcaagaatgccctgctgagcacaaacaaagccgtcgtgagcctgtctaacggcgtgtccgtgctgacatctaaggtgctggacctgaagaactacatcaacaaccagctgctgcctattgtgaaccagcaaagttgtagaatcagccccatcgaaaccgtgatcgagtttcagcagaaaaacagcagactgctggaaatcactcgggaattttcagtgaatgccggcgtgaccacccctctgagcacatacatgctgaccaatagcgagctgcttagcctgatcaacgacatgcctatcaccaatgaccagaagaagctgatgtctagcaacgtgcccattgtgcggcagcagagctacagcatcatgagcatcatcaaggaagaggtgctggcttatgtggtgcaactgccaatctacggcgtgatcgacacgccttgctggaagctgcacaccagccctctgtgtaccaccaacatcaaagagggctccaatatctgcctgaccagaacagatagaggctggtactgcgacaacgccggaagcgtgagttttttcccacaggccgacacctgtaaagtgcagtccaatagagtgttctgcgacaccatgaacagcctgacactgcccccggaagtgagcctgtgcaataccgatatcttcaacagcaagtacgactgcaagattatgaccagcaagacagacatcagctctagcgtgatcacatctctgggagccatcgtgtcctgctacggcaagaccaagtgcaccgccagcaacaaaaaccgcggaatcatcaaaacattcagcaacggttgtgattacgtctccaacaagggcgtggacacagtgagcgtgggcaacaccctgtactacgtcaacaaactggaaggaaagaacctgtacgtgaagggagaacctatcatcaattactatgatcctctggtgttccccagcgatgagttcgacgcctccatctctcaggtgaacgagaagatcaaccagtctctggctttcatccggcggagcgacgagctgctg

SEQ ID NO: 163 - DNA, 1401 bp, synthetic construct
  source 1..1401: mol_type = other DNA
cagaacatcaccgaggagttctaccagagcacctgttctgccgtgtccagaggatacttctcagccctgagaaccggctggtatacatccgtgatcacaatcgagctttctaacatcaaggagcctaagtgcaacggtacagacacaaaggtgaagctgatcaaacaggagctggataagtacaagaacgccgtgaccgagctgcagctgctgatgcagagcggcggcggaggctctggaggcggcggcagcggcggcggcggcagcagattccctcctttccccctgggcgtcggctctgctatcgcctctggcatcgccgtgtctaaggtgctgcacctggaaggcgaggtgaacaagatcaagaacgctctgctgagcaccaacaaggccgtggtctccctgagcaatggcgtgagcgtgctgacaagcaaggtgctggacctgaaaaattacatcaacaaccagctgctgcctatcgtgaaccagcagagctgcagaatcagccctatcgagacagtgattgagtttcagcaaaagaacagccggctgctggaaatcactcgggaatttagcgtcaatgccggcgtgacaacccctctgagcacctacatgctgacaaatagcgagctgctgtccctcatcaatgatatgcctattaccaacgaccagaaaaagctgatgagcagcaacgtgcccatcgtgcggcagcaaagctacagcatcatgagcatcatcaaggaagaggtgctcgcctacgtggtgcaactgcctatctacggagttatcgataccccttgctggaagctgcacaccagccccctgtgtaccaccaacatcaaggaaggctctaatatctgcctgactagaacagacagaggctggtactgcgacaacgctggcagcgtgtccttcttcccacaggccgacacctgcaaggtgcagagcaaccgggtgttttgtgacaccatgaactctctgaccctgcctccagaggtgagcctctgcaacaccgacattttcaacagcaaatacgactgcaagatcatgaccagcaagacagatatctccagcagcgtgatcacatctctgggagccatcgttagctgctacggcaagacaaaatgcaccgcctccaacaaaaatagaggcatcatcaaaaccttctccaatggctgtgattacgtgagcaacaagggcgtggacaccgtgagcgtgggcaacaccctgtattacgtgaacaagctggaaggaaagaacctgtacgttaagggagaacctattatcaactactacgaccccctggtgttcccctctgacgagttcgacgccagcatcagccaggtgaacgagaagatcaaccagtccctggcgttcatccgcagaagcgatgagctgctg

SEQ ID NO: 164 - DNA, 1401 bp, synthetic construct
  source 1..1401: mol_type = other DNA
caaaacatcacagaggagttctaccagtctacctgtagcgccgtgtccagaggctatttctctgctctgagaaccggctggtacaccagcgtgatcaccatcgagctgagcaacatcaaggagcctaagtgcaatggcaccgacacaaaggtgaagctgatcaagcaggagctggataagtataagaacgccgtcaccgagctgcagctgctgatgcagtctggcggtggcggcagccctggaggcggatctggcggcggcggcagcagattcctgggcttccccctgggagtgggcagcgccatcgctagcggcatcgccgtgagcaaggttctgcacctggagggcgaggtgaacaagatcaagaacgccctgctgagtacaaataaggctgtcgtgagccttagcaatggagtgtctgtgctgacatccaaggtgctggacctgaaaaattacatcaacaatcagctgctccccattgtgaaccagcagagctgccggatcagccctatcgaaaccgtgatcgagttccagcaaaaaaacagcagactgctggaaatcacccgggaatttagcgtaaacgccggcgtgaccacccccctgtccacctacatgctgaccaacagcgagctcctgtctctgatcaatgacatgcctatcaccaacgaccagaagaaactgatgagcagcaacgtgcctatcgtgcggcagcaaagctacagcattatgagcatcatcaaggaagaggtgctggcctacgtggtgcagctgcctatttacggcgtgatcgacaccccttgctggaagctgcacaccagcccactgtgcaccacaaacatcaaggaaggctccaacatctgcctgacacgcaccgatagaggctggtactgcgacaacgccggcagcgtcagcttcttcccccaggccgacacctgcaaggtgcagtccaacagagtgttctgcgatacaatgaacagcctgacactgcctcctgaggtgtctctctgcaacaccgacatcttcaactctaagtatgactgcaaaatcatgacctctaagacagatatctcttctagcgtgatcactagcctgggcgccatcgtgagctgttacggcaagaccaagtgtacagcctctaataagaatagaggaattatcaagaccttcagcaacggatgtgactacgtgagcaacaagggcgtggacacagtgtcagtcggcaacaccctgtactacgtgaacaagctggaaggaaaaaacctgtacgtgaaaggagaacctatcatcaactactacgaccccctggtgtttccaagcgacgagtttgatgccagtatcagccaggtgaacgagaagatcaaccagtccctggctttcatcagacggagcgatgagctgctg

SEQ ID NO: 165 - DNA, 1401 bp, synthetic construct
  source 1..1401: mol_type = other DNA
cagaacatcaccgaggaattttaccagagcacatgcagcgccgtgtccagaggctacttcagcgctctgcggaccggctggtacaccagcgtgatcacaatcgagctgagcaacatcaaggaacccaagtgcaacggcaccgacaccaaggtgaaactgatcaaacaggagctggataagtacaagaatgccgtgacagagctgcagctgctgatgcagagcggaggaggcggtcctggcggcggcggcagcggcggaggaggctcccggtttcctcctttcctgctcggcgtgggatctgctatcgccagcggaatcgccgtctctaaggtgctgcacctggaaggcgaagtgaacaagatcaagaacgccctgctgtctacaaacaaggccgtggtgtccctgagcaatggcgtctccgtgctgactagcaaggttctggacctgaagaactacatcaacaaccaactgctccctatcgtgaaccagcaatcttgtagaatcagccccattgagaccgtgatcgagttccagcagaaaaactctagactgctggaaatcacccgggaatttagcgtgaatgctggcgttacaacacctctgagcacatacatgctgacaaatagcgagctgctgagcctgatcaatgacatgcctatcaccaacgatcagaagaagctgatgtctagcaatgtgcctatcgtgagacagcagtcatattctatcatgagcatcatcaaggaagaggtgctggcctacgtcgtgcagctgccaatctacggcgtgatcgacaccccctgctggaagctgcacaccagccctctgtgtaccacgaacatcaaggagggctctaatatttgcctgaccagaacagatagaggctggtactgcgataacgccggaagcgtgtctttcttcccccaggccgacacctgtaaagtgcagagcaacagagtgttctgcgacacaatgaactcgctgaccctgccacctgaggtgtctctttgtaacaccgacatcttcaatagcaagtacgactgcaagatcatgacctctaaaaccgatatcagcagcagcgtgatcacaagcctgggcgctatcgtgagctgctacggcaagaccaagtgcaccgcctctaacaagaaccgcggcatcatcaaaaccttcagcaacggctgcgactacgtgtccaacaaaggcgtggacaccgtgtccgtgggcaacaccctgtactacgtgaacaagctggaaggcaagaacctgtatgtgaagggcgagcctattatcaactactacgaccccctggtgttccctagcgatgagttcgacgccagcatcagccaggtgaacgagaagatcaatcaaagcctggccttcatccggagaagcgacgagctgctg

SEQ ID NO: 166 - DNA, 1401 bp, synthetic construct
  source 1..1401: mol_type = other DNA
cagaacatcaccgaggagttctaccagagcacctgtagcgccgtgagccggggatatttcagcgctctgagaaccggctggtacaccagcgtgataacaatcgaactgagcaacatcaaggaacctaagtgtaacggcaccgacaccaaggtgaagctgatcaagcaggagctggacaagtacaagaatgccgttacagagctgcagctgctgatgcagagcggcggcggcggccctggaggcggccccagcggaggaggaggtagccggtttcctccattcccactgggcgttggcagcgccatcgcctctggcatcgccgtgtccaaggtgctgcacctggaaggcgaagtgaacaagatcaagaatgccctgctgtctaccaacaaggccgtggtgagcctgagcaatggcgtcagcgtcctgaccagcaaggtgctggatctgaagaactacatcaacaaccagctgctgccaattgtgaaccagcaatcttgtagaatctcccctatcgagacagtgatcgaatttcagcagaagaacagcagactgctggagatcacaagggagttcagcgttaatgctggcgtgaccacacctctgagcacctacatgctgaccaattctgagctgctgagcctgatcaatgacatgcctatcaccaacgaccagaaaaaactgatgagcagcaacgtgcccattgtgcgccagcagtcctacagcatcatgagcatcatcaaggaagaggtgctggcttacgtcgtgcaactgcccatctacggcgtgatcgacactccctgctggaagctgcacacctcacctctctgtacaaccaacatcaaagagggatctaacatctgcctaacacggaccgacagaggatggtactgcgacaacgccggctctgtgtccttcttcccccaggcagatacatgtaaagtgcagtctaatagagtgttctgcgatactatgaactctttgacactgcctcctgaggtgtctctgtgcaacaccgatatcttcaacagcaaatacgactgcaagatcatgacctctaaaaccgacatcagcagcagcgtgattacaagcctgggcgctatcgtgtcctgctacggcaaaaccaagtgcaccgcctccaacaaaaacagaggtatcatcaagacctttagtaacggctgcgactacgtctccaacaagggcgtggacacagtgagcgtgggcaacacactgtattacgtgaacaagctggaaggcaagaacctgtacgtgaagggcgagcctattatcaattactacgatcctctcgtgttccctagcgatgagttcgacgccagcatcagccaggtgaacgagaagatcaaccaaagcctggccttcatccggagaagcgacgagctgctg

SEQ ID NO: 167 - DNA, 1464 bp, synthetic construct
  source 1..1464: mol_type = other DNA
caaaacatcaccgaagagttctaccagagcacatgcagcgctgtttccagaggctacttcagcgcactgagaacaggctggtatacctctgtgattacaatcgagctttctaacatcaaggaacccaagtgtaacggcacggatacaaaagtgaagctgatcaagcaggaactggataagtacaagaacgccgtgaccgagctgcagctgctgatgcagaacacccctgctgccaacaacagagccagaagagaagcccctcagtacatgaactacactatcaataccacaaagaacctgaacgtgagcatctccaagaaacgcaagcggaggttcctgggatttctgctgggagtgggtagcgctatcgccagcggcatagccgtgagcaaggtgctgcacctgcccggcgaggtgaacaagatcaagaacgccctgctgagcaccaacaaggccgtggtgagcctgagcaacggcgtgagcgtgcttacatccaaggtgctggacctgaagaactacatcaacaaccagctgctgcccatcgtgaaccaacagagctgcagaattagcaacatcgaaaccgtgatcgagtttcagcaaaagaacagcagactgctggaaatcaccagagagttcagcgtcaatgccggcgtcaccacccctctgagcacatacatgctgaccaatagcgaactgctgagcctgatcaacgacatgcctattaccaacgatcagaaaaagctgatgagcagcaatgtgcctatcgtgcggcagcagagctacagcatcatgagcatcatcaaagaggaagtgctggcctacgtggtgcagctgcctatctacggcgtgatcgacacaccttgctggaaactgcacaccagccccctgtgtacaaccaatatcaaggaaggcagcaatatctgcctaacaagaaccgacagaggctggtactgcgacaacgctggctctgtgtccttcttcccacaggccgacacctgcaaggttcagtctaatagagtgttctgcgacaccatgaactctctgaccctgccacctgaggtctccctgtgcaacacagatatcttcaacagcaaatacgactgcaagatcatgacctccaagaccgatatcagttcaagcgtgatcacaagcctgggcgccatcgtgagctgttatggcaaaaccaagtgcaccgcctctaacaaaaaccggggcatcatcaagaccttctctaacggatgtgactacgtgtccaacaagggcgtcgacaccgtgtcggttggcaacaccctgtactacgtgaacaagctggagggcaagaatctgtacgtgaagggagagcctatcatcaactattacgatcctctggtgtttcccagcgacgagttcgacgccagcatcagccaggtgaatgagaagatcaaccagagcctggccttcatccggcggagcgacgagctgctg

SEQ ID NO: 168 - DNA, 1464 bp, synthetic construct
  source 1..1464: mol_type = other DNA
caaaatatcaccgaggagttctaccagagcacctgcagcgctgtgagccgcggctacttcagcgccctgaggaccggctggtacaccagcgtgatcaccatcgaactgtctaacatcaaagagcccaagtgtaatggaaccgataccaaggtgaagctgatcaaacaggagctggacaagtacaagaacgccgtgaccgagctgcagctgctgatgcagaatacccctgccgccaacaacagagccagacgggaagcccctcagtacatgaactacaccatcaacaccacaaagaacctgaacgtgtccatctccaagaagcggaagcggagattcctgggcttcctgctgggcgtgggatctgctatcgcctctggcatcgccgtgtctaaagtgctgcacctgccaggggaggtgaataagatcaagaacgccctgctgtctacaaacaaggccgtggtcagcctgtccaatggcgtgtccgtgctgaccagcaaggtgctggatctgaagaactacatcaacaaccagctgctcccaattgtgaaccagcaatcctgcagaatctcccctatcgagacagtcatcgaatttcagcagaagaacagcagactgctggaaatcacaagagagttcagcgtgaacgccggagtgaccaccccactgagcacatacatgctgacaaacagcgagctgctgagcctgattaacgacatgcctatcacaaacgaccagaaaaagctgatgagcagcaacgtgcccattgtgagacagcagtcatatagcatcatgagcatcatcaaagaggaagtgctcgcctacgtggtgcagctgcctatctacggcgtgatcgacacaccttgttggaagctgcacacctcccctctgtgtaccacaaacatcaaggaaggctccaatatctgcctgacaagaaccgatagaggctggtattgcgacaacgctggcagcgtgtctttcttcccccaggccgacacatgcaaggtgcagagcaacagagtgttctgcgacacaatgaacagcctgaccctgccccccgaggtgagcctgtgcaacaccgacatcttcaactctaagtacgactgcaagatcatgaccagcaaaaccgatatcagcagtagcgtgattaccagcctgggcgccatcgtgagctgctacggcaagaccaagtgcaccgccagcaacaaaaacagaggcatcatcaagacattttctaacggctgtgactacgttagcaacaagggcgtcgacaccgtaagcgtgggcaacaccctgtactacgtgaataagctggaaggaaagaacctttacgttaaaggcgagcctatcatcaactactacgatcctctggtgttcccttctgatgagttcgacgccagcatcagccaggtgaatgagaagattaatcaatctctggcttttatccggcggagcgacgagctgctg

SEQ ID NO: 169 - DNA, 1464 bp, synthetic construct
  source 1..1464: mol_type = other DNA
cagaatatcacggaggagttctaccagagcacatgcagcgccgtctccagaggctacttcagcgctctgagaaccggatggtataccagcgtgatcacaatcgagctgagcaacatcaaagagcctaagtgcaacggtacagatacaaaggtgaagctgattaagcaggagctggataagtacaagaacgccgtgaccgagctgcagctgctgatgcagaacacccctgccgccaacaaccgggcccggagagaggcccctcaatacatgaactacaccatcaataccacaaaaaatctgaacgtgtccatcagcaagaagagaaagcgcagattcctgggatttccactgggcgtgggctctgctatcgccagcggcatcgccgtgtccaaggtgctgcacctgcccggcgaggtgaacaagatcaagaacgccctgctgtctacaaacaaggccgtggtgtctctgagcaacggcgtgtctgtgctcacaagcaaagtgctcgacctgaagaactacatcaacaaccagctgctccctatcgtgaaccagcaaagctgtagaatctctcctatcgaaaccgtgatcgagttccagcagaaaaacagcagactgctggaaatcacaagggagttcagcgtcaatgctggcgtcaccacccctctgagcacctacatgctgacaaacagcgagctgctgagcctgattaatgacatgcctatcaccaacgaccagaagaaactgatgtctagcaatgtgcccatcgtgcggcagcaaagctacagcatcatgagcatcataaaagaagaagtgctggcctacgtggtgcagctgcctatctacggcgtgatcgacaccccctgctggaagctgcacaccagccccctgtgcaccacaaacatcaaggagggcagcaacatttgtctgaccagaaccgatagaggctggtactgcgacaacgccggcagcgtttcattcttccctcaggccgacacatgcaaggtgcagagcaatcgggtgttctgcgacaccatgaacagcctgaccctgccacctgaagtgtcgctgtgtaacacagacatcttcaactccaaatacgactgcaagatcatgaccagcaaaaccgacatcagctctagcgtcatcaccagcctgggcgccatcgtgtcctgctacggcaagaccaagtgcaccgccagcaacaagaatagaggaatcatcaagactttttctaacggctgtgattacgtgtccaacaaaggcgtggacaccgtgagcgtgggaaataccctgtactacgtgaacaagctggaaggcaagaacctgtacgttaagggcgaacccatcatcaactattatgatcctctggtgttccccagcgatgagttcgacgcctccatctctcaggtgaacgagaagatcaaccagtctcttgcttttattagacggagcgacgagctcctg

SEQ ID NO: 170 - DNA, 1464 bp, synthetic construct
  source 1..1464: mol_type = other DNA
caaaacatcacggaagaattttaccagtccacctgcagtgccgtgtccagaggatatttcagcgccctgaggaccggctggtacaccagcgtgatcacaatcgagctgagcaatatcaaggaacccaagtgcaatgggaccgataccaaggtgaaactcatcaagcaggagctggataagtacaagaacgctgtgaccgagctgcagttgctgatgcagaacacccctgccgccaacaacggctctgctagcgaggcccctcagtacatgaactacaccatcaataccacaaagaacctgaacgtgagcatcagcaagaaaggaaagggcagatttctgggcttcctgctgggcgtgggctctgccatcgcctctggcatcgccgtgagcaaagtgctgcacctgcctggagaagtgaacaaaatcaagaacgctctgctgagcaccaacaaggccgtggtgagcctgagtaatggcgtgagcgtgctgacctctaaggtgctggacctgaagaactacatcaacaaccagctgctgcccattgtgaaccagcaatcgtgcagaatctctaacatcgaaaccgtgatcgagtttcagcagaagaacagccggctgctggaaatcacacgggagttcagcgtgaatgccggcgtgacaacacctctgtccacctacatgctgacaaactccgagctgctgagcctgatcaatgatatgcctatcaccaacgaccagaaaaagctgatgagcagcaacgtgcccatcgtgcggcagcagagctacagcatcatgagcattattaaggaggaagtgctggcctacgtcgtccagctgccaatctacggcgtgatcgacaccccatgttggaagctgcacaccagccctctgtgtaccaccaacatcaaagaaggcagcaacatctgcctgaccagaaccgacagaggctggtattgcgataacgctggcagcgtgtccttcttcccccaggccgatacatgtaaagtgcagagcaacagagtgttctgcgacacaatgaacagcctgaccctgcctcctgaggtgtccctgtgtaacacagacatcttcaactctaagtacgactgcaagatcatgaccagcaagaccgacatctcttctagcgtcatcaccagcctcggcgccatcgtgtcatgctacggcaagaccaagtgcacagccagcaacaagaatcggggaataatcaaaaccttctctaacggctgcgactacgtgagcaacaaaggcgtcgacacagtgtcggttggaaatacactgtactacgtgaacaagctggagggcaagaatctgtacgtcaagggcgagcctatcatcaactattacgaccccctggtgttccctagcgacgagttcgacgccagcatcagccaagtgaacgagaagatcaaccagtctctggccttcatcagaagaagcgatgagctgctt

SEQ ID NO: 171 - DNA, 1464 bp, synthetic construct
  source 1..1464: mol_type = other DNA
caaaatatcaccgaggagttctaccagtccacctgcagcgctgtgtctagaggttacttctccgccctgcggaccggctggtacaccagcgtcatcaccatcgaactcagcaatatcaaggaacctaagtgcaacggcaccgacaccaaggtgaagctgatcaagcaggagctggataagtacaagaacgccgtgaccgagctgcagctgctgatgcagaacacccctgccgccaacaacggctctgcaagcgaggcccctcagtatatgaactatacaatcaacacaacaaagaacctgaacgtgtccatcagcaagaagggcaagggcagattcctgggcttcctgctcggcgtgggcagcgctattgccagcggcatcgccgtgtccaaagtgctgcacctgccaggcgaagtgaacaagattaaaaacgctctgcttagcaccaacaaggccgtggtgagcctgtcaaatggagtttccgtgctgaccagcaaagtgctggacctgaagaactacatcaacaaccagttgctgcccatcgtgaatcaacagagctgtagaatcagccccatcgagacagtaattgagtttcagcaaaagaacagccggctgctggaaatcactcgggagttcagcgtgaacgccggcgttacaacaccactgtctacatacatgctgacaaacagcgagctgctgtctctgatcaacgacatgcccatcaccaatgatcagaagaaactgatgtctagtaacgtgcctatcgttagacagcagagctacagcatcatgagcatcatcaaggaagaggtgctggcttacgtggtgcagctgcctatctacggcgtgatcgacaccccttgctggaagctccacacctcccctctgtgcacaacaaatatcaaggagggcagcaacatctgcctgaccagaaccgatagaggctggtattgcgacaacgccggaagcgtgtcttttttcccccaggccgacacctgtaaagtccagagcaacagagtgttctgcgacaccatgaacagcctgacactgccacctgaggtgagcctgtgtaacaccgacatcttcaactctaagtacgattgcaagatcatgaccagcaagaccgatatcagcagcagcgtgatcaccagcctgggcgccatcgtgagctgctacggcaaaaccaaatgcaccgccagcaacaagaatcggggcatcatcaagacattctctaacggatgtgactacgtgtccaacaagggagtggacacagtgtccgtgggcaacaccctgtactacgtgaacaagctggaaggcaagaacctgtacgtgaaaggagagcctatcatcaattactacgaccccctggtctttcctagcgacgagttcgacgcctctatcagccaggtgaacgagaagatcaaccagtctctggccttcattagaaggtccgatgaactgctg

SEQ ID NO: 172 - DNA, 1464 bp, synthetic construct
  source 1..1464: mol_type = other DNA
caaaacatcacagaggagttctaccagagcacatgttctgccgtgtccagaggctacttcagcgccctcagaaccggctggtatacatctgtgatcaccatcgagctgagcaatatcaaggaacctaagtgcaatggcaccgatacaaaggtgaagctgatcaagcaggagctggataagtacaagaatgctgtcaccgaactgcagctgctgatgcagaacacccctgccgccaacaacggaagcgccagcgaggcccctcaatacatgaactacaccatcaataccaccaagaacctgaacgtgtctatcagcaagaagggaaaaggcagattcctgggcttccctctgggcgtcggcagcgctatcgcctcaggtatcgccgtgtccaaggtgctgcacctgcctggcgaggtgaacaaaatcaaaaacgctctgctgagcaccaacaaggccgtggtgtccctgtctaatggcgtttccgtgctgaccagcaaagtgctggacctgaagaactatatcaacaaccagctgctgcccatcgtgaaccagcagtcttgccggatttctcctattgagacagtgattgagtttcagcaaaagaactctagactgcttgaaatcacccgcgagttcagcgtcaatgccggcgtgaccacacccctgagcacctacatgctgacaaacagcgagctgctgagcctgatcaatgatatgcctatcaccaacgaccagaagaagctgatgagcagcaacgtgccaatcgtgcggcagcagagctacagcatcatgagcatcatcaaggaagaagtgctggcctacgtcgtgcagctgcctatctacggcgtgatcgacaccccatgttggaagctgcacacaagccccctgtgcacaaccaacatcaaggagggcagcaacatctgcctgactagaacagatagagggtggtactgcgacaacgctggctccgtgtcttttttcccccaggccgacacctgcaaagtgcagagcaatagagtgttctgcgacacaatgaacagcctgaccctgcctccagaggtgagtctgtgtaacaccgacatcttcaacagcaaatacgactgcaagatcatgacctctaagacagatatcagcagcagcgttatcacctccctgggagccatcgtgagctgctacggcaaaaccaagtgcaccgccagcaacaagaaccggggcatcatcaagaccttcagcaatggatgtgactacgtgagcaacaagggcgtggacaccgtgtccgtgggcaacacgctgtactacgtgaataaactcgaaggcaagaacctgtacgtgaaaggagaacctatcatcaactattacgaccccctggtgtttcctagcgacgagttcgacgccagcatcagccaggtgaacgagaagatcaaccagagtctcgccttcatccggagaagcgatgagctactg

SEQ ID NO: 173 - DNA, 1347 bp, synthetic construct
  source 1..1347: mol_type = other DNA
cagaacatcaccgaggagttctaccagagcacctgtagcgccgtgtccaggggctactttagcgccctgcggaccggctggtacaccagcgtgatcacaatcgagctttctaatatcaaggaacccaagtgcaacggaacagacaccaaggtgaaactgatcaagcaggagctggataagtataagaatgccgtgacagagctgcagctgctgatgcagagcacccctgccaccggcagcggctctgctatcgccagcggcatcgccgtgagcaaagtgctgcacctggaaggagaggtgaacaagatcaagaacgctctgctgtctaccaacaaggccgtggtgtccctgagcaacggcgtgtctgtgctgacgagcaaggtgctggacctgaagaactacatcaacaaccaactgctgcctatcgtgaaccagcagagctgcagaatcagcaatatcgaaaccgtgattgagttccagcaaaagaatagccgcctgctggaaatcacaagagagttcagtgtgaatgcaggcgtcactacacctctgagcacatacatgctgacaaacagtgaactgctatctctgatcaacgacatgcctatcaccaacgatcagaaaaagctgatgagcagcaacgtgcctattgtgcggcagcagagctacagcatcatgagcatcatcaaggaagaggtgctggcctacgtggtccaactgccaatctatggcgtgatcgacaccccctgctggaagctccacacctcccctctgtgcaccacaaacatcaaagaaggctccaacatctgcctgaccagaaccgaccggggctggtactgtgacaacgccggcagcgtgagcttcttcccccaggctgatacctgtaaagtgcagagcaacagagtgttctgcgacacaatgaactccctgaccctgcctcctgaggtgagcctgtgtaacacagacatcttcaacagcaagtacgactgcaagattatgacctccaagaccgatattagcagctctgtgatcacctctctgggcgccatcgtgtcatgctacggcaagacaaagtgcacagcctctaacaaaaatagaggcatcatcaaaacattcagcaacggctgcgattacgtgagcaacaagggagtggacaccgtgagcgttggaaataccctgtactacgttaacaagctggagggcaagaacctgtatgtcaagggcgagcctatcatcaattactacgaccccctggtgtttccatctgatgagtttgacgcctctatcagccaggtgaacgagaagatcaaccagtccctggccttcatcagaagaagcgacgagctgctc

SEQ ID NO: 174 - DNA, 1347 bp, synthetic construct
  source 1..1347: mol_type = other DNA
cagaacatcacagaggagttctaccagtctacatgtagcgctgtgtctcggggctacttcagcgccctgagaacaggctggtacaccagcgtgatcaccatcgagctgagcaacatcaaagaacccaagtgcaacggaaccgataccaaggtgaaactgatcaagcaggagctggacaagtacaagaatgccgtgaccgagctgcagctgctgatgcagtccacacctgctacaggtagcggctccgccatcgccagcggcatcgccgtgagcaaagtgctgcacctggaaggcgaggtgaacaaaatcaaaaacgccctgctgagcacaaacaaggccgtggtctctctgagcaacggcgtgtccgtcctgaccagcaaggtgctggatctgaagaactacatcaacaaccagctgctgcccatcgtgaatcaacagagctgcagaataagccccatcgagacagtgatcgagtttcagcaaaagaacagcagactgctcgaaatcactagagagttctctgtgaatgctggcgttacaacacctctgagcacctacatgctgaccaacagcgagctgctgtctctcatcaatgacatgcctatcaccaacgaccagaaaaagctgatgagcagcaatgtgcctattgtgcggcagcagagctacagcatcatgagcatcatcaaggaagaagtgctcgcctacgtggtgcaacttcctatctacggcgtgatcgacaccccgtgctggaagctgcacacctcccctctgtgtaccaccaatatcaaggaaggctctaacatctgcctgacaagaaccgatagaggatggtattgtgacaacgccggctccgtgtcattcttcccccaggccgacacatgcaaggtccagagcaatcgggtgttctgcgacaccatgaactcactgaccctgccacctgaggtgagcctgtgcaataccgacatctttaacagcaaatacgactgcaagatcatgaccagcaagacagatatcagcagctctgttatcactagcctcggcgccatcgtgtcttgttacggaaagaccaagtgcaccgctagcaacaagaaccgcggcatcattaagaccttcagcaacggctgcgactacgtgtctaacaagggcgtggacaccgtgagcgtgggcaacaccctgtactacgtgaacaagctggaaggcaagaatctgtacgtgaagggagaacctatcatcaactactatgatcctctggtgtttccatctgatgagttcgacgcctccatcagccaggtcaacgagaagatcaaccagagcctggccttcatccggagatccgacgagctgctg

SEQ ID NO: 175 - DNA, 1347 bp, synthetic construct
  source 1..1347: mol_type = other DNA
cagaacatcaccgaggagttctaccagagcacatgcagcgccgtgtccagaggatacttcagcgccctgagaaccggctggtacaccagcgtgatcaccatcgagctctctaacatcaaggaacctaagtgcaacggtacggacaccaaggttaagctgatcaagcaggagctggataagtacaaaaacgccgtgacagagttgcagctgcttatgcagtctacccctgctacaggcagcggctccgccatcgcttctggcatcgccgtctccaaagtgctgcacctgcctggagaagtgaacaagatcaaaaacgccctgctgagcacaaacaaggccgtggtgtccctgtctaatggagttagcgtgctgacaagcaaggtgctggacctgaagaattacatcaacaaccagctgctgcctatcgtcaaccaacaaagctgcagaatctcccctattgagacagtgatcgagtttcagcagaagaatagccggctgctggaaatcacccgggaatttagcgtgaacgccggagtgaccacacctctgagcacctacatgctgaccaacagcgagctgctgagcctgatcaacgacatgcctatcaccaatgaccagaaaaagctcatgtctagcaatgtgcctatcgtgcggcagcagagctacagcatcatgagcatcatcaaggaagaggtgctggcctacgtcgtgcagctgccaatttacggcgtgatcgacaccccatgttggaagctgcacaccagccctctgtgtaccacaaacatcaaagagggctctaacatttgcctgacaaggaccgatagaggctggtattgcgacaacgctggcagcgtgtccttcttccctcaggccgacacctgcaaggtccaatctaatagagtgttctgcgataccatgaacagcctgaccctgccccccgaggtgagcctgtgcaacacagatatcttcaactccaagtatgattgcaagatcatgaccagcaagaccgacatcagcagcagcgtgatcacatctctgggcgctatcgtgagttgttacggcaagacaaaatgcaccgccagcaacaagaacagaggaatcatcaaaacctttagcaacggctgtgactacgtgtctaataagggcgtcgacacagtgagcgtgggcaacaccctgtactacgtgaacaagctggaaggcaaaaatctgtacgtgaagggcgaacccatcattaactactacgaccccctggtgttccccagcgacgagttcgacgccagcatcagccaggtgaacgagaagatcaaccagtctctggccttcatccggagaagcgatgagctgctg

SEQ ID NO: 176 - DNA, 1398 bp, synthetic construct
  source 1..1398: mol_type = other DNA
caaaacatcaccgaggaattttaccagtctacatgctctgctgtctcccggggctacttcagcgccctgagaaccggctggtacacaagcgtgattaccatcgagctgtctaatatcaaggaacctaagtgcaacggtacagataccaaggttaaactgatcaaacaggagctggacaagtacaagaacgccgtgacagagctgcagctgctgatgcagaacacccctgccgccaacaaccgggccagaggctccggcagcggaagaagcctgggcttcctgttgggcgtcggcagcgcgatcgcctctggcatcgccgtgtcaaaggtgctgcacctggaaggcgaagtgaacaaaatcaaaaacgctctcctgagcacaaacaaggccgtggtgagcctgagcaatggcgtgtccgtgctgaccagcaaggtgctggatctgaagaactacatcaacaaccagctgctgcctatcgtgaaccagcagagctgcagaatcagccccatcgaaacggtgatcgagtttcagcaaaagaacagcagactgctggaaatcaccagagagttcagcgtcaacgctggcgtgaccacacctctgtccacctacatgctgaccaacagcgagctgctgagcctgatcaacgacatgcctattaccaatgatcagaaaaagctgatgagcagcaacgtgcccatcgtgcggcagcagagctacagcatcatgagcatcatcaaggaagaggtgctggcttacgttgtgcagctgcctatctacggcgtgatcgacaccccttgttggaagctgcacacaagcccactgtgcacaacaaacatcaaggagggaagcaacatctgcctgacccggaccgacagaggctggtattgcgacaacgccggctctgtgagcttcttcccccaggccgacacctgcaaggtgcagtccaatagagtgttctgcgacacaatgaacagcctgacactgccccccgaggtgagcctttgtaataccgatatcttcaactctaagtacgactgcaagatcatgacatctaaaacagacatcagctctagcgtgatcacctccctcggcgccatcgtgtcctgctacggcaaaaccaagtgtaccgcctcgaacaagaacagaggaatcatcaagaccttcagcaacggatgtgactacgtgagcaataaaggagtggacaccgtgtctgtgggcaacaccctgtattacgtgaacaagctggaaggcaagaacctgtacgtgaagggcgagcctattatcaactactacgatcctctggtctttccatctgatgagttcgacgccagcatcagccaggtgaacgagaagatcaatcaaagcctggccttcatcaggcggagcgacgagctgctc

SEQ ID NO: 177 - DNA, 1398 bp, synthetic construct
  source 1..1398: mol_type = other DNA
caaaatatcacagaggagttctaccagtctacctgcagcgccgtcagcaggggctacttctctgccctgcggaccggctggtacacttccgtgatcaccatcgagctgagcaacatcaaggaacctaagtgcaacggcaccgatacaaaggtgaagctgatcaaacaggagctggataagtacaagaacgccgtgaccgagctgcagctgctgatgcagaacacacctgccgcaaataacagagccagaggatctggcagcggcagaagcctgggcttcctgctgggagtgggaagtgctatcgcctctggcatcgctgtgtccaaggtgctgcacctgcccggggaagtgaacaagatcaagaacgctctgctgtctacaaataaggccgtggtgagcctgagcaacggcgtcagcgtgctgacctctaaggtgctggacctgaagaactacatcaacaatcagctgctgcccatcgtgaatcaacagtcttgcagaatcagccctattgaaaccgtgatcgagtttcagcagaaaaacagccggctgctggaaatcacaagagagttcagcgtgaacgccggcgttaccacacccctgagcacctacatgctgacaaactctgagctgctgtctctcatcaacgatatgcctatcacaaacgaccaaaagaaactgatgagcagcaacgtgcctatcgttagacagcagagctacagcatcatgtccatcatcaaagaagaggtgctggcctacgtcgtgcagctgcctatctacggcgtgatcgacaccccttgttggaagctgcacaccagcccactgtgtaccaccaacatcaaggagggcagcaatatctgcctgaccagaacagacagaggctggtactgcgacaacgctggcagcgtgtcctttttcccccaggccgacacatgcaaagtgcagagcaatcgggtgttctgcgacaccatgaacagcctgaccctgcctccagaggtgagcctctgtaataccgacatcttcaacagcaagtatgattgcaagatcatgacctctaaaaccgacatcagcagcagcgtgatcacatctctgggcgccatcgtctcgtgctacggaaagaccaagtgcaccgccagcaacaagaaccgggggatcattaagaccttcagcaatggatgtgactacgtgtccaacaagggcgtggacaccgtgagcgtgggcaacacactgtactacgtgaacaaactggaaggcaagaacctgtatgttaagggcgaacccattatcaactactatgatcctctggtgtttcctagcgacgagttcgacgccagcatcagccaggtgaacgagaagattaaccagagcctggccttcatccggagatcagatgagctgctc

SEQ ID NO: 178 - DNA, 1347 bp, synthetic construct
  source 1..1347: mol_type = other DNA
caaaacatcaccgaggagttctaccagagcacctgcagcgccgtgagcagaggctacttcagcgctctgaggacaggctggtatacaagcgtgatcaccatcgaacttagcaatatcaaagaacctaagtgcaacggcaccgacacaaaggtgaaactgatcaagcaggagctggacaagtataagaacgccgtgaccgagctgcagctgctgatgttcctgggctttccactgggcgtgggcagcgccattgcctctggcatcgctgtgtccaaggtgctgcacctggaaggcgaggtgaacaagatcaagaacgccctgctgagcaccaacaaggccgtggtgagcctgagcaacggcgtgtccgtcctgaccagcaaagtgctggacctgaagaactacatcaacaaccaactgctgcccatcgtgaaccagcagagctgcagaatttccaacatcgagacagtgatcgagtttcagcaaaagaacagccggctgctggaaatcacaagagagttctctgtgaacgctggcgtgaccacacccctgtctacctacatgctgacaaactccgagctgctgagcctgatcaacgacatgcctatcaccaacgaccagaaaaagctgatgagcagcaatgtgcccatcgtgcggcagcagagctacagcatcatgagcatcatcaaggaagaggtgctggcctacgtggtgcagctgcctatctacggcgtgatcgacacaccttgttggaagctgcacaccagccctttatgcacaacaaacatcaaggaaggcagcaacatctgcctgacccggaccgatagaggctggtactgcgacaacgccggctctgtgtccttcttccctcaggctgatacctgtaaagtgcagtctaacagagtgttctgcgataccatgaacagcctgaccctgccacctgaggtgagcctgtgtaacacggatatcttcaacagcaagtacgactgcaagattatgaccagcaagaccgacatctcttctagcgtcattacctctctgggagccatcgtgagttgctacggcaagactaagtgcaccgccagcaacaagaaccggggcatcatcaagacattcagcaatggatgtgattacgttagcaacaaaggcgtcgacaccgtgtccgttggaaataccctctactatgttaataaactggaaggaaagaatctgtacgtgaagggcgagcctatcatcaactactacgaccccctcgtgtttcctagcgacgagttcgacgccagtatctctcaggtgaacgagaagatcaatcagagcctggccttcatcagaagaagcgatgagctgctg

SEQ ID NO: 179 - DNA, 1347 bp, synthetic construct
  source 1..1347: mol_type = other DNA
cagaacatcactgaagagttctaccagagcacctgcagcgccgtgagcagaggttacttcagcgccctgagaaccggctggtatacaagcgtgatcaccatcgagctgtctaacatcaaggaacccaagtgtaatggcaccgacaccaaggtgaagctgatcaaacaggagctggataaatacaagaacgccgtgaccgagctgcagctgctgatgttcctgggcttccccctgggcgtgggctctgctatcgcctccggcatcgctgtgtctaaggttctgcacctggaaggcgaggtgaataagatcaaaaatgctctgctgagcaccaacaaggccgtggtctccctgagcaatggcgtcagcgtgctgaccagcaaggtgctggacctgaagaattacatcaacaaccaactgctgccaatcgtgaaccagcagagctgccggatctcacctattgagacagtgatcgagtttcagcagaagaacagcagactgctggaaatcacccgggaatttagcgtgaacgccggcgtgacaacacctctgagcacatacatgctgaccaacagcgagctgctgtcgctgatcaacgacatgcctatcacaaacgaccagaaaaagctgatgtcaagcaacgtgcctattgtgcggcagcaaagctacagcatcatgagcatcattaaagaggaagtcctggcctacgtggtgcaactccctatctacggcgttatcgacaccccctgttggaagctgcacacctctcctctgtgcaccaccaatatcaaggaaggcagcaatatctgcctgacacgcaccgatagaggctggtattgcgataacgccggcagcgtgtctttcttcccacaggccgatacatgtaaagtgcagagcaacagagtgttctgcgacacaatgaacagcctgacactgcctcctgaggtgtccctctgcaacaccgacatcttcaactccaagtatgactgcaagatcatgaccagcaagacagatatctcctccagcgtgatcacctctctgggagccatcgtgagctgctacggcaagaccaagtgcaccgcctccaacaagaaccggggcatcatcaaaaccttcagcaacggatgtgactacgtgagcaacaagggagtggacacagtgtctgtgggcaacaccctgtactacgtcaacaagctggaaggaaagaacctgtacgttaagggagagcccattataaactactacgaccctctggtgttccccagcgacgagttcgacgccagcatctctcaggtgaacgagaagatcaatcagtctctggcttttatcagaagatctgatgagctgcta

SEQ ID NO: 180 - DNA, 1347 bp, synthetic construct
  source 1..1347: mol_type = other DNA
cagaacatcaccgaggagttctaccagagcacatgttccgctgtgtcccggggctacttcagcgccctgagaaccggctggtacacctctgtgatcacgatcgagctgagcaatattaaggaacccaagtgcaacggcacagacaccaaggtgaagctgatcaagcaggagctggataagtacaagaacgccgtgaccgagctgcagctgctgatgttcctaggatttccactgggcgtgggatctgctatcgcatctggcattgccgtgagcaaagtgctgcacctgcctggcgaggtgaacaagatcaagaacgccctgctgagcaccaacaaggccgtggtcagtctgtctaacggcgtgtccgtgctgacatctaaggtgctggacctcaagaactacatcaacaaccagctgctgccaatcgtcaatcaacagagctgcaggatcagccctatcgagacagtgatcgagtttcagcaaaagaacagcagactgctggaaatcacaagagaatttagcgtgaatgctggcgtgacaacccctctgagcacctacatgctgacaaatagcgagctgctgagcctgatcaacgacatgcctatcaccaacgaccagaaaaagctgatgtccagcaacgtgcctattgtgcggcagcagagctacagcatcatgagcatcatcaaagaagaagtgctggcctacgtggtgcagctgcctatctacggcgttatcgacacaccttgctggaagctgcacacctcccctctgtgcaccaccaacatcaaagagggcagcaatatctgcctgaccagaaccgatagaggctggtactgcgacaacgccggcagcgtgagcttcttccctcaggccgacacctgtaaagtgcagagcaaccgggttttctgcgataccatgaacagcctgacactgccccccgaggtgtccctgtgtaacaccgacatcttcaactccaagtacgattgcaagatcatgacaagcaagaccgatatcagcagctctgttatcaccagcctgggagccatcgtgtcttgttacggcaagaccaagtgcaccgcctccaacaagaaccggggaatcatcaagacattcagcaatggctgcgactacgtgagcaacaagggcgtcgacaccgtgagcgtgggcaacaccctgtattatgtgaacaaactggaaggaaagaatctgtacgtgaaaggcgaacctattatcaactactacgaccccctggtgttccccagcgacgagttcgacgccagcatcagccaggtgaacgagaagatcaaccaatctctggccttcatcagaagatctgatgagctgctc